European Patent Application EP 4 438 620 A1, published October 2, 2024. Title: CHO cells with optimized host cell protein profile. Applicant: Sartorius Stedim Cellca GmbH. The sequence listing filed with the application follows.

SEQUENCE LISTING (156 sequences)

SEQ ID NO: 1 - protein, 533 aa, Cricetulus griseus
MANKQVCNPRNPCTDGTHDCNKNAKCNYLGHYSDPMYRCECKPGYAGNGIICGEDTDLDGWPNEDLVCVANATYHCKKDNCPNLPNSGQEDYDKDGIGDACDDDDDNDKIPDDRDNCPFHYNPAQYDYDRDDVGDRCDNCPYNHNPDQADTDNNGEGDACAVDIDGDGILNERDNCQYVYNVDQRDTDMDGVGDQCDNCPLEHNPDQLDSDSDLIGDTCDNNQDIDEDGHQNNMDNCPYVPNANQADHDKDGKGDACDHDDDNDGIPDDRDNCRLVPNPDQKDSDGDGRGDACKDDFDHDNVPDIDDICPENVDISETDFRRFQMIPLDPKGTSQNDPNWVVRHQGKELVQTVNCDPGLAVGYDEFNAVDFSGTFFINTERDDDYAGFVFGYQSSSRFYVVMWKQVTQSYWDTNPTRAQGYSGLSVKVVNSTTGPGEHLRNALWHTGNTPGQVRTLWHDPRHIGWKDFTAYRWRLSHRPKTGYIRVVMYEGKKIMADSGPIYDKTYAGGRLGLFVFSQEMVFFSDMKYECRDS

SEQ ID NO: 2 - protein, 2486 aa, Cricetulus griseus
MLRGPGPGLLLAVLCLGTAVRCTEAGKSKRQTQQIVQPQQIVQPQSPVAVSQSKPGCFDNGKHYQINQQWERTYLGNALVCTCYGGSRGFNCESKPEPEETCFDKYTGNTYKVGDTYERPKDSMIWDCTCIGAGRGRISCTIANRCHEGGQSYKIGDKWRRPHETGGYMLECLCMGNGKGEWTCKPIAEKCFDHAAGTSYVVGETWEKPYQGWMMVDCTCLGEGSGRITCTSRNRCNDQDTRTSYRIGDTWTKKDNRGNLLQCVCTGNGRGEWKCERHALQSTSAGSGSLTDVRTAVYQPQTHLQPAPYGHCVTDSGVVYSVGMQWLKSQGNKQMLCTCLGNGVSCQETAVTQTYGGNSNGEPCVLPFTYNGRTFYSCTAEGRQDGHLWCSTTSNYEQDQKYSFCTDHTVLVQTRGGNSNGALCHFPFLYNNRNYTDCTSEGRRDNMKWCGTTQNYDADQKFGFCPMAGKMKKASHEEICTTNEGVMYRIGDQWDKQHDLGHMMRCTCVGNGRGEWSCIPYSQLRDQCIVDDITYNVNDTFHKRHEEGHMLNCTCFGQGRGRWKCDPIDQCQDSETRTFYQIGDSWEKFVHGVRYQCYCYGRGIGEWHCQPLQTYPGTTGPVQVIITETPSQPNSHPIQWNAPEPSHITKYILRWRPKTSVGRWKEATIPGHLNSYTIKGLTPGVVYEGQLISIQQYGHREVTRFDFTTSAGTPVTSNTVTGETAPFSPVVATSESITEITASSFVVSWVSASDTLSGFLVEYELSEEGGKPQYLDLPSTATSVNIPDLLPGRKYIVNVYQISEEGKQSLILSTSQTTAPDAPPDPTVDQVDDTSIVVRWSRPQAPITGYRIVYSPSVEGSSTELNLPETANSVTLSDLQPGVQYNITIYAVEDNQESAPVFIQQETTGTPRSDKVPPPKDLQFVEVTDVKVTIMWTPPDSPVTGYRVDVLPVNLPGEHGQRLPVNRNTFAEITGLTPGVTYHFNVYAVNQGRESKPLTAQQTTKLDAPTNLQFVNESDRTVLVTWIPPRARIAGYRLTVGLTRGGQPKQYNVGPSASKYPLRNLQPGSEYTVTLVAVKGNQQSPKATGVFTTLQPMSSIPPYNTEVTETTIVITWTPAPRIGFKLGVRPSQGGEAPREVTSESGSIVVSGLTPGVEYTYTIQVLRDGQEKDAPIVNRVVTPLSPPTNLHLETNPDTGVLTVSWERSVTPDITGYRITTTPTNGQQGSSLEEVVHADQSSCTFENLNPGLEYNVSVYTVKDDKESAPISDTIIPEVPQLTDLSFVDITDSTIGLRWTPLNSSTIIGYRITVVATGEGIPIFEDFVDSSVGYYTVTGLEPGIDYDISVITLINGGESAPTTLTQQTAVPPPTDLRFTNIGPDTMRVTWAPPPSIELTNLLVRYSPVKNEEDVAELSISPSDNAVVLTNLLPGTEYLVSVSSVYEQHESTPLRGRQKTGLDSPTGFDSSDITANSFTVHWVALRAPITGYIIRHHAEQSVGRPRQDRVPPSRNSITLSNLNPGTEYIVSIIAVNGREESAPLIGQQSTVSDVPRDLEVIASTPTSLLISWEPPAVSVRYYRVTYGETGGNSPVQEFTVPGSKSTATINNIKTGTDYTITLYAITGRGDSPASSKPISINYRTEIDKPSQMQVTDVQDNSISVRWLPSSSPVTGYRVTTTPKNGPGPSKTKTAGPDQTEMTIEGLQPTVEYVVSVYAQNQNGESQPLVQTAVTNIDRPKGLAFTDVDVDSIKIAWESPQGQVSRYRVTYSSPEDGIHELFPAPDGEEDTAELQGLRPGSEYTVSVVALHDDMESQPLIGIQSTAIPAPTNLKFTQVTPTSFSAQWVAPNVQLTGYRVRVTPKEKTGPMKEINLSPDSSSVVVSGLMVATKYEVSVYALKDTLTSRPAQGVITTLENVSPPRRARVTDATETTITISWRTKTETITGFQVDAIPANGQPPVQRTISPDIRTYTITGLQPGTDYKIHVYTLNDNARSSPVIIDASTAIDAPSNLRFLATTPNSLLVSWQAPRARITGYIIKYEKPGSPPREVVPRPRPGVTEATITGLEPGTEYTIYVIALKNNQKSEPLIGRKKTDELPQLVTLPHPNLHGPEILDVPSTVQKTPFITNPGYDTENGIQLPGTTHQQPSVGQQMIFEEHGFRRTTPPTAATPVRLRPRPYLPNVDEEVQIGHVPRGDVDYHLYPHVPGLNPNASTGQEALSQTTISWTPFQESSEYIISCHPVGTDEEPLQFQVPGTSTSATLTGLTRGVTYNIIVEALQNQRRHKVREEVVTVGNAVNEGLNQPTDDSCFDPYTVSHYAIGEEWERLSDSGFKLTCQCLGFGSGHFRCDSSKWCHDNGVNYKIGEKWDRQGENGQRMSCTCLGNGKGEFKCDPHEATCYDDGKTYHVGEQWQKEYLGAICSCTCFGGQRGWRCDNCRRPGGEPSPDGTTGHTYNQYTQRYHQRTNTNVNCPIECFMPLDVQADRDDSRE

SEQ ID NO: 3 - protein, 199 aa, Cricetulus griseus
MGIMNSFVNDIFERIAGEASRLAHYNKRSTITSREIQTAVRLLLPGELAKHAVSEGTKAVTKYTSSKSSVRSAACCIKACSQLKAQCFSSQRFTVTMSGRGKGGKGLGKGGAKRHRKVLRDNIQGITKPAIRRLARRGGVKRISGLIYEETRGVLKVFLENVIRDAVTYTEHAKRKTVTAMDVVYALKRQGRTLYGFGG

SEQ ID NO: 4 - protein, 472 aa, Cricetulus griseus
MLKEMIKSGMNVARLNFSHGTHEYHAETIKNVRTATESFASDPILYRPVAVALDTKGPEIRTGLIKGSGTAEVELKKGATLKITLDNAYMEKCDENILWLDYKNICKVVEVGSKIYVDDGLISLQVKEKGADYLVTEVENGGSLGSKKGVNLPGAAVDLPAVSEKDIQDLKFGVEQGVDMVFASFIRKAEDVHEVRKVLGEKGQNIKIISKIENHEGVRRFDEILEASDGIMVARGDLGIEIPAEKVFLAQKMMIGRCNRAGKPVICATQMLESMIKKPRPTRAESSDVANAVLDGADCIMLSGETAKGDYPLEAVRMQHLIAREAEAAIYHLQLFEELRRLAPITNDPTEAAAVGAVEASFKCCSGAIIVLTKSGRSAHQVARYRPRAPIIAVTRNPQTARQAHLYRGIFPVLCKDAVQDAWAEDVDLRVNLAMNVGKARGFFKTGDVVIVLTGWRPGSGYTNTMRVVPVP

SEQ ID NO: 5 - protein, 447 aa, Cricetulus griseus
MKILLLCVGLLLTWDNGMVLGEQEVSDNELKEMSTQGSRYINKEIQNAVQGVKQIKTLIEKTNEERKSLLNSLEEAKKKKEDALDDTRDTEMKLKAFPEVCNETMMALWEECKPCLKQTCMKFYARVCRSGSGLVGRQLEEFLNQSSPFYFWMNGDRIDSLMESDRQQSQVLDAMQDSFTRASGIMDMLFQDRFFTHEPQDTHYFSPFGFPHRRPHFLYPKSRLVRSLIPLSHYGPPSFHDMFQPFLEMIHQAQQAMDVQFHRPAFQFPDKGLREGEDDRAVCKEIRHNSTGCLKMKGQCEKCQEILSVDCSANNPAQAHLRQELNDSLQMAERLTQQYNELLHSLQTKMLNTSSLLEQLNEQFNWVSQLANLTQGEDQYYLRVSTVTTHSNNSEEPSRVTEVVVKLFDSDPITVVLPEEVSKDNPKFMDTVAEKALQEYRKKSRAE

SEQ ID NO: 6 - protein, 199 aa, Cricetulus griseus
MSSGNAKIGYPAPNFKATAVMPDGQFRDICLSEYRGKYVVFFFYPLDFTFVCPTEIIAFSDRAEEFKKLNCQVIGASVDSHFCHLAWINTPKKQGGLGPMNIPLVSDPKRTIAQDYGVLKADEGISFRGLFIIDDKGILQQITINDLPVGRSVDEILRLVQAFQFTDKHGEVCPAGWKPGSDTIKPDVQKSKEYFSKQK

SEQ ID NO: 7 - protein, 333 aa, Cricetulus griseus
MVKVGVNGFGRIGRLVTRAAFTSGKVEVVAINDPFIDLNYMVYMFQYDSTHGKFKGTVKAENGKLVINGKAITIFQERDPANIKWGDAGAEYVVESTGVFTTMEKAGAHLKGGAKRVIISAPSADAPMFVMGVNQDKYDNSLKIVSNASCTTNCLAPLAKVIHDNFGIVEGLMTTVHAITATQKTVDGPSGKLWRDGRGAAQNIIPASTGAAKAVGKVIPELNGKLTGMAFRVPTPNVSVVDLTCRLEKPAKYEDIKKVVKQASEGPLKGILGYTEDQVVSCDFNSDSHSSTFDAGAGIALNDNFVKLISWYDNEFGYSNRVVDLMAYMASKE

SEQ ID NO: 8 - protein, 375 aa, Cricetulus griseus
MDDDIAALVVDNGSGMCKAGFAGDDAPRAVFPSIVGRPRHQGVMVGMGQKDSYVGDEAQSKRGILTLKYPIEHGIVTNWDDMEKIWHHTFYNELRVAPEEHPVLLTEAPLNPKANREKMTQIMFETFNTPAMYVAIQAVLSLYASGRTTGIVMDSGDGVTHTVPIYEGYALPHAILRLDLAGRDLTDYLMKILTERGYSFTTTAEREIVRDIKEKLCYVALDFEQEMATAASSSSLEKSYELPDGQVITIGNERFRCPEALFQPSFLGMESCGIHETTFNSIMKCDVDIRKDLYANTVLSGGTTMYPGIADRMQKEITALAPSTMKIKIIAPPERKYSVWIGGSILASLSTFQQMWISKQEYDESGPSIVHRKCF

SEQ ID NO: 9 - protein, 249 aa, Cricetulus griseus
MKTLVPALELTDSYEAPNIVFCKACQFVMQKFSALTANKDAVDLMMKSVSKACTLIPGPDSTKCTEVIQTFGPSLLDILLREVSADMCGVIRLCSGNPDSVETLEQPAVPILSALPKQPALRAIVPQKKTGGFCEVCKKLVSYLEHNLEKNSTKEEILAALEKGCSFLPDPYQKECDDFVSEYEPLLVEILVQVMDPSFVCSKIGACPSASKLLLGTEKCVWGPSYWCQNMETAARCNAVDHCKRHVWN

SEQ ID NO: 10 - protein, 2323 aa, Cricetulus griseus
MLLGPGHTLSAPALALAVTLTLLVRSASPASFFGENHLEVPVPTALTRVDLLLQFSTSQPDALLLLAAGQADHLLLQLYSGRLQVRLVLDQKEMKLQTPTDIVLSDSAPHTLVLTVSNSWAVLSVDGILNTSTPIPKAHLEVTYGLFVGGSGSLDLPYLKGLSRPLRGCIHSASLNGRNLLRPLTPDVREGCAEELSAGDDVGLGFSGPHSLAAFPAWSTQEEGTLEFTLTTRSQQAPLAFQAGDQRGNFIYVAIFEGHLRAVVEKGQGTMVLRNSVPVSDGQPHEVSVHIDAHRLEISVDQYPTRTFNRGVLSYLEPHGSLLLGGLDAEASRHLQEHRLGLAPGDVNISLVGCIEDFSINGRRQGLRDAWLTRDMAAGCRPEEDEYEEEAYGPYETFSTLAPEAWPAMELPEPCIPEPGLPPVFANFTQLLTISPLVVAEGGTAWLEWRHVQPTLDLTEAELRKSQVLFSVSQSARHGELELDIPGAQTRKMFTLLDVVNRKARFVHDGSEDTSDQLMLEVSVTARAPVPSCLRRGQIYILPIQVNPVNDPPRIIFPHGSLMVILEHTQKPLGPEIFQAYDPDSACEGLTIQLLGASTGIPVEHRDQPGEAVTEFSCRDLEAGNIVYVHRGGPAQDLTFRVSDGMQASAPATLKVVAVRPAIQILHNTGLHLAQGSAAPILPANLSVETNAVGQDVSVLFRVTGTLRFGELQKQGAGGVEGTEWWETLAFHQRDVEQGRVRYLSTDPQHHTQDMVEDLTLEVQVGQETLSNLSFPVTIQRATVWMLRLEPLHTQNPHQETLTPAHLEASLEGEAGPYPHTFHYELVQAPRKGNLQLQGTRLSDGQSFSQSDLQAGHVTYRATMRTSEAADDSFRFRVLSPPHFSPLYTFPIHIGGDPNAPVLTNVLLIVPEGGEGVLSADHLFVKSLNSASYLYEVMEQPHHGRLAWKEPKGKATPVTSFTNEDLLHGRLVYQHDDSETIEDDIPFVATRQGEGSGDMAWEEVRGVFRVAIQPVNDHAPVQTISRVFHVARGGQRLLTTDDVAFSDADSGFTDAQLVLTRKDLLFGSIVAMEEPTRPIYRFTQEDLRKKQVLFVHSGADHGWLQLQVSDGQHQATAMLEVQASEPYLHVVNNSSLVVPQGGQGTIDTAVLHLDTNLDIRSGTEVHYHVTAGPHSGQLLRDGQSVNSFTQQDLLEGAILYSHNGSLSPHDTVALSVAAGPVHTNTILQVTIALEGPLAPLQLVQHKKIYVFQGEAAEIRRDQLEVAQEAVQPADIMFSLRSPPSAGYLVMVSHGASADEPPSLDPVQSFSQEAVNSGRVLYLHSRPGAWSDSFSLDVASGLGDPLEGIFVQLEVLPTAIPLKVQNFSVPEGGTRTLAPPLLQITGPYFPTLPGLLLQVLEPPQHGALQKEDQPQDGSLGTFSWREVEEQLIRYVHDGSETPTDSFVLVANASEMDRQSQPMAFTVTILPVNDQPPVLTTNTGLQIWEGATVPIPPEALRGTDNDSGPEDLIYTIQQPSNGRIALRVAPDTEVRHFTQAQLDNGLVLFSHRGALEGGFHFDLSDGAHTSSGHFFRVVAQKQVLLSLEGSRKLTVCPESVQPLSSQSLRASSSTGTDPRHLLYRVVRGPQLGRLFHAQQGSAEEALVNFTQAEVNAGNILYEHGKYPEPFWEAHDTIGLLLSSPPARDVAATLAVVVSFDAACPQRPSRLWRNKGLWVPEGQRAKITVASLDASNLLASVPASQRTRHDVLFQVTQFPTRGQLLVSEEPLHARRPHFLQSELAAGQLVYAHGGGGTQQDSFRFRAHLQGPTGASVAGPQTSEAFAITVRDVNERPPQPQASIPLRVTRGSRAPVSRAQLSVVDPDSAPGEIEYEVQRAPHNGFLSLAGDNTGPVTHFTQADVDAGRLAFVANGSSVAGIFQLSMSDGASPPIPMSLAVDVLPSTIEVQLRAPLEVPQALGRSSLSRQQLQVISDREEPEVAYRLTQGPRYGQLLVGGQPASAFSQMQVDQGEVVFAFTNFSSSQDHFKVLALARGVNASATVNVTVQALLHVWAGGPWPQGTTLRLDPTVLDASELANRTGSMPHFRLLAGPRYGRVVRVSQAHTEPRSNRLVEHFTQQDLEEGRLGLEVGRPEGRSTGPAGDSLTLELWARGVPPAVALLDFATEPYHAAKSYSVALLSVPEAARTETEKPGRNTPTGQPGPAASSPIPTMARSGFLGFLEANMFSVIIPVCLVLLLLALILPLLFYLRKRNKTGKHDVQVLTAKPRNGLAGDTETFRKVEPGQAIPLTTVPGQGPPPGGQPDPELLQFCRTPNPALRNGQYWV

SEQ ID NO: 11 - protein, 382 aa, Cricetulus griseus
MSESSEGYTYTETSVLLLRFKVPKSSKSKMATLKDQLIVNLLKEEQTPQNKITIVGVGAVGMACAISILMKDLADELALVDVMEDKLKGEMMDLQHGSLFLRTPKIVSGKDYSVTANSKLVIVTAGARQQEGESRLNLVQRNVNIFKFIIPNVVKYSPDCKLLIVSNPVDILTYVAWKISGFPKNRVIGMDILTYVAWKISGFPKNRVIGSGCNLDSARFRYLMGERLGVHPLSCHGWVLGEHGDSSVPVWSGVNVAGVSLKNLNPELGTDTDKEQWNEVHKQVVDSAYEVIKLKGYTSWAIGLSVADLAESIMKNLRRVHPISTMIKGLYGIKDDVFLSVPCVLGQNGISDVVKVTLTSEEEARLKKSADTLWGIQKELQF

SEQ ID NO: 12 - protein, 3140 aa, Cricetulus griseus
MALAGIDTLLIQASYTQQPAESRVSGISMDIAVPDYTGQDSALEVEQCTCPPGYRGPSCQDCDTGYTRMPSGLYLGTCERCNCHGHSEACEPETGVCQSCQHHTEGAHCEQCQPGFYGDAQRGTPQDCQPCPCYGAPAAGQAAHTCFLDTDGHPTCDSCSAGHSGRHCERCAPGYYGNPSQGQPCHRDGQGPEDLGCGCDPHGSVSSQCDASGQCQCKAQVEGLTCSHCRPHHFYLSASNPEGCLPCFCMGVTQQCASSSYSRHQISTQFAPGDFQGFALVNPQRNSQLTGGFTVESVSGGSQLSFGNFAHLGQESFYWQLPETYQGDKVAAYGGKLRYTLSYTSGPQGSPLSDPDIQITGNNIMLVASQPAPQGPERRSYEIIFREEFWRRPDGQPATREHLLMALADLDELLIRATFSSVPRAASISAVSLEVAQPGPSGGPRALEVEECRCPPGYVGLSCQDCAPGYTRTGSGLYLGHCELCECNGHSDLCHPETGACSRCQHNTAGEFCELCATGYYGDATAGTPEDCQPCACPLTNPENMFSRTCESLGAGGYRCTACEPGYTGQYCEQCAPGYEGNPNVQGGRCQPLTKDFLEVQIHPSRSVVPQGGPHSLRCQVNGSPPHYFYWSREDGRPISSGAQQRHQGSELHFPSVQPSDAGVYICTCQNLHHTSNSRAELLVTEAPSKPITVTVEEQRSQSVRPGADVTFICTAKSKSPAYTLVWTRLHNGKLPSRAMDFNGILTIRNVQPSDAGTYVCTGSNMFAMDQGTATLHVQVSGTSTAPVVSIHPPQLTVQPGQLAEFRCSATGNPTPTLEWTGGPSGQLPQKAQIHGGILRLPAIEPSDQGQYLCRALSSAGQHVARAMLQVHGGSGPRVQVSPERTQVYEGHTVRLYCRAAGVPSASITWRKEGGSLPPQARSDNTEIPTLLIPAITPADAGFYLCVATSPTGTAQARIQVVVLSASGTSSVPVRIESSSPSVTEGQTLDLNCAVMGLTYTQVTWYKRGGSLPPHAQVHGSRLRLPRVSPADSGEYVCRVESDLGPKEASIVVSVLHGVHSGPSYTPATGSTPPIRIESSSSHVAEGQTLDLNCVVPGQAQVTWRKRGGSLPARHQTHGPLLRLHQVSPADSGEYVCHVVLGSEHIESSVLVTIEPSEAIPAPGPVLPVRIESSSSTVAEGQTLDLNCVVAGQAHAQVTWYKRGGSLPARHQVRGSRLYIFQASPVDAGEYVCRAGNGQEATITVKVTGNQGANFAYPPGSTPRIRIESSSSHVAEGQTLDLNCVVQGQAHAQVTWHKRGGSLPARHQTHGSLLRLYQVSPIDSGEYVCRVEGGPVPLESSVLVTIEPAGSGPALGVTPPVRIETSPSHVAEGQSLDLNCLVAGQAHPQISWHKRGGSLPARHQVHGSRLRLLQVTPADSGEYVCRVVSGSGTHEASVLVTIQQRLIPSHSQSVVHPVRIESSSPSLANGHTLDLNCLVASHAPHTITWYKRGGSLPSRHQIVGSRLRIPQVTPADSGEYVCHVSNGVGSQETSLIVNIESRGPSHVPSVSPPMRIETSSPIVVEGQTLDLNCVVVGQPQATITWYKRGGSLPSKHQAHGSRLRLHQVSVADSGEYVCRANNNIDAQETSIMISVSPSNSSPSAPAGATPIRIESSSSNVAEGQTVDLNCVVPGHAHAQVTWHKRGGSLPARHQAYGSRLRLHQVSPADSGEYVCRVLSSSGPLEASVLVSITAPTTNAHVPGGVPPIRIETSSSRVAEGQTLDLSCVVPGQAHAQVTWHKRGGSLPAGHQVHGHILRLNHVSPADSGEYSCQVTGSSGTLEASVLVNIESTNPRPIPAPGLAQPIYIESSSSHVAEGQTLDLNCVVPGQAHAQVTWHKRGGSLPARHQTHGSLLRLHHISPADSGEYVCQVAGSSRPEHEASFTVTVPPSAGSSYRLRSPVISIEPPSLTVQQGQDASFKCLIHEGATPINLEWKTRNQELEDNVHISPNGSIITIVGTRPSNHGAYRCVASNAYGVAQSVVNLSVHGSPTVSVLPEGPVHVKMGKDITLECVSAGEPRSSPRWTRLGTPVKLEPRIYGLMNSHAMLKISSAKPSDAGTYVCLAQNALGKAQKQVEVIVDTGTVAPGAPRVQVEEAELTLEAGHTATLHCSATGNPPPTIHWSKLRAPLPWQHRVEGNTLVIPRVAQQDSGQYICNATNSAGHTEATVVLHVESPPYATIIPEHTSVQPGKPVQLQCLAHGTPPLTFQWSRVAGILPERAVARNELLHLELTGPADSGRYRCQVSNKVGSAEAFAQVLVQGPSGDLPETSIPVGSTPTVQVTPQLETKNVGASVEFHCAVPNERGTHLRWLKEGGQLPPGHSVQDGVLRIQNLDQSCQGTYVCQAHGPWGQAQASAQLIVQALPSVLINVRTSVHSVVVGHSVEFECLALGDPKPQVTWSKVGGHLRPGIVQSGSVIRIAHVELTDAGQYRCAATNAAGTTQSHVLLLVQALPQISTPPEVRVPAGSAAVFPCMASGYPTPAITWSKVDGDLPPDSRLENNMLMLPSVRPQDAGTYVCTATNRQGKVKAFAYLQVPERVVPYFTQTPYSFLPLPTIKDAYRKFEIKITFRPDSADGMLLYNGQKRIPGSPTNLANRQPDFISFGLVGGRPEFRFDAGSGMATIRHPTPLALGQFHTVTLLRSLTHGSLIVGNSAPVNGTSQGKFQGLDLNEELYLGGYPDYGAIPKAGLSSGFVGCVRELRIQGEEIIFHDLNLTTHGISHCPTCQDRPCQNGGQCHDSESSSYTCVCPAGFTGSRCEHSQALHCHPEACGPDATCVNRPDGRGYTCRCHLGRSGMRCEEGVTVTTPSMSGTGSYLALPALTNTHHELRLDVEFKPLAPDGILLFSGGKSGPVEDFVSLAMVGGHLEFRYELGSGLAVLRSHEPLALGRWHRVSAERLNKDGSLRVDGGRPVLRSSPGKSQGLNLHTLLYLGGVEPSVQLSPATNMSAHFRGCVGEVSVNGKRLDLTYSFLGSQGVGQCYDSSPCERQPCRNGATCMPAGEYEFQCLCQDGFKGDLCEHEENPCQLQEPCLNGGTCWGAHCLCLPGFSGPRCQQGAGYGVVESDWHLEGSGGNDAPGQYGAYFHDNGFLGLPGNIFSRR

SEQ ID NO: 13 - protein, 429 aa, Cricetulus griseus
MSILKVLAREIFDSRGNPTVEVDLYTSKGLFRAAVPSGASTGIYEALELRDNDKTRYMGKGVSKAVEHINKTIGPALVSKKLDVVDQEKIDKLMIEMDGTENKSKFGANAILGVSLAVCKAGAAEKGVPLYRHIADLAGNPEVILPVPAFNVINGGSHAGNKLAMQEFMILPVGASTFREAMRIGAEVYHNLKNVIKEKYGKDATNVGDEGGFAPNILENKEALELLKTAIGKAGYTEQVVIGMDVAASEFFRSGKYDLDFKSPDDPSRHITPDQLADLYKSFIQEYPVVSIEDPFDQDDWEAWKNFTASAGIQVVRDDLTVTNPKRIAKAVSEKSCNCLLLKVNQIGSVTESLQACKLAQSNGWGVMVSHRSGETEDTFIADLVVGLCTGQIKTGAPCRSERLAKYNQILRIEEELGSKAKFAGRSWS

SEQ ID NO: 14 - protein, 474 aa, Cricetulus griseus
MESKALLLVALGVWLQSLTASQGGVAAADGGRDFTDIESKFALRTPDDTAEDNCHLIPGIAESVSNCHFNHSSKTFVVIHGWTVTGMYESWVPKLVAALYKREPDSNVIVVDWLYRAQQHYPVSAGYTKLVGNDVARFINWMEEEFNYPLDNVHLLGYSLGAHAAGVAGSLTNKKVNRITGLDPAGPNFEYAEAPSRLSPDDADFVDVLHTFTRGSPGRSIGIQKPVGHVDIYPNGGTFQPGCNIGEAIRVIAERGLGDVDQLVKCSHERSIHLFIDSLLNEENPSKAYRCNSKEAFEKGLCLSCRKNRCNNVGYEINKVRAKRSSKMYLKTRSQMPYKVFHYQVKIHFSGTESDKQLNQAFEISLYGTVAESENIPFTLPEVSTNKTYSFLIYTEVDIGELLMMKLKWKSDSYFSWSDWWSSPGFVIEKIRVKAGETQKKVIFCAREKVSHLQKGKDSAVFVKCHDKSLKKSG

SEQ ID NO: 15 - protein, 466 aa, Cricetulus griseus
MSTRSVSSSSYRRMFGGPGTSSRPSSNRSYVTTSTRTYSLGSALRPSTSRSLYSSSPGGAYVTRSSAVRLRSSMPGVRLLQDSVDFSLADAINTEFKNTRTNEKVELQELNDRFANYIDKVRFLEQQNKILLAELEQLKGQGKSRLGDLYEEEMRELRRQVDQLTNDKARVEVERDNLAEDIMRLREKLQEEMLQREEAESTLQSFRQDVDNASLARLDLERKVESLQEEIAFLKKLHDEEIQELQAQIQEQHVQIDVDVSKPDLTAALRDVRQQYESVAAKNLQEAEEWYKSKFADLSEAANRNNDALRQAKQESNEYRRQVQSLTCEVDALKGTNESLERQMREMEENFALEAANYQDTIGRLQDEIQNMKEEMARHLREYQDLLNVKMALDIEIATYRKLLEGEESRISLPLPNFSSLNLRETNLESLPLVDTHSKRTLLIKTVETRDGQVINETSQHHDDLE

SEQ ID NO: 16 - protein, 654 aa, Cricetulus griseus
MKFPMVAAALLLLCAVRAEEEDKKEDVGTVVGIDLGTTYSCVGVFKNGRVEIIANDQGNRITPSYVAFTPEGERLIGDAAKNQLTSNPENTVFDAKRLIGRTWNDPSVQQDIKFLPFKVVEKKTKPYIQVDIGGGQTKTFAPEEISAMVLTKMKETAEAYLGKKVTHAVVTVPAYFNDAQRQATKDAGTIAGLNVMRIINEPTAAAIAYGLDKREGEKNILVFDLGGGTFDVSLLTIDNGVFEVVATNGDTHLGGEDFDQRVMEHFIKLYKKKTGKDVRKDNRAVQKLRREVEKAKRALSSQHQARIEIESFFEGEDFSETLTRAKFEELNMDLFRSTMKPVQKVLEDSDLKKSDIDEIVLVGGSTRIPKIQQLVKEFFNGKEPSRGINPDEAVAYGAAVQAGVLSGDQDTGDLVLLDVCPLTLGIETVGGVMTKLIPRNTVVPTKKSQIFSTASDNQPTVTIKVYEGERPLTKDNHLLGTFDLTGIPPAPRGVPQIEVTFEIDVNGILRVTAEDKGTGNKNKITITNDQNRLTPEEIERMVNDAEKFAEEDKKLKERIDTRNELESYAYSLKNQIGDKEKLGGKLSSEDKETMEKAVEEKIEWLESHQDADIEDFKAKKKELEEIVQPIISKLYGSAGPPPTGEEDTSEKDEL

SEQ ID NO: 17 - protein, 646 aa, Cricetulus griseus
MSKGPAVGIDLGTTYSCVGVFQHGKVEIIANDQGNRTTPSYVAFTDTERLIGDAAKNQVAMNPTNTVFDAKRLIGRRFDDAVVQSDMKHWPFMVVNDAGRPKVQVEYKGEAKSFYPEEVSSMVLTKMKEIAEAYLGKTVTNAVVTVPAYFNDSQRQATKDAGTIAGLNVLRIINEPTAAAIAYGLDKKVGAERNVLIFDLGGGTFDVSILTIEDGIFEVKSTAGDTHLGGEDFDNRMVNHFIAEFKRNDKKDISENKRAVRRLRTACERAKRTLSSSTQASIEIDSLYEGIDFYTSITRARFEELNADLFRGTLDPVEKALRDAKLDKSQIHDIVLVGGSTRIPKIQKLLQDFFNGKELNKSINPDEAVAYGAAVQAAILSGDKSENVQDLLLLDVTPLSLGIETAGGVMTVLIKRNTTIPTKQTQTFTTYSDNQPGVLIQVYEGERAMTKDNNLLGKFELTGIPPAPRGVPQIEVTFDIDANGILNVSAVDKSTGKENKITITNDKGRLSKEDIERMVQEAEKYKAEDEKQRDKVSSKNSLESYAFNMKATVEDEKLQGKINDEDKQKILDKCNEIISWLDKNQTAEKEEFEHQQKELEKVCNPIITKLYQSAGGMPGGMPGGFPGGGAPPSGGASSGPTIEEVD

SEQ ID NO: 18 - protein, 216 aa, Cricetulus griseus
MLRISGRNMKVLFAAALIVGSVVFLLLPGPSVANDKKKGPKVTVKVFFDLHIGDEPVGRVTFGLFGKTVPKTVDNFVALATGEKGFGYKNSKFHRVIKDFMIQGGDFTRGDGTGGKSIYGERFPDENFKLKHYGPGWVSMANAGKDTNGSQFFITTVKTSWLDGKHVVFGKVLEGMDVVRKVESTKTDSRDKPLKDVIIADCGKIEVEKPFAIAKE

SEQ ID NO: 19 - protein, 858 aa, Cricetulus griseus
MVNFTVDQIRAIMDKEANIRNMSVIAHVDHGKSTLTDSLVCKAGIIASARAGETRFTDTRKDEQERCITIKSTAISLFYELSENDLNFIKQSKDGSGFLINLIDSPGHVDFSSEVTAALRVTDGALVVVDCVSGVCVQTETVLRQAIAERIKPVLMMNKMDRALLELQLEPEELYQTFQRIVENVNVIISTYGEGESGPMGNIMIDPVLGTVGFGSGLHGWAFTLKQFAEMYVAKFAAKGEGQLGPAERAKKVEDMMKKLWGDRYFDPANGKFSKSANSPDGKKLPRTFCQLILDPIFKVFDPIMNFRKEETAKLIEKLDIKLDSEDKDKEGKPLLKAVMRRWLPAGDALLQMITIHLPSPVTAQKYRCELLYEGPPDDEAAMGIKSCDPKGPLMMYISKMVPTSDKGRFYAFGRVFSGVVSTGLKVRIMGPNYTPGKKEDLYLKPIQRTILMMGRYVEPIEDVPCGNIVGLVGVDQFLVKTGTITTFEHAHNMRVMKFSVSPVVRVAVEAKNPADLPKLVEGLKRLAKSDPMVQCIIEESGEHIIAGAGELHLEICLKDLEEDHACIPIKKSDPVVSYRETVSEESNVLCLSKSPNKHNRLYMKARPFPDGLAEDIDKGEVSARQELKARARYLAEKYEWDVAEARKIWCFGPDGTGPNILTDITKGVQYLNEIKDSVVAGFQWATKEGALCEENMRGVRFDVHDVTLHADAIHRGGGQIIPTARRCLYASVLTAQPRLMEPIYLVEIQCPEQVVGGIYGVLNRKRGHVFEESQVAGTPMFVVKAYLPVNESFGFTADLRSNTGGQAFPQCVFDHWQILPGDPFDNSSRGSQVVAETRKRKGLKEGIPALDNFLDKL

SEQ ID NO: 20 - protein, 339 aa, Cricetulus griseus
MWWSLIPLSCLLALASAHNKPSFHPLSDDLINYINKRNTTWQAGRNFHNVDISYLKRLCGTIMGGPKLPERVAFAEDMELPENFDAREQWSNCPTIKQIRDQGSCGSCWAFGAVGAMSDRLCIHTNGHVNVEVSAEDLLTCCGSQCGDGCNGGYPSGAWNFWIKKGLVSGGLYNSHVGCLPYTIPPCEHHVNGSRPQCTGEGDTPKCTKSCEAGYSPSYKEDKHYGYTSYSVSNNEKEIMAEIYKNGPVEGAFTVFSDFLTYKSGVYKHEAGDIMGGHAIRILGWGVENSVPYWLVANSWNVDWGDNGLFKILRGEDHCGIESEIVAGIPRTDLYWGRF

SEQ ID NO: 21 - protein, 733 aa, Cricetulus griseus
MPEETQTQDQPMEEEEVETFAFQAEIAQLMSLIINTFYSNKEIFLRELISNSSDALDKIRYESLTDPSKLDSGKELHINIIPNKQDRTLTIVDTGIGMTKADLINNLGTIAKSGTKAFMEALQAGADISMIGQFGVGFYTAYLVAEKVTVITKHNDDEQYAWESSAGGSFTVRTDTGEPMGRGTKVILHLKEDQTEYMEERRIKEIVKKHSQFIGYPITLFVEKERDKEVSDDEAEEKEDKEEEKEKEEKGIDDKPEIEDVGSDEEEEEKKDGDKKKKKKIKEKYIDQEELNKTKPIWTRNPDDITNEEYGEFYKSLTNDWEEHLAVKHFSVEGQLEFRALLFVPRRAPFDLFENRKKKNNIKLYVRRVFIMDNCEELFPEYLNFIRGVVDSEDLPLNISREILQQSKILKVIRKNLVRKCLELFHELAEDKENYKKFYEQFSKNIKLGIHEDSQNRKKLSELLRYYTSASGDEMVSLKDYCTRMKENQKHIYFITGETKDQVANSAFVERLRKHGLEVIYMIEPIDEYCVQQLKEFEGKTLVSVTKEGLELPEDEEEKKKQEEKKTKFENLCKIMKDILEKKVEKVVVSNRLVTSPCCIVTSTYGWTANMERIIKAQALRDNSTMGYMAAKKHLEINPDHSIIETLRQKAEADKNDKSVKDLVILLYETALLSSGFSLEDPQTHANRIYRMIKLGLGIDEDDPTVDDTSAAVTEEMPPLEGDDDTSRMEEVD

SEQ ID NO: 22 - protein, 221 aa, Cricetulus griseus
MKFWGQEKKEVVPPYTIVYFPVRGRCEAMRILLADQGQSWKEEVVTVETWRKGSLKSTCLYGQLPKFEDGDLTLYQSNAILRHLGRSLGLYGKDQREAALVDMVNDGVEDLRCKYITLIYTKYEEGKDDYVKALPGHLKPFETLLSQNQGGKAFIVGDQISFVDYNLLDLLLIHQVLAPGCLDNFPLLSAYVARLSARPKIKAFLSSPDHVNRPINGNGKQ

SEQ ID NO: 23 - protein, 462 aa, Cricetulus griseus
MGKEKTHINIVVIGHVDSGKSTTTGHLIYKCGGIDKRTIEKFEKEAAEMGKGSFKYAWVLDKLKAERERGITIDISLWKFETSKYYVTIIDAPGHRDFIKNMITGTSQADCAVLIVAAGVGEFEAGISKNGQTREHALLAYTLGVKQLIVGVNKMDSTEPPYSQKRYEEIVKEVSTYIKKIGYNPDTVAFVPISGWNGDNMLEPSANMPWFKGWKVTRKDGSASGTTLLEALDCILPPTRPTDKPLRLPLQDVYKIGGIGTVPVGRVETGVLKPGMVVTFAPVNVTTEVKSVEMHHEALSEALPGDNVGFNVKNVSVKDVRRGNVAGDSKNDPPMEAAGFTAQVIILNHPGQISAGYAPVLDCHTAHIACKFAELKEKIDRRSGKKLEDGPKFLKSGDAAIVDMVPGKPMCVESFSDYPPLGRFAVRDMRQTVAVGVIKAVDKKAAGAGKVTKSAQKAQKAK

SEQ ID NO: 24 - protein, 278 aa, Cricetulus griseus
MGGSSYTCSCLPGFSGDGRACQGLSTVAPPIHQRPVVPTAVIPLPPGTHLLFAQTGKIERLPLEGNTMKKTEAKAFLHIPAKVIIGLAFDCVDKVVYWTDISEPSIGRASLHGGEPTTIIRQDLGSPEGIALDHLGRNIFWTDSQLDRIEVARMDGTQRRVLFDTGLVNPRGIVTDSVGGPLKIVQAKRCMFTLYALVLCRNSVIAMDLAISKEMDAFHPHKQTRLYGITIALSQCPQGHNYCSVNNGGCTHLCLPTPGSRTCRCPDNTLGVDCIERK

SEQ ID NO: 25 - protein, 623 aa, Cricetulus griseus
MEGYHKPDQQKLQALKDTANRLRISSIQATTAAGSGHPTSCCSAAEIMAVLFFHTMRYKALDPRNPHNDRFVLSKGHAAPILYAVWAEAGFLPETELLNLRKISSDLDGHPVPKQAFTDVATGSLGQGLGAACGMAYTGKYFDKASYRVYCMLGDGEVSEGSVWEAMAFAGIYKLDNLVAIFDVNRLGQSDPAPLQHQLDVYQKRCEAFGWHAIIVDGHSVEELCKAFGQAKHQPTAIIAKTFKGRGITGIEDKESWHGKPLPKNMADQIIQEIYSQIQSKKKILATPPQEDAPSVDIANIRMPTPPSYKVGDKIATRKAYGQALAKLGHASDRIIALDGDTKNSTFSDIFKKEHPDRFIECYIAEQNMVSIAVGCATRNRTVPFCSTFAAFFTRAFDQIRMAAISESNINLCGSHCGVSIGEDGPSQMALEDLAMFRSIPMSTVFYPSDGVATEKAVELAANTKGICFIRTSRPENAIIYSNNEDFQVGQAKVVLKSKDDQVTVIGAGVTLHEALAAAELLKKEKISIRVLDPFTIKPLDRKLILECARATKGRILTVEDHYYEGGIGEAVSAAVVGEPGVTVTRLAVSQVPRSGKPAELLKMFGIDKDAIVQAVKGLVTKG

SEQ ID NO: 26 - protein, 430 aa, Cricetulus griseus
MQIFVKTLTGKTITLEVEPSDTIENVKAKIQDKEGIPPDQQRLIFAGKQLEDGRTLSDYNIQKESTLHLVLRLRGGMQIFVKTLTGKTITLEVEPSDTIENVKAKIQDKEGIPPDQQRLIFAGKQLEDGRPLSDYNIQKESTLHLVLRLRGGMQIFVKTLTGKTITLEVEPRDTIENVKAWIQDKEGIPPDQQRLIFAGKQLEDGRPLSDYNIQKESTLHLVLRLRGGMQIFVKTLTGKTITLEVEPRDTIENVKAWIQDKEGIPPDQQRLIFAGKQLEDGRPLSDYNIQKESTLHLVLRLRGGMQIFVKTLTGKTITLEVEPRDTIENVKAWIQDKEGIPPDQQRLIFAGKQLEDGRPLSDYNIQKESTLHLVLRLRGGMQIFVKTLTGKTITLEVEPSNTIKKSKQEDGRTFLTTLSRKSTPCACSWA

SEQ ID NO: 27 - protein, 268 aa, Cricetulus griseus
MASTDNLCGHVIPEAGKTELSARPGPQRNGAVLVGLLQCGRAHISSQTLPHPAVIAEGKLPVLLLGRSSELRPGEFVVAIGSPFSLQNTVTTGIVSTTQRGGKELGLRNSDMDYIQTDAIINDGEVIGINTLKVTAGISFAIPSDKIKKFLTESHDRQAKGKAVTKKKYIGIRMMSLTSSSKAKELKDRHRDFPDVLSGAYIIEVIPDTPAEAGGLKENDVIISINGQSVVTANDVSDVIKKENTLNMVVRRGNEDIMLTVIPEEIDP

SEQ ID NO: 28 - protein, 723 aa, Cricetulus griseus
MLDASGWKPAAWTWVLLLQLLLAGPGDCLSRQELFPFGPGQGDLELEAGDDVVSPALELIGELSFYDRSDITSVYVTTNGIIAMSEPPARESHPGTFPPSFGSVAPFLADLDTTDGLGNVYYREDLSPSIMQMAAEYVQRGFPEVPFQPTSVVVVTWESVAPYEGPSGSSAQEGKRNTFQAVLASSNSSSYAIFLYPEDGLQFFTTFSKKDENQVPAMVGFSQGLVGFLWRSDGAYNIFANDRESIENLAKSSNAGHQGVWVFEIGSPATAKGVVSADVNLGLDDDGSDYEDEEYDLATSHLGLEDMATQPFPSPSPRRGNTHPHDVPRVLSPSYEATERPHGIPTERTRTFQLPAERFHQQHPQVIDVDEVEETGIVFSYNIGSQQTCANNRHQCSVHAECRDYATGFCCRCVANYTGNGRQCVAEGSPQRVNGKVKGRIFVGNSQVPVVFENTDLHSYVVMNHGRSYTAISTIPETVGYSLLPLAPIGGIIGWMFAVEQNGFKNGFSITGGEFTRQAEVTFLGHPGKLVLKQHFSGIDEHGHLTINTELDGRVPQIPYGSSVHIEPYTELYHYSSSVITSSSTREYTVTEPDPDGTAPSHTHVYQWRQTITFQECVHDDSRPALPSTQQLSVDSVFVLYNQEERILRYALSNSIGPVREGSPDALQNPCYIGTHGCDSNAACRPGPGTQFTCECSIGFRGDGQTCYGIVFWSEVWGSGLLV

SEQ ID NO: 29 - protein, 1475 aa, Cricetulus griseus
MAVRPMRRCLQALVLCFSLGAMAVVASKPGAGCPSRCLCFRTTVRCMHLLLEAVPAVSPQTSILDLRFNRIREIQPGAFRRLRNLNTLLLNNNQIKRIPSSAFEDLENLKYLYLYKNEIQSIDRQAFKGLASLEQLYLHFNQIETLDPESFQHLPKLERLFLHNNRITHLVPGTFSHLESMKRLRLDSNALHCDCEILWLADLLKTYAQSGNAQAAATCEYPRRIQGRSVATITPEELNCERPRITSEPQDADVTSGNTVYFTCRAEGNPKPEIIWLRNNNELSMKTDSRLNLLDDGTLMIQNTQEADEGVYQCMAKNVAGEAKTHEVTLRYLGSPARPTFVIQPQNTEVLVGESVTLECSATGHPLPQITWTRGDRTPLPTDPRVTITPSGGLYIQNVEQSDSGEYTCFASNSVDSIHATAFIIVQALPQFTVTPQSRVVIEGQTVDFQCEAKGYPQPVIAWTKGGSQLSVDRRHLVLSSGTLRISGVALHDQGQYECQAVNIIGSQKVVAHLTVQPRVTPVFASIPSDMTVEVGTNVQLPCSSQGEPEPAITWNKDGVQVTESGKFHISPEGFLTINDVGTADAGRYECVARNTIGYSSVSMVLSVNVPDVSRNGDPYVATSIVEAIATVDRAINSTRTHLFDSRPHSPNDLLALFRYPRDPYTVGQARAGEIFERTLQLIQDHVQHGLMVDLNGTSYHYNDLVSPQYLSLIANLSGCTAHRRVNNCSDMCFHQKYRTHDGTCNNLQHPMWGASLTAFERLLKAVYENGFNTPRGINPQRQYNGHVLPMPRLVSTTLIGTEVITPDEQFTHMLMQWGQFLDHDLDSTVVALSQARFSDGQHCSNVCSNDPPCFSVMIPPNDPRVRSGARCMFFVRSSPVCGSGMTSLLMNSVYPREQINQLTSYIDASNVYGSTDHEARSIRDLASHRGLLRQGIVQRSGKPLLPFATGPPTECTRDENESPIPCFLAGDHRANEQLGLTSMHTLWFREHNRIAAELLKLNPHWDGDTVYHETRKIVGAEIQHITYRHWLPKILGEVGMKMLGEYRGYDPSVNAGIFNAFATAAFRFGHTLINPLLYRLDENFEPIPQGHVPLHKAFFSPFRIVNEGGIDPLLRGLFGVAGKMRVPSQLLNTELTERLFSMAHTVALDLAAINIQRGRDHGIPPYHDYRVYCNLSAAYTFEDLKNEIKSPEIREKLQRLYGSTLNIDLFPALMVEDLVPGSRLGPTLMCLLSTQFRRLRDGDRLWYENPGVFSPAQLTQLKQTSLARILCDNSDNITRVQQDVFRVAEFPHGYSNCEDIPRVDLRVWQDCCEDCRTRGQFNAFSYHFRGRRSLEFSYEEDKPTKRARRQKALSVKYGKHLSNATSATHKHLEGPATNDLKKFIMEMQTVITDLRKQITSLESRLSTTECVDDSGESHSNNTKWKKDRCTVCECKKGQVTCFVEACQPAACPEPVKLEGACCPVCLRDTEEEKP

SEQ ID NO: 30 - protein, 245 aa, Cricetulus griseus
MDKNELVQKAKLAEQAERYDDMAACMKSVTEQGAELSNEERNLLSVAYKNVVGARRSSWRVVSSIEQKTEGAEKKQQMAREYREKIEAELRDICNDVLSLLEKFLIPNASQAESKVFYLKMKGDYYRYLAEVAAGDDKKGIVDQSQQAYQEAFEISKKEMQPTHPIRLGLALNFSVFYYEILNSPEKACSLAKTAFDEAIAELDTLSEESYKDSTLIMQLLRDNLTLWTSDTQGDEAEAGEGGEN

SEQ ID NO: 31 - protein, 475 aa, Cricetulus griseus
MFRAALSPLLLLLLVSWASRGEAAPDQDEIDCLPGLDKQPDFQQYSGYLRASDNKHFHYWFVESQKDPKNSPVVLWLNGGPGCSSLDGFLTEHGPFLIQPDGITLKYNPYSWNLIANMLYIESPAGVGFSYSDDKTYVTNDTEVAQNNYEALKDFFRLFPEYKDNKLFLTGESYAGIYIPTLAVLVMQDPSMNLQGLAVGNGLSSYEQNDNSLVYFAYYHGLLGNRLWTLLQTHCCSQNKCNFYDNKDPECVNNLLEVSRIVSNSGLNIYNLYAPCAGGVPGTDRYEDTLVIHDFGNIFTRLPLKRKYHQTLLLRSGDKARMDPPCTNTTAPSTYLNNPYVRKALHIPEKLPRWDMCNLVVNLQYRRLYQSMNSQYLKLLSSQKYQILLYNGDVDMACNFMGDEWFVDSLNQKMEVQRRPWLVDYGESGEQVAGFVKEFSHITFLTIKGAGHMVPTDKPRAAFTMFSRFLNKEPY

SEQ ID NO: 32 - protein, 164 aa, Cricetulus griseus
MVNPTVFFDISADGEPLGRVSFELFADKVPKTAENFRALSTGEKGFGYKGSSFHRIIPGFMCQGGDFTRHNGTGGRFIYGEKFEDENFILKHTGPGILSMANAGPNTNGSQFFICTAKTEWLDGKHVVFGKVKEGMNIVEAMERFGSRNGKTSKKITISDCGQL

SEQ ID NO: 33 - protein, 740 aa, Cricetulus griseus
MREEKRRGEEEREEKQKKKSREKRSRECLTNPIRLLLEYTDSSYEEKKYTMGDAPDFDRSQWLNEKFKLGLDFPNLPYLIDGSHKITQSNAILRYIARKHNLCGETEEERIRVDIVENQAMDTRMQLIMLCYNPDFEKQKPEFLKTIPEKMKMYSEFLGKRPWFAGDKGLKKISAYMKTSRFLRRPIFSKMAQWSNKSQWLNEKFKLGLDFPNLPYLIDGSHKITQSNAILRYIARKHNLCGETEEERIRVDILENQAMDTRMQLAMVCYSPDFEKRKPEYLEGLPEKMKLYSEFLGKRPWFAGDKVTYADFLVYDILDQHRIFAPKCLDSFPNLKDFLARFELPYLIDGSHKVTQSNAILRYIARKHNLCGETEEERIRVDTLENQVMDTRIQLMIVCCNPDFVTYVDFLAYDILDQYQMFEPNCLDAFPNLKDFLARFEGLKKISAYMKTNRFLPSPLCLKQVTWRNNHGELGSMVPGSAHLGAGQSRSGTAQSPRCALLLQVESSARGLTAVSKAGTEIMPVTLGYWDIRGLGHAIRLLLEYTETSYEEKRYAMGDAPDYDRSQWLNDKFKLGLDFPNLPYLIDGPYKVTQSNAILRYLGRKHNLCGETEEERVRVDILEKQVMDTRIQMGTLCYSPDFEKRKPEFLKGLPDHLKLYSEFLGTSPWFAGDKITFADFLVYDVLDQHQMFEPKCLDAFPNLRDFVARFEGLKKISAYMKTNRFLPSPLYLKQATWGNK

SEQ ID NO: 34 - protein, 803 aa, Cricetulus griseus
MRVLWVLGLCCVLLTFGFVRADDEVDVDGTVEEDLGKSREGSRTDDEVVQREEEAIQLDGLNASQIRELREKSEKFAFQAEVNRMMKLIINSLYKNKEIFLRELISNASDALDKIRLISLTDENALAGNEELTVKIKCDKEKNLLHVTDTGVGMTREELVKNLGTIAKSGTSEFLNKMTEAQEDGQSTSELIGQFGVGFYSAFLVADKVIVTSKHNNDTQHIWESDSNEFSVIADPRGNTLGRGTTITLVLKEEASDYLELDTIKNLVRKYSQFINFPIYVWSSKTETVEEPLEEDEAAKEEKEESDDEAAVEEEEEEKKPKTKKVEKTVWDWELMNDIKPIWQRPSKEVEEDEYKAFYKSFSKESDDPMAYIHFTAEGEVTFKSILFVPTSAPRGLFDEYGSKKSDYIKLYVRRVFITDDFHDMMPKYLNFVKGVVDSDDLPLNVSRETLQQHKLLKVIRKKLVRKTLDMIKKIADEKYNDTFWKEFGTNIKLGVIEDHSNRTRLAKLLRFQSSHHSTDITSLDQYVERMKEKQDKIYFMAGSSRKEAESSPFVERLLKKGYEVIYLTEPVDEYCIQALPEFDGKRFQNVAKEGVKFDESEKTKENREATEKEFEPLLNWMKDKALKDKIEKAVVSQRLTESPCALVASQYGWSGNMERIMKAQAYQTGKDISTNYYASQKKTFEINPRHPLIRDMLRRVKEDEDDKTVLDLAVVLFETATLRSGYLLPDTKAYGDRIERMLRLSLNIDPEAQVEEEPEEEPEDTTEDTEQDEEEEVDAGTEEEEEEEQETAKESTAEKDEL

SEQ ID NO: 35 - protein, 417 aa, Cricetulus griseus
MSLSNKLTLDKLDVKGKRVVMRVDFNVPMKNNQITNNQRIKAAVPSIKFCLDNGAKSVVLMSHLGRPDGVPMPDKYSLEPVAAELKSLLGKDVLFLKDCVGPEVENACANPAAGTVILLENLRFHVEEEGKGKDASGNKIKAEPAKIDAFRASLSKLGDVYVNDAFGTAHRAHSSMVGVNLPQKAGGFLMKKELNYFAKALESPERPFLAILGGAKVADKIQLINNMLDKVNEMIIGGGMAFTFLKVLNNMEIGTSLYDEEGAKIVKDLMAKAEKNGVKITLPVDFVTADKFDENAKTGQATVASGIPAGWMGLDCGTESSKKYAEAVARAKQIVWNGPVGVFEWEAFARGTKSLMDEVVKATSRGCITIIGGGDTATCCAKWNTEDKVSHVSTGGGASLELLEGKVLPGVDALSNV

SEQ ID NO: 36 - protein, 369 aa, Cricetulus griseus
MSPLWLLTLLLALSQALPFEQKGFWDFTLDDGLLMMHDEEASGSDTTSGVPDLDSLTPTFSAMCPFGCHCHLRVVQCSDLGLKTVPKEISPDTTLLDLQNNDISELRKDDFKGLQHLYALVLVNNKISKIHEKAFSPLRKLQKLYISKNHLVEIPPNLPSSLVELRIHDNRIRKVPKGVFSGLRNMNCIEMGGNPLENSGFEPGAFDGLKLNYLRISEAKLTGIPKDLPETLNELHLDHNKIQAIELEDLLRYSKLYRLGLGHNQIRMIENGSLSFLPTLRELHLDNNKLSRVPAGLPDLKLLQVVYLHSNNITKVGINDFCPMGFGVKRAYYNGISLFNNPVPYWEVQPATFRCVTDRLAIQFGNYKK

SEQ ID NO: 37 - protein, 438 aa, Cricetulus griseus
MCRMIWKAAVLLSLALGAGALAVGVDDPEDAGKHWVVIVAGSNGWYNYRHQADACHAYQIIHRNGIPDEQIIVMMYDDIANSEDNPTPGIVINRPNGTDVYAGVLKDYTGEDVTPENFLAVLRGDAEAVKGKGSGKVLRSGPQDHVFVYFTDHGATGLLVFPNEDLHVKDLNKTIRYMYEHKMYQKMVFYIEACESGSMMNHLPNDINVYATTAANPHESSYACYYDEERNTYLGDWYSVNWMEDSDVEDLTKETLHKQYHLVKSHTNTSHVMQYGNKSISTMKVMQFQGMKHSTSSPISLPPVTRLDLTPSPEVPLTILKRKLMSTNDLKQSQNLVGQIQRLLDARHVIEKSVHKIVSLLAGFGETAERLLSERAVLMAHDCYQEAVTHFRTHCFNWHSPTYEYALRHLYVLANLCEKPYPIDRIKMAMDKVCLSHY

SEQ ID NO: 38 - protein, 574 aa, Cricetulus griseus
MALLWLFSLWLLVPGTQGTEDGDMRLVNGASASEGRVEIFYRGQWGTVCDNLWNILDANVVCRALGYENATRALGRAAFGPGQGPVMLDEVECAGTEPSLANCSSLGWLKSRCGHEKDAGVVCSNETESMHILDLSGDLPDALGQIFDSQQGCDLFIQVTGQGHRDLTLCAHKLILNTNSEAQALWHAEGSSVIMRVDVDCMPVVRDFLRYFYSRRIEVTMSSVKCLHKLASAYGATQLRDYCSRLFATLLPEDPTFHTPLELYEYAQATRDSVLEELCVQFLAWNFEPLTQVEAWLSVPTTLLQALLSKSELAVSSELDLLKAVDQWSAESGASHAEVEGLVEQVRFPMMLPQQLFELQFNLSLYQGHQALFQRKTMEALEFHTVPFPVLAKYRGLNLTENTYKPRLYTSSTWSTLVTDRSSRSQGAQVYGYYSYGYDSVSRYSPYRSFQTPQHPSFLFTDKLISWSATYLPTVQSCWNYGFSCTSDELPVLGLTKSSYSEPMIGYENKALMLCGGHSVVDVTNFAGSKAPVPSALDTNSSKISSLFPCTSGAFSGFRVVIRPFYLTNSTDLD

SEQ ID NO: 39 - protein, 585 aa, Cricetulus griseus
MAAPMDRSPGGRAVRALRLALALASLTEVLLNCPAGALPTQGPGRRRQNLDPPVSRVRSVLLDAASGQLRLVDGIHPYAVAWANLTNAIRETGWAYLDLGTNGSYNDSLQAYAAGVVEASVSEELIYMHWMNTMVNYCGPFEYEVGYCEKLKSFLEINLEWMQREMELSQDSPYWHQVRLTLLQLKGLEDSYEGRLTFPTGRFTIKPLGFLLLQIAGDLEDLEQALNKTSTKLSLGSGSCSAIIKLLPGARDLLVAHNTWNSYQNMLRIIKKYQLQFRQGPQEAYPLIAGNNLVFSSYPGTIFSGDDFYILGSGLVTLETTIGNKNPALWKYVQPQGCVLEWIRNIVANRLALDGATWADIFKQFNSGTYNNQWMIVDYKAFIPNGPSPGSRVLTILEQIPGMVVVADKTEDLYKTTYWASYNIPFFEIVFNASGLQDLVAQYGDWFSYTKNPRAQIFQRDQSLVEDMNSMVRLIRYNNFLHDPLSLCEACIPKPNAENAISARSDLNPANGSYPFQALYQRPHGGIDVKVTSFSLAKRMSMLAASGPTWDQLPPFQWSLSPFRSMLHMGQPDLWTFSPISVPWD

SEQ ID NO: 40 - protein, 126 aa, Cricetulus griseus
MPEPVKSAPAPKKGSKKAVTKAQKKDGKKRKRSRKESYSVYVYKVLKQVHPDTGISSKAMGIMNSFVNDIFERIAGEASRLAHYNKRSTITSREIQTAVRLLLPGELAKHAVSEGTKAVTKYTSSK

SEQ ID NO: 41 - protein, 465 aa, Cricetulus griseus
MWGCRLGLLLLLLAGQAALEARRSRWRRELAPGLHLRGIRDAGGRYCQERDMCCRGRADDCALPYLGATCYCDLFCNRTVSDCCPDFWDFCLGVPPPFPPIQGCMHGGRIYPVFGTYWDNCNRCTCQEKGQWECDQEPCLVDPDMINAINRGNYGWQAGNHSAFWGMTLDEGIRYRLGTIRPSSSVMNMNEIYTALGRGEVLPRAFEASEKWPNLIQEPLDQGNCAGSWAFSTAAVASDRVSIHSMGHMTPILSPQNLLSCDTHHQQGCRGGRLDGAWWFLRRRGVVSDNCYPFVGREQNEAGTSSRCMMHSRAMGRGKRQATSRCPNGQVDSNDIYQVTPAYRLGSDEKEIMKELMENGPVQALMEVHEDFFLYQSGIYSHTPISQGRPEQYRRHGTHSVKITGWGEEKLPDGRTIKYWTAANSWGPWWGERGHFRIVRGTNECDIESFVLGVWGRVGMEDMGH

SEQ ID NO: 42 - protein, 1617 aa, Cricetulus griseus
MLIERSSDFGKTWGVYRYFAYDCESSFPGISTGPMKKVDDIICDSRYSDIEPSTEGEVIFRALDPAFKIEDPYSPRIQNLLKITNLRIKFVKLHTLGDNLLDSRMEIREKYYYAVYDMVVRGNCFCYGHASECAPVDGIDEAVEGMVHGHCMCRHNTKGLNCELCMDFYHDLPWRPAEGRNSNACKKCNCNEHSSSCHFDMAVFLATGNVSGGVCDDCQHNTMGRNCEQCKPFYYQHPERDVRDPNLCEPGSENGGICDGYTDFSAGLIAGQCRCKLHVEGERCDVCKEGFYGLSAEDPFGCKSCACNPLGTIPGGNPCDSETGYCYCKRLVTGQRCDQCLPQHWGLSNDLDGCRPCDCDLGGALNNSCSEDSGQCSCLPHMIGRQCNEVESGYYFTTLDHYIYEAEDANLGPGVIVVERQYIQDRIPSWTGPGFVRVPEGAYLEFFIDNIPYSMEYDILIRYEPQLPDHWEKAVITIQRPGKIPTSSRCGNTVPDDDNQVVSLSPGSRYIVLPRPVCFEKGMNYTVRLELPQYTASGSDVENPYTLIDSLVLMPYCKSLGIFTAGGSGDGEVTNSAWETFQRYRCLENSRSVVKTPMTDVCRNIIFSISAMIHQTGLACECDPQGSLSSVCDPNGGQCQCRPNVVGRACNRCAPGTFGFGPNGCKPCDCDLQGSVDAFCDAVTGQCHCFQGIYARQCDRCLPGHWGFPSCQPCQCNGHAEDCDTVTGECLSCQDYTTGHNCERCLAGYYGDPIIGSGDHCRPCPCPDGPNSGRQFARSCYQDPITLQLACVCDPGYIDFGGSCQPCQCHHNIDTTDPEACDKETGRCLKCLYHTEGDHCQLCQYGYYGDALRQDCRKCVCNYLGTVQEHCNGSDCHCDKATGQCLCLPNVIGQNCDQCAPNTWQLASGTGCESCNCNAAHSFGPSCNEFTGQCQCMPGFGGRTCSECQELFWGDPDVECRACDCDPRGIETPQCDQSTGQCVCVEGVEGPRCDKCTRGYSGVFPDCTPCHQCFALWDVIIGELTNRTHKFLEKAKALKISGVIGPYRETVDSVEKKVNEIKDILAQSPAAEPLKNIGNLFEEAEKLTKDVSEKMAQVEMRLSDTASQSNSTAGELAALQAEAKSLEKTVKELAEQLEFIKNSDIQGALDSVTKYFQISLEAEKRVNASTTDPNSTVEQSALTRDRVEDLMLERESQFKEEQEEQARLLDELAGKLQSLDLSAAAEMTCGTPPGADCSESECGGPNCRTDEGEKKCGGPGCGGLVTVAHSAWQKAMDFDRDVLSALAEVEQLSKMVSEAKVRADEAKQNAQDVLLKTNATKEKVDKSNEDLRNLIKQIRDFLTEDSADLDSIEAVANEVLKMEMPSTPQQLQNLTEDIRERVETLSQVEVILQQSAADIARAELLLEEAKRASKSATDVKVTADMVKEALEEAEKAQIAAEAAIKQADDDIQGTQNLLTSIESETAASEESLSNASQRISKLERNVEELKRKAAQNSGEAEYIEKVVYSVKQSADDVKKALDGELDEKYKKVESLIAQKTEESADARRKAELLQNEAKTLLAQANSKLQLLEALERKYEDNQKYLEDKAQELVRLEGEVRSLLKDISEKVAVYSTCL

SEQ ID NO: 43 - protein, 152 aa, Cricetulus griseus
MANSERTFIAIKPDGVQRGLVGEIIKRFEQKGFRLVGLKFMQASEDLLKEHYIDLKDRPFFTGLVKYMHSGPVVAMVWEGLNVVKTGRVMLGETNPADSKPGTIRGDFCIQVGRNIIHGSDSVESAEKEIGLWFQPEELVDYKSCAQNWIYE

SEQ ID NO: 44 - protein, 913 aa, Cricetulus griseus
MRYLRVKAKPLMTEFSVKSTIISRYAFTTVSCRVLNRASEDQDVEFQMQIPAAAFITNFTMLIGDKVYQSEITEKEKKSRDRIKEKRNKTTDDNEEKETDTFRASLVIPSKDKAAFLLSYEELLQRRLGKYEHSISVRPQQLVGRLTVEMNILERSGISALEVLPLHNSRKKGSGIAEGDVGPPPSTVINQNETFAKVIFKPTVVQQAKIAQNGILGDFIIRYDVKREQTIGDIQVLNGYFVHYFAPKDLPPLPKNVVFVLDTSASMVGMKLQQTREALVTILNDLRPQDHFNIIGFSNRIKVWKDHLLPVTPDNIRNGKLYIYHLSPTGGTDINGALQMAIKLLNNYVAQNDIEDRSVSLIVFLTDGKPTFGETNTLKILSNTKEATGGQICIFTIGIGNDVDFKLLEKLSLENCGLTRHVHEEEKAGEQLIGFYDEIRTPLLSDIRIDYPPDVVEHATKTLFPNYFNGSEIVIAGKMVDRKFDQFHVEVTASNSKKFVILKKDIPVESQKLGNDVTATPGPVPDGGKDPNHIERLWSYLTVKELLSSWRQSSSEQEKEQLRQKVQALALNYHFLTPFTSMKLKKPGLRTDGLEDTRGMSAATGPETVVQSVRGADMQPGPALKKPYSPRIKISKTSVDGDPHFVVDFPLSNLTVCFNIDGEPGDILRLVSDHLDSGVTVNGELIGAPAPPNGHKKQRTYFRTITILINRPERSYLEITPNRVILDGGDRLVLPCNQSVVVGSRGLEVSVSANANVTVTIQGTIAFVILIHLYKNPAPFQRNHLGFYIANSKGLSNNCHGLLGQFLNQDAKLIEAPAVYNKNLSGQSFAQTEGIPEAVLKVKGRRVPVVWKQRKIYNGQEQVDCWFDRNNAAKLIDGVYKNYLASHPFDTENILGLRMSRKAETGSLHEESV

SEQ ID NO: 45 - protein, 624 aa, Cricetulus griseus
MASSKEVQFFKAFSKNGSGITLPVADASVETLRRKLIDALESHSDMWSSSRPKLKPAKLVEINEFFAETNEDYLVLIFEDKDSYVGREVTLDLFQHHIPVHRVLNTERNAVSKFGVVEFPSCYLLFRNGSFSRVPVVMESRLFYTSYLKGMSGPILVDPPTTTISTDAPVTTDVVPTVWKVANHARIYMADLESSLHYIFLVEVGKFSVLEGQRLLALKKLVAVLAKYFPGRPLAQNFLHSIHDWLQRQQRKKIPYKFFRAALDNRKEGIVLTEKVNWVGCQGSKPHFRGFPCSLWILFHFLTVQASRYSENHPQEPADGQEVLQAMRSYVQWFFGCRDCAEHFENMAASTMHRVRSPTSAVLWLWTSHNKVNARLSGAPSEDPYFPKVQWPLRELCFDCHNEINGREPVWDLEATYRFLKAHFSSENIILDTPVAGLATQRNPQILGATPEPVMDALELETRNSVLGHERAASTESPGATALNVPVGKPEASGPQALYTGQGPPEHMEEPQRVTQGHTQGQQHLSKRDTEVLTLPEVNHLQGPLELRRGGRSPKQLVNIPEGEPEAPAIRGQGPWLQVLGRGFSHLDISLCVGLYSVSFVCLLAMYTYFRARLRTPKGHLVTQ

SEQ ID NO: 46 - protein, 420 aa, Cricetulus griseus
MRWKIIQLQYCFLLVPCMLTALEAVPIDVDKTKVHNTEPVESARIDPPDTGLYYDEYLKQVIDVLETDQHFREKLQKADIEEIRSGRLSKELDLVSHHVRTKLDELKRQEVARLRMLIKAKLDSLQDTGMNHHLLLKQFEHLNHQNPDTFESSDLDMLIKAATADLEQYDRTRHEEFKKYEMMKEHERREYLKTLNEEKRKEEESKFEEMKRKHENHPKVNHPGSKDQLKEVWEEADGLDPNDFDPKTFFKLHDVNNDGFLDEQELEALFTRELEKVYDPRNAEDDMIEMEEERLRMREHVMNEIDNNKDRLVTLEEFLRATEKKEFLEPDSWETLGQQQLFTEEELKEYESIIAMQENELKKRADELQKQKEELQRQHDHLEAQKQEYQQAVQQLEHKKFQQGIAPSGPAGELEFKPRM

SEQ ID NO: 47 - protein, 306 aa, Cricetulus griseus
MASSGSVQQPRLVLLMLVLAGAARASLYFRPGRTCYHPLRGDQIAQLGRRTYPRPHEYLSPSDIPKNWDWRNVKGVNYASITRNQHIPQYCGSCWAHGSTSAMADRINIKRKGAWPSTLLSVQNVIDCGNAGSCEGGNDLPVWAYAHKHGIPDETCNNYQAKDQDCDKFNQCGTCTEFKVCHTIQNYTRWRVGDYGSLSGREKMMAEIYANGPISCGIMVTEKMDNYTGGIYAELQEQTSINHIVSVAGWGVSSDGIEYWIVRNSWGEPWGERGWMRIVTSTYKGGTGASYNLAIEEACTYGDPIV

SEQ ID NO: 48 - protein, 2530 aa, Cricetulus griseus
MPAQCAWTSILTLLVWLGVARAGPFSPRSNVTLPAPRPPPQPGGPSSQLYEHTVEGGEKQVVFTHRINLPPSAGCGCPPGTEPPVPASEVQALKVRLEILEELVKGLKEHCSGGCCPTAAQAGTGQTDVRSLCSLHGVFDLSRCACSCEPGWGGPTCSDPTDTKTPTSSPPSASRTCPDDCNDQGRCVRGRCVCFPGYSGPSCGWPSCPGDCQGRGRCVQDCGVRTCPADCNRRGRCEDGRCLCDPGYTGPACATRMCPGDCRGRGRCVQGVCLCYAGYSGEDCGQEEPPASACPGGCGPRELCREGQCVCVEGFRGPDCAIQTCPGDCRGRGECLQGRCICQDGYAGDDCGEEVPAIQNMRMHLLEETTVRTEWTRAPGPVDAYEIQFIPMTEGASPPFTARVPSSASAYDQRGLAPGQDYQVTVRALRGTSWGPPASKTITTMIDGPQDLRVVAVTPTTLDLSWLRPQAEVDRFVVSYVSAGNQRVRLEVPPEADRTQLTDLMPGVEYVVTVTAERGRAVSYPASIRANTASDGAHLVTTARHPKPEVLGSAVDGALIVSLDGLRGQFERVVLRWRPLPPAEGPSGELTVDGSERTVRLPNLRPGTTYHVEVHGVRAGQTSKSYAFITTTGSLPSGLLEATDEPPPSGPSTTQGAQAPILILEHHPLGELQVLGRDKAGRLRVAWTAQPGTFSHFQLRMQVAEGPWAHEELLPGDVRQALVPPPPPGAPYKLLLQGITPGGKPSVPITYQGIMDRAEEQPGKPSVLPRLGELTVSSLTSDSLLLHWTVLEGEFDSFVIQYKDKDGPQVIPVEGPQRSAPVTSLEPGRKYRFILYGLIGKKKHGPLVAEAKILLQSDPSPGSPPRLGELWVTDPTPDSLHLSWTVPEGQFDSFLVQYRDKEGRPLVVPVEGPERSVVVSPLDPNHKYRFTLFGVANKKRYGPLTADGTTAPAKEEGFSEQPLLGELTVTGMTPDSLRLSWTVARGPFDSFVIQYKDAQGQPQTVPVAGDENEVTVPGLESNRKYKMNLYGLRGRQRVGPVSVVAKTAPPHIVDQPSSPPEPSTEAPQPLEKPRLGELTVTDATPDSLSLSWTVPEGQFDQFVIQYKNGDGQPKVVRVPGHEDQVTIPGLEPDHKYKMNLYGIHSGQRVGPVSVVGVTAAEEETPSPTEPSTEAPEPREEPLLGELTVTGSSPDSLSLSWTVPQGDFDSFTVQYKDSDGRPQVVRVGGQEREATVRDLEPGRKYKMNLYGLHDGQRVGPVSTVGVTDSQPEEEIPPAIEPPLEPRLEELTVTGVTPNSVSLSWMVPEGQFDSFMVQYKDRDGQPQEVPVSSDQRKVTILDLDPARKYKMNFYGLHGRRRVGPLSVLAMTDTLPPAPPPATEAPKLEPRLGELMVTDVTPDSVGLLWTVPEGEFDSFMVQYKDRDGQPQVVPVAADQREVTIPGLEPSRKYKFLLFGLRDGRRRGQVSVETKTDSLRLSWTVPEGHFDSFMVQFKDKGGPQVLPVDGHERTATITALDAGRKYRFLLYGLQGKKRFGPLTTEGTTEPMNTVDHTGVKAPPKPRLGEELRVTSVTQDSVDLSWTVSEGHFDSFVVQYKDRDGQSQVVPVEGGHREVRVSGLDPGHRYKLLLYGLRESKRVGPLSVIAVTGPKEATEAWTEVPTTSTPSVEPHLRELRVEEATPHSLRLSWVVTEGEFDSFEVQYTDRDGKLKVVSTEGDQSDVILTGLESDHRYLVTLYGFHDGHRVDSAQIEALTVPWEEEEPTEPPTVTPKPKPHLGELTVTDATPDSLSLSWTVPEGQFDQFVIQYKNGDGQPKVVRVPGHEDQVTIPGLEPDHKYKMNLYGIHSGQRVGPVSVVGVTAAEEETPSPTEPSTEAPEPREEPLLGELTYKDSDGRPQVVRVGGQEREATVRDLEPGRKYKMNLYGLHEGQRVGPVSTVGVTDPEEDAPSLKPRLEELTVTDATPDSLSLSWTVPEGQFDHFLVQYRNGDGQPKVVRVPGHEDQVTIPGLEPDHKYKMNLYGIHNGQRVGPVSVVGVTAAEEETPSPTEPSTEAPEPREEPLLGELTVTGSSPDSLSLSWTVPQGDFDSFTVQYKDSDGRPQVVRVGGQEREATVRDLEPGRKYKMNLYGLHDGQRVGPVSTVGVTDPEEETTTTQVVPTMTTKPPPERPRLGELTVADATPDSLSLSWTVPEGQFDHFLVQYRNGDGQPKVVRVPGHEDQVTIPGLEPDHKYKMNLYGIHSGQRVGPVSVVGGDFDSFTVQYKDSDGRPQVVRVGGQEREATVRDLEPGRKYKMNLYGLHDGQRVGPVSTVGVTSPEEETTTTQVVPTTTPTKPILGELTVTDATPDSLRLSWTVPEGQFDHFLVQYRNGDGQPKVVRVPGHEDQVTIPGLEPDHKYKMNLYGIHSGQRVGPVSVVGVTAAEEETPSPTEPSTEAPEPREEPLLGELTVTGSSPDSLSLSWTVPQGDFDSFTVQYKDSDGRPQVVRVGGQEREATVRDLEPGHKYKMNLYGLHQGQRVGPVSTVGVTGEC

SEQ ID NO: 49 - protein, 244 aa, Cricetulus griseus
MSTVHEILCKLSLEGDHSTPPSAYGSVKPYTNFDAERDALNIETAVKTKGVDEVTIVNILTNRSNAQRQDIAFAYQRRTKKELPSALKSALSGHLESVILGLLKTPAQYDASELKASMKGLGTDEDSLIEIICSRTNQELQEINRVYKEMYKTDLEKDIISDTSGDFRKLMVALAKGRRAEDGSVIDYELIDQDARELYDAGVKRKGTDVPKWISIMTERSVCHLQKGGCCARETSVPGGSWMA

SEQ ID NO: 50 - protein, 2488 aa, Cricetulus griseus
MPMWDEEEDEEAKKQTPKQRLLGWIQNKLPQLPITNFSRDWQSGRALGALVDSCAPGLCPDWDSWDASKPVNNAREAMQQADDWLGIPQVITPEEIVDPNVDEHSVMTYLSQFPKAKLKPGAPLRPKLNPKKARAYGPGIEPTGNMVKKRAEFTVETRSAGQGEVLVYVEDPAGHQEEAKVTANNDKNRTFSVWYVPEVTGTHKVTVLFAGQHIAKSPFEVYVDKSQGDASKVTAQGPGLEPSGNIANKTTYFEIFTAGAGTGEVEVIIQDPTGQKGTVEPQLEARGDSTYRCSYQPTMEGVHTVHVTFAGVPIPRSPYTVTVGQACNPAACRAVGRGLQPKGVRVKETADFKVYTKGAGSGELKVTVKGPKGEERVKQKDLGDGVYGFEYYPTIPGTYTVTITWGGQNIGRSPFEVKVGTECGNQKVRAWGPGLEGGVVGKSADFVVEAIGDDVGTLGFSVEGPSQAKIECDDKGDGSCDVRYWPQEAGEYAVHVLCNSEDIRLSPFMADIREAPQDFFPDRVKARGPGLEKTGVAVNKPAEFIVDAKHAGKAPLRVQVQDNEGCPVDATVKDNGNGTYSCSYVPRKPVKHTAMVSWGGVSIPNSPFRVNVGAGSHPNKVKVYGPGVAKTGLKAHEPTYFTVDCTEAGQGDVSIGIKCAPGVVGPTEADIDFDIIRNDNDTFTVKYTPRGAGSYTIMVLFADQATPTSPIRVKVEPSHDASKVKAEGPGLSRTGVELGKPTHFTVNAKTAGKGKLDVQFSGLAKGDAVRDVDIIDHHDNTYTVKYTPVQQGPVGISVTYGGDNIPKSPFSVGVSPSLDLSKIKVSGLGDKVDVGRDQEFTVKSKGAGGQGKVASKIVSPSGAAVSCKVEPGLGADNSVVRFVPREEGPYEVEVTYDGVPVPGSPFPLEAVAPTKPSKVKAFGPGLQGGNAGSPARFTIDTKGAGTGGLGLTVEGPCEAQLECLDNGDGTCSVSYVPTEPGDYNINILFADTHIPGSPFKAHVVLCFDASKVKCSGPGLERATAGEVGQFQVDCSSAGSAELTIEICSEAGLPAEVYIQDHGDGTHTITYIPLCPGAYTVTIKYGGQPVPNFPSKLQVEPAVDTSGVQCYGPGIEGQGVFREATTEFSVDARALTQTGGPHVKALVAIPSGNLTETYVQDCGDGTYKVEYTPYEEGVHSVDVTYDGSPVPSSPFKVPVTEGCDPSRVRVHGPGIQSGTTNKPNKFTVETRGAGTGGLGLAVEGPSEAKMSCMDNKDGSCSVEYIPYEAGTYSLNVTYGGHQVPGSPFKVPVHDVTDASKVKCSGPGLSPGMVRANLPQSFQVDTSKAGVAPLQVKVQGPKGLVEPVDVVDNADGTQTVNYVPSREGPYSISVLYGEEEVPRSPFKVKVLPTHDASKVKASGPGLNTTGVPASLPVEFTIDAKDAGEGLLAVQITDPEGKPKKTHIQDNHDGTYTVAYVPDVTGRYTILIKYGGDEIPFSPYRVRAVPTGDASKCTVTGAGIGPTIQIGEETVITVDTKAAGKGKVTCTVCTPDGSEVDVDVVENEDGTFDIFYTAPQPGKYVICVRFGGEHVPNSPFQVTALAGDQPTVQTPLRTQQLAPQYTYPQGSQQTWVSERPMVGVNGLDVTTLRPFDLVIPFTIKKGEITGEVRMPSGKVAQPSITDNKDGTVTVRYSPSEAGLHEMDIRYDNMHIPGSPLQFYVDYVNCGHVTAYGPGLSHGVVNKPATFTVNTKDAGEGGLSLAIEGPSKAEISCTDNQDGTCSVSYLPVLPGDYSILVKYNDQHIPGSPFTARVTGDDSMRMSHLKVGSAADIPINISETDLSQLTATVVPPSGREEPCLLKRLRNGHVGISFVPKETGEHLVHVKKNGQHVASSPIPVVISQSEIGDASRVRVSGQGLREGHTFEPAEFIIDTRDAGYGGLSLSIEGPSKVDINTEDLEDGTCRVTYCPTEPGNYIINIKFADQHVPGSPFSVKVMGEGRVKESITRRRRAPSVANVGSHCDLSLKIPEISIQDMTAQVTSPSGKTHEAEIVEGENHTYCIRFVPAEMGMHTVSVKYKGQHVPGSPFQFTVGPLGEGGAHKVRAGGPGLERAEAGVPAEFSIWTREAGAGGLAIAVEGPSKAEISFEDRKDGSCGVAYVVQEPGDYEVSVKFNEEHIPDSPFVVPVASPSGDARRLTVSSLQESGLKVNQPASFAVSLNGAKGAIDAKVHSPSGALEECYVTEIDQDKYAVRFIPRENGIYLIDVKFNGTHIPGSPFKIRVGYYGHGGDPGLVSAYGAGLEGGVTGSPAEFIVNTSNAGAGALSVTIDGPSKVKMDCQECPEGYRVTYTPMAPGSYLISIKYGGPYHIGGSPFKAKVTGPRLVSNHSLHETTSVFVDSLTNPATVPQLATSGPSPTDVSKVVAKGLGLSKAYVGQKSSFTVDCSKAGNNMLLVGVHGPRTPCEEILVKHMGSRLYSVSYLLKDKGEYTLVVKWGDEHIPGSPYRIMVP

SEQ ID NO: 51 - protein, 331 aa, Cricetulus griseus
MSGRGKQGGKARAKAKTRSSRAGLQFPVGRVHRLLRKGNYSERVGAGAPVYLAAVLEYLTAEILELAGNAARDNKKTRIIPRHLQLAIRNDEELNKLLGRVTIAQGGVLPNIQAVLLPKKTESHHKAKGNSAARVPASASACAKRKASGPPVSELITKAVAASKERSGVSLAALKKALAAAGYDVEKNNSRIKLGLKSLVSKGTLVQTKGTGASGSFKLNKKAASGEAKPKAKKAGAAKAKKPAGAAKKPKKAAGTATPKKSTKKTPKKAKKPAAAAGAKKAKSPKKAKAAKPKKAPKSPAKAKAVKPKAAKPKTAKPKAAKPKKTAAKKK

SEQ ID NO: 52 - protein, 364 aa, Cricetulus griseus
MPYPYPALTPEQKKELSDIAHRIVAPGKGILAADESTGSIAKRLQSIGTENTEENRRFYRQLLLTADDRVNPCIGGVILFHETLYQKADDGRPFPQVIKSKGGVVGIKVDKGVVPLAGTNGETTTQGLDGLSERCAQYKKDGADFAKWRCVLKIGEHTPSALAIMENANVLARYASICQQNGIVPIVEPEILPDGDHDLKRCQYVTEKVLAAVYKALSDHHVYLEGTLLKPNMVTPGHACTQKFSNEEIAMATVTALRRTVPPAVTGVTFLSGGQSEEEASINLNAINKCPLLKPWALTFSYGRALQASALKAWGGKKENLKAAQEEYIKRALANSLACQGKYTPSGQSGAAASESLFISNHAY

SEQ ID NO: 53 - protein, 316 aa, Cricetulus griseus
MVSHLQLNNGAKMPILGLGTWKSPPGQVTEAVKAAIDIGYRHIDCAQVYQNEKEVGMALQEKLKEQVVKRQDLFIVSKLWCTFHDKSMVKGACQKTLSDLQLDYLDLYLIHWPTGFKPGPDYFPLDESGNVIPSETDFVDTWTAMEQLVDEGLVKSIGVSNFNPLQIERILNKPGLKYKPAVNQIECHPYLTQEKLIEYCQSKGIVVTAYSPLGSPDRPWAKPEDPSLLEDPRIKAIASKYNKTTAQVLIRFPIQRNLVVIPKSVTPARIAENLKVFDFELSKEDVTTLLSYNRNWRVCALMSCAKHKDYPFHAEV

SEQ ID NO: 54 - protein, 417 aa, Cricetulus griseus
MLLSVPLLLGLLGLAAAEPAVYFKEQFLDGDDWTNRWVESKHKSDFGKFVLSSGKFYGDQEKDKGLQTSQDARFYALSARFEPFSNKGQTLVVQFTVKHEQNIDCGGGYVKLFPGSLDQKDMHGDSEYNIMFGPDICGPGTKKVHVIFNYKGKNVLINKDIRCKDDEFTHLYTLIVRPDNTYEVKIDNSQVESGSLEDDWDFLPPKKIKDPNAAKPEDWDERAKIDDPTDSKPEDWDKPEHIPDPDAKKPEDWDEEMDGEWEPPVIQNPEYKGEWKPRQIDNPDYKGTWIHPEIDNPEYSPDANIYAYDSFAVLGLDLWQVKSGTIFDNFLITNDEAYAEEFGNETWGVTKASEKQMKDKQDEEQRLKEEEEDKKRKEEEEAEDKEDEDDRDEDEEDEDEKEEDEEDTTPGQTKDEL

SEQ ID NO: 55 - protein, 135 aa, Cricetulus griseus
MACGLVASNLNLKPGECLKVRGEVAPDAKSFVLNLGKDSNNLCLHFNPRFNAHGDANTIVCNSKDNGAWGTEHREPAFPFQPGSTVEVCITFDQADLTIKLPDGHEFKFPNRLNMEAINYMAADGDFKIKCVAFE

SEQ ID NO: 56 - protein, 132 aa, Cricetulus griseus
MCDAFVGTWKLVSSENFDDYMKEVGVGFATRKVAGMAKPNMIISVNGDVITIRSESTFKNTEISFKLDQEFEEITADDRKVKSVITLDGGALVQVQKWDGKSTTIKRKREGDKLVVECVMKGVTSTRTYERA

SEQ ID NO: 57 - protein, 451 aa, Cricetulus griseus [sequence omitted]

SEQ ID NO: 58 - protein, 479 aa, Cricetulus griseus
MSEDEEDDSSGEEVVIPQKKGKKATATPAKKVVVSQTKKVAVPTPAKKAAVTPGKKAAATPAKKAVTPAKAVATPGKKGATQAKALVATPGKKGAVTPAKGAKNGKNAKKEDSDEDEDDDDDEDDSDEDEEDEEEDEFEPPVVKGKQGKVAAAAPASEDEDEEEDEEEEEEDEEEEDDSEEEEAMEITPAKGKKAPAKVVPVKAKNVAEEEDDDDAPAKVVPVKAKNVAEEDDDDEEEDEDEEEDEEEEEDEEEEEEEEEEEPVKPAPGKRKKEMTKQKEVPEAKKQKVEGSESTTPFNLFIGNLNPNKSVAELKVAISELFAKNDLAVVDVRTGTNRKFGYVDFESAEDLEKALELTGLKVFGNEIKLEKPKGRDSKKVRAARTLLAKNLSFNITEDELKEVFEDALEIRLVSQDGKSKGIAYIEFKSEADAEKNLEEKQGAEIDGRSVSLYYTGEKGQRQERTGKNSTWSGELKFES

SEQ ID NO: 59 - protein, 893 aa, Cricetulus griseus
MSVCICLLHPLWGRTFLLILSVAVAQSHWPSEPSEAMRDWKNQLEASMHSVLSDFHETVPTVVGIPDGTAVVGRSFRVSIPTELIASSGDTIKVSAAGKEILPSWLHWDPHSNTLEGLPLDTDKGVHYISVSAARPGANGSHVPQTSSVFSIEVYPEDHNEPQSVRAASSDPGEVVSSACAVDEPVTVLTVILDADLTKMTPKQRIDLLSRMQSFSEVELHNMKLVPVVNNRLFDMSAFMAGPGNAKKVVENGALLSWKLGCSLNQNSVPDIRGVETPAREGAMSAQLGYPVVGWHIANKKPTLPKRIRRQIHATPTPVTAIGPPTTAIQEPPSRIVPTPTSPAIAPPTETMAPPVRDPVPGKPTVTTRTRGAIIQTPTLGPIQPTRVSEAGTTIPGQIRPTLTIPGYIEPTAVVTPPTTTTKKPRVSTPKPATPSTDSSTTTTRRPTKKPRTPRPVPRVTTKAPITRLETASPPTRIRTTTSGLPRGGEPNQRPELKNHIDRVDAWVGTYFEVKIPSDTFYDNEDTTTDKLKLTLKLREQQLVGEKSWVQFNSNSQLMYGLPDNSHVGKHEYFMHATDKGGLSAVDAFEIHVHKRPQGDKAPARFKAKFAGDPAPVVNDIHKKIALVKKLAFAFGDRNCSTITLQNITRGSIVVEWTNNTLPLEPCPKEQIIGLSRRIADENGKPRPAFSNALEPDFKAVSIAVTGAGSCRHLQFIPVAPPSPGTSAAPATEVPDRDPEKSSEDDVYLHTVIPAVVVAAILLIAGIIAMICYRKKRKGKLTLEDQATFIKKGVPIIFADELDDSKPPPSSSMPLILQEEKAPLPPPEYPNQSVPETTPLNQDTVGEYTPLRDEDPNAPPYQPPPPFTAPMEGKGSRPKNMTPYRSPPPYVPP

SEQ ID NO: 60 - protein, 697 aa, Cricetulus griseus
MSAKAISEQTGKELLYKYICTTSAIQNRFKYARVTPDTDWARLLQDHPWLLSQSLVVKPDQLIKRRGKLGLVGVNLTLDGVKSWLKPRLGHEATVGKAKGFLKNFLIEPFVPHSQAEEFYVCIYATREGDYVLFHHEGGVDVGDVDAKAQKLLVGVDEKLNTEDIKRHLLVHAPEDKKEILASFISGLFNFYEDLYFTYLEINPLVVTKDGVYILDLAAKVDATADYICKVKWGDIEFPPPFGREAYPEEAYIADLDAKSGASLKLTLLNPKGRIWTMVAGGGASVVYSDTICDLGGVNELANYGEYSGAPSEQQTYDYAKTILSLMTREKHPDGKILIIGGSIANFTNVAATFKGIVRAIRDYQGPLKEHEVTIFVRRGGPNYQEGLRVMGEVGKTTGIPIHVFGTETHMTAIVGMALGHRPIPNQPPTAAHTANFLLNASGSTSTSVDFSQVSIEEQRCKERSQEGKSATLFSRHTKAIVWGMQTRAVQGMLDFDYVCSRDEPSVAAMVYPFTGDHKQKFYWGHKEILIPVFKNMADAMKKHPEVDVLINFASLRSAYDSTMETMSYAQVQFGHAGACANQASETAVAKNQALKEAGVFVPRSFDELGEIIQSVYEDLVAKGAIVPAQEVPPPTVPMDYSWARELGLIRKPASFMTSICDERGQELIYAGMPITEVFKEEMGIGGVLGLLWFQRR

SEQ ID NO: 61 - protein, 462 aa, Cricetulus griseus
MWELKSRWRAVGLGLLLLLSAAAQAAPSAPRRYTPDWQSLDSRPLPRWFDEAKFGVFVHWGVFSVPAWGSEWFWWHWQSERIPAYENFMKENYPPGFSYADFGPQFTARFFHPDQWAALFQAAGAKYVVLTTKHHEGFTNWPSPVSWNWNSKDVGPHRDLVGELGAAVRKRNLRYGLYHSLLEWFHPLYLLDKKNGFKTQYFVGAKTMPELYDLVNSYKPDLIWSDGDWESPDTYWNSTAFLAWLYNDSPVKDEVVVNDRWGQNCSCHHGGYYNCEDKYTPHSLPKHKWEMCTSVDSASWGYRRDMTLSTIASEQEIIEELIQTVSLGGNYLLNIGPTKDGLIDPIFQERLLAVGKWLQINGEAIYASHPWRVQFEKNITVVWYTSKDSAVYATFLYWPENGIINLKSPQTTSATKVTMLGMEGYLTWTQDLQDGFLISLPPLPPTALPVEFAWTLKLINVK

SEQ ID NO: 62 - protein, 3735 aa, Cricetulus griseus
MAKRGGRLCAGSAPRAGGPRSPAPPSLLLLLLLAGLAPLGEARTPGGDGFSLHPPYFNLAEGARITASATCGEEAPTRNASRPTEDLYCKLVGGPVAGGDPNQTIQGQYCDICTAANSNKAHPVSNAIDGTERWWQSPPLSRGLEYNEVNVTLDLGQVFHVAYVLIKFANSPRPDLWVLERSTDFGHTYQPWQFFASSKRDCLERFGPRTLERITQDDDVICTTEYSRIVPLENGEIVVSLVNGRPGAMNFSYSPLLRDFTKATNIRLRFLRTNTLLGHLMGKALRDPTVTRRYYYSIKDISIGGRCVCHGHADVCDAKDPSDPFRLQCACQHNTCGGSCDRCCPGFNQQPWKPATTDNANECQSCNCHGHAHDCYYDPEVDRRNASQNQDNVYQGGGVCLDCQHHTTGINCERCLPGFYRAPDQPLDSPYVCRRCNCESDFTDGTCEDLTGRCYCRPNFTGEHCTACAEGYTGFPHCYPVPHNDTREQVSPAGQIVNCDCNAAGTQGNACRKDPRLGRCVCKPNFQGSHCELCAPGFYGPNCQSCQCSSPGVASGLCDPESGQCTCRTGFEGDKCDHCALGYFHFPLCQLCGCSPAGTLPEGCDEAGRCQCRPGFDGPHCDRCLPGYHGYPDCHACACDPQGSLDQLCGVGGSCRCRPGYAGTTCQECSPGFHGFPSCIPCHCSAHGSLHTNCDPTTGQCSCRPRVTGLRCDMCVPGAYNFPYCEAGSCHPAGLAPANPALPESQASCTCRAHVEGPSCDRCKPGYWGLSPSNPEGCTRCSCDPRGTLGGVTECQLGNGQCFCKAHVCGQACAACKDGFFGLDHADYFGCRGCRCDVGGALGQGCEPRTGACRCRPNTQGPTCSEPTKDHYLPDLHHMRLELEEAATPQGHGVRFGFNPLEFENFSWRGYAHMTPIQPRIVARLTVTAPDLFRLVFRYVNRGPTSVNGRVSVREEGRLSSCVNCTEQSQPVAFPPSTEPAFVTVPQRGFGEPFVLNPGTWTLLVEAEGVLLDYVVLLPSTYYEAALLQHRVTEACTYRPSAVHSTENCLLHAHLPLDGFPSAAGTEALCLHDNSLPQPCPTEQLSPSHPPLVTCVGSDVDIQLEMAVPRPGRYALVVEYVSEESHQEVGVAVHTPQRAPQQGMLNLHPCPYSSLCRGLALDTQHHLATFHLDSEASIRLTAEQAHFFLHRVTLVPVEEFSTEFVEPRVFCVSTHGTFNASSSACLPSRFPKPPQPIILKDCQVLPLPPDLPLSQSQEVTPGAPPAGPQPRPPTIVDPNAEPTLLRHPQGTVVFTTHVPTLGRYAFLLHSYQPVHPKFPVEVLINGGRVWQGHANASFCPHGYGCRTLVLCEGQTMLDVTDNELTVTVRVPEGRWLWLDYILIVPEDAYSSTYLHEEPLDKSYDFISHCATQGYHISPSSSSLFCRNAATSLSLFYNNGALPCACHEVGAISPTCEPFGGQCPCRGHVIGRDCSRCATGYWGFPHCRPCDCGTRLCDELTGQCICPPRTVPPDCLVCQPQTFGCHPLVGCEECNCSGPGVQELADPTCDMDSGQCKCRPNVAGRRCDTCAPGFYGYPSCRPCDCHEAGTVASVCDPFTGQCHCKENVQGSRCDQCRLGTFSLDAANPKGCTRCFCFGATERCGSSNHARHEFVDMEGWVLLGSDRQVVPHQHRPEMELLHADLRLLADSFPELYWQAPPSYLGDRVSSYGGTLQYELHSEIQRGDVFISYESRPDVVLQGNQMSIAFMELAYPPPGHVHRRQLQLVEGNFRHLETHNPVSREEIMMVLAGLEQLQIRALFSQTSATVSLRRVVLEVASEAGRGPPASNVELCMCPANYRGDSCQECAPGYYRDIKGLFLGRCVPCQCHGHSDRCLPGSGTCVSCQHNTEGDQCERCRVGFVRTDPNDPAAPCVSCPCPLAVPSNNFADGCVLRNGRTQCLCRPGYAGASCERCAPGFFGNPLVLGSSCQPCDCSGNGDPNMIFSDCDPLTGACRGCLRHTTGPHCESCAPGFYGNALLPGNCTRCDCSPCGTETCDPQSGRCLCKAGVTGQRCDRCLEGHFGFEQCQGCRPCTCGPAAKGSKCHPQSGQCHCQPGTTGPQCRECAPGYWGLPEKGCRRCQCPQGHCDPHTGRCTCPPGLSGERCDTCSQQYQVPVPGGPGGHGIHCEVCDHCVVLLLDDLEQAGALLPAIREQLRGINASSTAWARLHSLNASIADLKSKLRSPLGPRYQTTQQLQTLEQQSASLQQDIEQLGSQAIGAQDRAGQLTDNTEATLGRAQTLLETVRAVDRALRELASRIGQASPDGASAPSGEQLRWALAEMERLLRDMRTRDLGAQREVAEAELAEARRLMAHVQGQLTNFWEENQSLASHIRDQLAQFEAGLMDLREALNHAVNTTREADELNSRNQERLKEALQWKQELFRDNATIKAALQAARLTLGRVSELLQGMDQAKEDLEHLAASLDGAWTPLLKKMQAFSPASSKVDLVEAAETHAQKLHQLAINLSGIILGINQDRFIQRAVEASSAYTSILQAVQAAEAAAGQALQQASHTWETVVQRGLAARAQKLLANSSALEETILGHRERLGRAQGRLQAAATQLHDVRAKKDQLAAQIREAQAMLAMDTGETSEKIAHAKAVAAEAQDTATHVRSQLDSMQKNVERWQSQLGGLRGQDLGQVERDASTSVSTLEKTLPQLLAKLSRLENRGVHNASLALSANIGRVRKLIAQARGAANKVKVSMKFNGHSGVQLRTPRNLPDLAAYTALKFYLQSPVPAPAPGENTGDRFVLYMGSRQPTGDYMGVSLRNQKVHWVYKLGEAGHTTLSIDENIGEQFAAISIDRTLQFGHMSVTVEKPMVQEIKGDTVAPGLEGLLSLQPDDFVFYVGGYPKNFTPPEPLRFPGYLGCIEMDTLNEEVVSLYNFEQIFKLDTAVDKPCARSKATGDPWLTDGSYLDGSGFARISFEKQFSNTKRFDQELRLVSYNGIIFFLKQESQFLCLAVQEGTLVLLYDFGEGLKRATPLQTPHPLTAASKAIQVFLLAGSRKRVLVRVERATVFSVEQDNMLEMADAYYLGGVPPEQLPPSLRQLFPSGGSVRGCIKGIKALGKYVDLKRLNTTGISFGCTADLLVGRAMTFHGHGFLPLALPDVVPITGEVYSGFGFRGTQEDSLLYYRTSPDGPYQVFLKQGHLTLQFMGTAVETQRVFADGAPHYVAFYTNGTRVQLFVDDQLQQIESLREPPPTFQPQPQQSPQLLLGGLPKSGTSHNFSGCISNVFVKRLRGPQRVFDLQQNMGGVNVSIGCTPPQLIQTSRAMPQKVSRRSRQPGQDLACTPPWLQGTIQDAYQFGGPLPSYLQFVGISPSRRNRLHLSMLVRPHDASQGLLLSAAPLSSLGPSLVLFLSHGHFVAQTEGPGPGLRVQSHQQSRADQWHRVSVRWGLQQIQLVVDGSQTWSQKAPRHRGHRAKGPQSHTLFVGGLPDSSYSSKLPVSVGFSGCVKNLQLDKQPLRTPTRMVGVIPCVSGPLEDGLFFPGSEGIITLELSKAKLPYVSLELEVRPLAAAGLIFHLGQAEATPYIQLQMLTEQVLLRANDGAGEFSTWVTYPKLCDGQWHRVAVIKGRNTLRLEVDTQSNHTMGTSPVTLAAIPVPLHLGGLPKATAAQPELPAYRGCMRKLVVNGDPVTVTTSAQVQGTVGVSGCPSGTLASAHSEAPPRPMGKRKAPARRQVGSSGLWQANPITLPLLQR

SEQ ID NO: 63 - protein, 412 aa, Cricetulus griseus
MYYWVFQHFSVEGQLEFRALLFIPRRAPFDLFENKKKKNNIKLYVRRVFIMDSCDELIPEYLNFIRGVVDSEDLPLNISREMLQQSKILKVIRKNIVKKCLELFSELAEDKENYKKFYEAFSKNLKLGIHEDSTNRRRLSELLRYHTSQSGDEMTSLSEYVSRMKETQKSIYYITGESKEQVANSAFVERVPKRGFEAVYMTEPIDEYCVQQLKEFDGKSLVSVTKEGLELPEDEEEKKKMEESKAKFENLCKLMKEILDKKVEKVTISNRLVSSPCCIVTSTYGWTANMERIMKAQALRDNSTMGYMMAKKHLEINPDHPIVETLRQKAEADKNDKAVKDLVVLLFETALLSSGFSLEDPQTHSNRIYRMIKLGLGIDEDEVTAEEPSAAVPDEIPPLEGDEDASRMEEVD

SEQ ID NO: 64 - protein, 2503 aa, Cricetulus griseus
MEEVVIAGMSGKLPESENLQEFWANLIGGVDMVTDDDRRWKAGLYGLPKRSGKLKDLSKFDASFFGVHPKQAHTMDPQLRLLLEVSYEAIVDGGINPASLRGTNTGVWVGVSGSEASEALSRDPETLLGYSMVGCQRAMMANRLSFFFDFKGPSIALDSACSSSLLALQSAYQAIRNGECPAALVGGINVLLKPNTSVQFMKLGMLSPEGTCKSFDDSGNGYCRSEAVVAVLLTKKSLARRVYATILNAGTNTDGCKEQGVTFPSGEAQEQLIQSLYRPAGLAPESLEYIEAHGTGTKVGDPQELNGIVRSLCASRQGPLLIGSTKSNMGHPEPASGLAALTKVLLSLENGVWAPNLHFHNPNPEIPALLDGRLQVVDRPLPVRGGNVGINSFGFGGANVHVILQPNTQQAPAPAPHAALPHLLHASGRTAEAVQGLLEQGRKHSQDMAFVSMLNDIAATPTAAMPFRGYTVLGVEGDVQEVQQVPASKRPLWFICSGMGTQWRGMGLSLMRLDSFRESILRSDEAVKPLGIKVSDLLLSTDESTFDDIVHAFVGLTAIQIALIDLLTSVGLKPDGIIGHSLGEVACGYADGCLSQREAVLAAYWRGQCIKDAHLPPGSMAAVGLSWEECKQRCPSGVVPACHNSEDTVTISGPQAAVSEFVEQLKQEGVFAKEVRTGGLAFHSYFMEGIAPMLLQALKKVIREPRPRSARWLSTSIPEAQWQSSLARTSSAEYNVNNLVSPVLFQEALWHVPEHAVLLEIAPHALLQAVLKRGVKSSCTIIPLMKRDHKDNLEFFLTNLGKVHLTGIDVNPNALFPPVDFPAPRGTPLISPHIKWDHSQTWDVPAAEDFPNGSCSSSATVYSIDASPESPDHYLVDHCIDGRVLFPATGYLYLVWKTLARNLSLSLEETPVVFEDVTIHQATILPKTGTVPLEVRLLEASRAFEVSENGNLIVSGKVYQWEDPDSKLFDHPHVLNPPESTPVSRLTQTEVYKELRLRGYDYGPHFQGIVEASLEGEQGKLLWKGNWVTFLDTMLQVSILGVSQQSLRLPVRVTAIHIDPATHLQKVYTLEGENQVADVTTSLCLDSTVSGGVRISRLHTTAAPRRQQEQLVPTLEKFIFTPHVEDGCLSENTTLQRELQLCKDLAQALQTKATQQGLKMTVPGLEGPPQHGLSRLLAAACQLQLNGNLQLELGEALAQERVLLPEDPLISGLLNSQALKACVDTALENLPSLKMKVVEVLSGEGRLYSRIPSLLNTQPMLQLEYTATDLHPEALKDVQAKLQQHDIAQGQWNPEDPAPSNLGALDLVVCSCAVATLGNPALALSNMVAALKEGGFLLMHTVLRGHSLGETLACLPSAVQPGPSLSQEEWESLFSKKGLHLVGLKKSFYGTALFLCRRATLQDNPLFLPVEDTSYQWVDSLKRILAESSSQPVWLTATDCPTSGVVGLVNCLRKEPGGHRIRCILLSNLSTSSHTPKMGPGSSELQKVLKNDLVMNVYRDGAWGAFRHFLLEQDKPEEQTAHAFVNVLTRGDLASIRWVCSPLKHAQPTSPGTQLCTVYYASLNFRDIMLATGKLPPDAIPGKWASRDCMLGMEFSGRDKCGRRVMGLVPAEGLATSVLLSPDFLWEVPSSWTLEEAASVPVVYTTAYYSLVVRGRVQRGETVLIHSGSGGVGQAAISIALSLGCRVFTTVGSAEKRAYLQARFPQLDDTSFANSRDTSFEQHVLLHTGGKGVNLVLNSLAEEKLQASVRCLAQHGRFLEIGKFDLSNNHPLGMAIFLKNVTFHGILLDALFEEANDSWREVAALLQAGIRDGVVKPLKCTVFPKDQVEDAFRFMAQGKHIGKVLVQVREEEPEAVLPGAQPTLIPAISKTFCPAHKSYIITGGLGGFGLELARWLVLRGAQRLVLTSRSGIRTGYQAKQVQEWRRQGIHVLVSTSNASSLEGARALITEATKLGPVGGVFNLAMVLRDAMLENQTPELFQDVNKPKYNGTLNLDRTTREACPELDYFVAFSSVSCGRGNAGQTNYGFANSAMERICEQRRHDGLPGLAVQWGAIGDVGIVLEAMGTNDTVIGGTLPQRIASCMEVLDLFLNQPYAVLSSFVLAEKKAVAQGDGEAQRDLVKAVAHILGIRDLAGVNLDSSLADLGLDSLMGVEVRQILEHEHDLVLPMREVRQLTLRKLEELSSKAGSASETTAPKSKNDTALKQTQLNLSTLLVNPEGPTLTRLNSVQSSERPLFLVHPIEGSTTVFHSLAAKLSVPTYGLQCTQAAPLDSIPDLAAYYIDCIKQVQPEGPYRVAGYSFGACVAFEMCSQLQAQQGPTPTHNSLFLFDGSHTYVLAYTQSYRARMTPGCEAEAEAEAICYFIKQFTDAEHNKVLEALLSLKSLEDRVTAAVDLITKSHHSLDRRELSFAALSFYQKLRAADQYKPKAKYHGNVTLLRAKTGGTYGEDLGADYNLSQVCDGKVSVHIIEGDHRTLLEGSGLESIINIIHSSLAEPRVSVREG

SEQ ID NO: 65 - protein, 444 aa, Cricetulus griseus
MREIVHIQAGQCGNQIGAKFWEVISDEHGIDPTGTYHGDSDLQLDRISVYYNEATGGKYVPRAILVDLEPGTMDSVRSGPFGQIFRPDNFVFGQSGAGNNWAKGHYTEGAELVDSVLDVVRKEAESCDCLQGFQLTHSLGGGTGSGMGTLLISKIREEYPDRIMNTFSVVPSPKVSDTVVEPYNATLSVHQLVENTDETYCIDNEALYDICFRTLKLTTPTYGDLNHLVSATMSGVTTCLRFPGQLNADLRKLAVNMVPFPRLHFFMPGFAPLTSRGSQQYRALTVPELTQQVFDAKNMMAACDPRHGRYLTVAAVFRGRMSMKEVDEQMLNVQNKNSSYFVEWIPNNVKTAVCDIPPRGLKMAVTFIGNSTAIQELFKRISEQFTAMFRRKAFLHWYTGEGMDEMEFTEAESNMNDLVSEYQQYQDATAEEEEDFGEEAEEEA

SEQ ID NO: 66 - protein, 117 aa, Cricetulus griseus
MKSKELVDTLKVIPVVHRLNMPSDQDSTGKTSHESSQLDEPSVETHSHEQSQEHKQKASHESTELSDVIDSKESSKASQEHQSHEDKLVPDSKSKEDINHLKIRISHEIESSSSEVN

SEQ ID NO: 67 - protein, 659 aa, Cricetulus griseus
MKTDKRLSDKEVPPQGSADNLLVLTVATKETEGFRRFKRSAQFFNYKIQWVPSLDPASPSPRFGHSYDVVFASGPRELLKKFQQAKSRVVFSAEELIYPDRRLEAKYPTVSDGKRFLGSGGFIGYAPNLNKLVAEWEGQDSDSDQLFYTKIFLDPEKREQINISLGHSCSIFQNLDGALDEVVLKFEMGHVRARNLAYDTLPVVIHGNGPTKLQLNYLGNYIPRFWTFETGCTVCDEGLRSLKGIGDEALPTVLVGVFIEQPTPFLSLFFLRLLRLRYPQKRMRLFIHNHEQHHKLEVEKFLAEHGTEYQSVKLVGPEVRMANADARNMGADLCRQDQTCTYYFSVDADVALTEPDSLRLLIEQNKNVIAPLMTRHGRLWSNFWGALSADGYYARSEDYVDIVQGRRVGVWNVPYISNIYLIKGSALRAELQHVDLFHYSKLDADMSFCANVRQQEVFMFLTNRHTFGHLLSLDNYQTTHLHNDLWEVFSNPEDWKEKYIHENYTKALEGKLVEMPCPDVYWFPIFTEAACDELVEEMEHYGQWSLGDNKDNRIQGGYENVPTIDIHMNQITFEREWHKFLVEYIAPMTEKLYPGYYTRAQFDLAFVVRYKPDEQPSLMPHHDASTFTVNIALNRVGQDYEVSQGLGAQRQVEGGARLF

SEQ ID NO: 68 - protein, 203 aa, Cricetulus griseus
MAPFASLASGILLLLSLITSSKACSCAPPHPQTAFCNSDLVIRAKFMGPPEIIFNLYQRYEIKMTKMLKGFDAVGNAADFRFAYTPALESLCGYVHKSQNRSEEFLIAGRLRNGSLHISACSFLVPWYSLTPAQQKAFSKTYSAGCGVCTVFPCSTMPCKLESDTHCLWTDQILTGSEKGYQSRNFACLPRNPQLCAWQSLRA

SEQ ID NO: 69 - protein, 483 aa, Cricetulus griseus
MAQADIALIGQEDMGQNLILNMNDHGFVVCTFNRTVSKVDDFLANEAKGTKVVGAKSLKEMVSMLKKPRRIILLVKAGQAVDDFIEKLVPLLNTGDIIIDGGNSEYRDTTRRCRDLKAKGILFVGSGVSGGEEGARYGPSLMPGGNKEAWPHIKTIFQAIAAKVGTGEPCCDWVGEEGAGHFVKMVHNGIEYGDMQLICEAYHLMKDVLGMQHEEMAQAFEEWNKTELDSFLIEITANILKFRDTDGQELLPKIRDSAGQKGTGKWTAISALEYGMPVTLIGEAVFARCLSSLKEERVQASKTLTGPQKTQLAHNKESFLEDIRKALYASKIISYAQGFMLLRQAAMQFGWTLNYGGIALMWRGGCIIRSVFLGKIKDAFERNPELQNLLLDDFFKSAVDNCQDSWRRVVSTGVQAGIPMPCFTTALSFYDGYRHEVLPANLIQAQRDYFGAHTYELLAKPGEFIHTNWTGHGGSVSSSSYNA

SEQ ID NO: 70 - protein, 832 aa, Cricetulus griseus
MEEEVVNKHKPWLEPTYHGIVTENDNTVLLDPPLIALDKDSPLRFAGEICGFKIHGQNVPFDAVVVDKSTGEGIIRSKEKLDCELQKDYTFTIQAYDCGKGPDGTGVKKSHKATVHIQVNDVNEYAPVFKEKSYKAAVVEGKQHGSILRVEAVDADCSPQFSQICSYEILTPDVPFTVDKDGYIKNTEKLNYDKEHQYKLTVTAYDCGKKRATEDALVKISIKPACSPGWQGWSNRIEYEPGTGALAVFPSIHLETCDEPVTSVQATVELETSHIGKGCDRDTYSEKSLHRLCGAAAGTSELLPSPSGSLNWTVGLPTDNGHDSDQVFEFNGTQAVRIPDGVVSLDPKEPFTISVWMRHGPFGRKKETILCSSDKTGGDLHMTQFFRGNLAGLTIRSGKLADKKVIDCLYTCKEGLDLQVPEDGGRGVQIHASSSQAVLTLEGDDVGELDKAMQHVSYLNSRQFPTPGIRRLKITSTVKCFNEAACIEVPPVEGYVMVLQPEEPKISLSGVHHFARAASEFESPEGVSLFPELRIISTITREVEPEGDGSEDPTVQESLVSEEIVHDLDTCEVTVEGEELNPEQESLEVDMARLQQKGIEASHSDLGVVFTGVDTMASYEEVLHLLRYRNWHTRSLLDRKFKLICSELNGRYLSNEFKVEVNVIHTANPVEHANHMAAQPQFVHPEHRSFVDLSGHNLASPHPFAVVPSTATVVIVVCVSFLVFMIILGVFRIRAAHQRTMRDQDTGKENEMDWDDSALTITVNPMETYEDQHSPEEEEEEEEEEESEDGEEEEEITSAESESSEEEEGGPGDGQNATRQQQLEWDDSTLSY

SEQ ID NO: 71 - protein, 89 aa, Cricetulus griseus
MACPLDQAIGLLVAIFHKYSGKEGDKHTLSKKELKELIQKELTIGSKLQDAEIARLMDDLDRNKDQEVNFQEYVAFLGALALIYNEALK

SEQ ID NO: 72 - protein, 280 aa, Cricetulus griseus
MPREDRATWKSNYFLKIIQLLDDYPKCFIVGADNADSKQMQQIRMSLQGKAVVLMGKNTMMRKAIRGHLENNPALEKLLPHIRGNVGFVFTKEDLTEIRDMLLANKVPAAARAGAIAPCKVTVPAQNTGLGPEKTSFFQALGITTKTSRGTIEILSDVQLIKTGDKVGASEATLLNMLNISSFSFGLIIQQVFDNSSIYNPEVLDVTEQTLHSRFLEGVRNVVSGCLQIGYPTVASVPHSIINGYKRGLALSVETEYTFPLAEKVKAFLADPSTFAAAAL

SEQ ID NO: 73 - protein, 334 aa, Cricetulus griseus
MSEPIRVLVTGAAGQIAYSLLYSIGNGSVFGKDQPIILVLLDITPMMGVLDGVLMELQDCALPLLKDVIATDKEEVAFKDLDVAVLVGSMPRREGMERKDLLKANVRIFKAQGAALEKYAKKSVKVIVVGNPANTNCLTASKSAPSIPKENFSCLTRLDHNRAKSQIALKLGVTAEDVKNVIIWGNHSSTQYPDVNHAKVKLQGKEVGVYEALKDDSWLKGEFISTVQQRGAAVIKARKLSSAMSAAKAISDHIRDIWFGTPEGEFVSMGVISDGNSYGIPDDLLYSFPVVIKDKSWKFVEGLPINDFSREKMDLTAKELAEEKETAFEFLSSA

SEQ ID NO: 74 - protein, 592 aa, Cricetulus griseus
MWTLVSWLAFMAGLVAGTQCPDGQSCPIVCCLDPGGASYSCCNPILDTLPMVMSDRLSGICQVHDHCPGSYSCLLTVSGTSSCCPFPKGISCGDGYHCCPRGFHCSSDGTTCFRHSDSLLRAVQCPGSQFECPESSTCCVMLDGSWGCCPMPQASCCEDKIHCCPHGAFCDMIHTECISPRGTHPLLKKFPAQRKSRAVALHFSVVCPDAQTQCPDDSTCCELPSGKYGCCPMPNAVCCSDHLHCCPQDTVCDLIQSKCLSKKSTTYLLSRLFGNPVPILKEVECDSEVSCPDGYTCCYLTIGSWGCCPFSKAVCCEDHIHCCPEGFHCHTETGTCEMGGLRVPWMKKVKAPLSLLDAEIFQSDVPCDDFTVCPPDNTCCRLSSGGWGCCPIPEAVCCADHQHCCPKGFTCTAEGYCQGGNRMVAVLEKIHPHETFLSQIGDNNCDQHTSCPVGQTCCPSLKGDWACCQLPHAVCCEDRQHCCPTGYICNVKARTCEKAVNSIQIPVHLTLGPQVGEVECGTGHYCHDGQTCCRNSQGGWACCPYLEGTCCADGHHCCPIGFHCSVKGTKCFRRKIPHWDTSLTNPAPRQLL

SEQ ID NO: 75 - protein, 509 aa, Cricetulus griseus
MLPAVLTSLLGPFLVAWVLPLARGQTPNYTRPVFLCGGDVTGESGYVASEGFPNLYPPNKKCIWTITVPEGQTVSLSFRVFDMELHPSCRYDALEVFAGSGTSGQRLGRFCGTFRPAPVVAPGNQVTLRMTTDEGTGGRGFLLWYSGRATSGTGPPPGARRKWVMDPRVEWAAWGYWDEHQFCGGRMEKAQGTLTTPNWPESDYPPGISCSWHIIAPSDQVLTLLSRLPTSQCLYQVIMLTFGKFDVEPDTYCRYDSVSVFNGAVSDDSKRLGKFCGDKAPSPISSEGNELLVQFVSDLSVTADGFSASYKTLPRDAVEKELAPSPGEDVQLGPQSRSDPKTGTGPKVKPPSKPKFQPAEKPEVSPDTQETPVAPDPPSATCPKQYKRLGTLQSNFCASSLVVTGTVKTMVRGPGEGLTVTISLLGVYKSGGLDLPSPPTDTSLKLYVPCRQMPPMKKGASYLLMGQVEENRGPILPPESFLVPYKPNQDQILNNLRKRKCPSQPRPAA

SEQ ID NO: 76 - protein, 1126 aa, Cricetulus griseus
MAAVRTAPLLCGLLALLALCPGGSPQTVLTDDEIEEFLEGFLSELETQSPPREDDVEAQPLPEPTQRARKSKAGGKLRTDAEAPSEKNKDRGKKGKKDKGPKVTKQPLEGSTRPPKKGKEKTPKATKKPKEKPPKATKKPKEKPPKATKKPKEKPPKATKRPLAGKRLSTVAPLETLEWPLPPPSNPSPKELPQERGRTFPNTWQGQGEGTQVEAKEHQPEPEEETEAPTLDYNDQIEREDYEDFEYIRRQKQPRPTPSRKRLWPERPEEKAEEPEERKEIGPPLKPLLPPDYGDGYLIPNYDDMDYYFPHPPPQKPDVGQEVDEEKEEMKKPKKEGSSPKEETEDKWAVEKNKDHKGSRKGEDLEEEWAPVEKIKCPPIGMESHRIEDNQIRASSMLRHGLGAQRGRLNMQAGANEDDYYDGAWCAEDDSQTQWIEVDTRRTTRFTGIITQGRDSSIHDDFVTTFFVGFSNDSQTWVMYTNGYEEMTFHGNVDKDTPVLSELPDPVVARFIRIYPLTWNGSLCMRLEVLGCPVTPVHSYYAQNEVVITDNLDFRHHSYKDMRQLMKVVNEECPTITRTYSLGKSSRGLKIYAMEISDNPGEHELGEPEFRYTAGIHGNEVLGRELLLLLMQYLCREYRDGNPRVRSLVQDTRIHLVPSLNPDGYEVAAQMGSEFGNWALGLWSEEGFDIFEDFPDLNSVLWAAEEKKWVPYRVPNNNLPIPERYLSPDATVSTEVRAIIAWMEKNPFVLGANLNGGERFVSYPYDMARTPSQEQLLAAAMAAARGEDDEESSEAQETPDHAIFRWLAISFASAHLTMTEPYREGCQAQDYTNGMGIVNGAKWNPRSGTINDFSYLHTNCLELSIYLGCDKFPHESELPREWENNKEALLTFMEQVHRGIKGVVTDEQGIPIANATISVNGINHGVKTASGGDYWRILNPGEYRVTAHAEGYTSSAKTCNVDYDIGATQCNFILARSNWKRIREILAMNGNRPILRIDPSRPMTPQQRRMQQRRLQYRLRMREQMRLRRLNATTDPVTSPTPPPTPPPSPTPGITTRPWEIPPTTTTGWEESETETYTEIVTEFGTDYGTELEEEEMEEEEEEETVTGPTFPFTTVETYTVNFGDF

SEQ ID NO: 77 - protein, 781 aa, Cricetulus griseus
MSXXXXXXXXXXXXXXXXXXXXXXXXXXXXXXXXXXXXXXXXXXXXXXXXXXXXXXXXXXXXXXXXXXXXXXXXXXXXXXXXXXXXXXXXXXXXXXXXXXXXXXXXXXXXXXXXXXXXXXXXXXXXXXXXXXXXXXXXXXXXXXXXXXXXXXXXXXXXXXXXXXXXXXXXXXXXXXXXXXXXXXXXXXXXXXXXXXXXXXXXXXXXXXXXXXXXXXXXXXXXXXXXXXXXXXXXXXXXXXXXXXXXXXXXXXRSCSEVRQIYGAKGFSLSDVPQAEISGEHLRICPQGYTCCTSEMEENLANHSRMELETALHDSSRALQATLATQLHGIDDHFQRLLNDSERTLQDAFPGAFGDLYTQNTRAFRDLYAELRLYYRGANLHLEETLAEFWARLLERLFKQLHPQLLPTDDYLDCLGKQAEALRPFGDAPRELRLRATRAFVAARSFVQGLGVASDVVRKVAQVPLAPECSRAIMKLVYCAHCRGVPGARPCPDYCRNVLKGCLANQADLDAEWRNLLDSMVLITDKFWGPSGAENVIGGVHMWLAEAINALQDNKDTLTAKVIQGCGNPKVNPHDSGPEEKRRRGKLALQEKPPTGSLEKLVSEAKAKLRDIQDFWISLPGTLCSEKMAMSPASDDRCWNGISKGRYLPEVMGDGLANQINNPEVEVDITKPDMAIRQQIMQLKIMTNRLRGAYGGNDVDFQDASDDGSGSGSGGGCPDDTCGRRVSKKSSSSRTPLTHALPGLSEQEGQKTSAASCLEPHSFLLLLLVTLILAAARPRWR

SEQ ID NO: 78 - protein, 583 aa, Cricetulus griseus
MGRSWGAGGRGRRGLKGRRTQVGLPRSLATRNDPVSDFRSLPYPTSSRARDPTTMWKHWLALALVAVALVHGEEEPRSKSKICANVFCGAGRECAVTEKGEPTCLCIEQCKPHKRPVCGSNGKTYINHCELHRDACLTGSKIQVDYDGHCKVVCYQANRDELRRRIIQWLEAEIIPDGWFSKGSNYSEILDKYFKNFDNGDSHLDSSEFLKFVEQNETAINITTYADQENNKLLRGLCVDALIELSDENADWKLNFQEFLKCLNPSFNPPEKKCALEDETYADGAETEVDCNRCVCSCGHWVCTAMTCDGKTQKGAQTQTQEEMTRYAQELQKHQVLNLSGNCFQEVPASLLELSRLQTLSLGGNQLQSIPAEIENLQRLECLYLGGNFIKEIPPELANLPSLNYLVLCDNKIQSVPPQLSQLHSLRSLSLHNNLLTYLPREILNLIHLEELSLRGNPLVVRFVRDLTYDPPTLLELAARTIKIRSISYTPYDLPGNLLRYLGSASNCPNPKCGGVYFDCCVRQIKFVDFCGKYRLPLMHYLCSPECSSPCSSATHSSTSQSESDSEDEASVAAHRMQKVLLG

SEQ ID NO: 79 - protein, 444 aa, Cricetulus griseus
MSIVDCTANTNTCNKYGVSGYPTLKIFRDGEEAGAYDGPRTADGIVSHLKKQAGPASVPLRSEEEFKKFISDKDASVVGFFRDLFSDGHSEFLKAASNLRDNYRFAHTNVESLVKEYDDNGEGITLFRPSHLANKFEDKTVVYTEQKMTSGKIKRFIQESIFGICPHMTEDNKDLIQSKDLLTAYYDVDYEKNAKGSNYWRNRVMMVAKKFLDAGHKLNFAVASRKTFSHELSDFGLESTTGEVPVVAIRTAKGEKFVMQEEFSRDGKALERFLQDYFDGNLKRYLKSEPIPETNDGPVKVVVAENFDDIVNNEDKDVLIEFYAPWCGHCKNLEPKYKELGEKLSKDPNIVIAKMDATANDVPSPYEVKGSIPSSFIGPFIYVLFVTVGICVIEDSFGELVLSSCHLGGRELNDFINYLQREATTPPIIQEEKPKKKKKAQEDL

SEQ ID NO: 80 - protein, 216 aa, Cricetulus griseus
MAAQGEPPVQFKLVLVGDGGTGKTTFVKRHLTGEFEKKYVATLGVEVHPLLFHTSRGPIKFNVWDTAGQEKFGGLRDGYYIQAQSAIIMFDVTSRVTYKNVPNWHRDLVRVCENIPIVLCGNKVDVKDRKVKAKSIVFHRKKNLQYYDISAKSNYNFEKPFLWLSRRLTGDPNLEFVAMPALAPPEVIMDPVLAMKYERDLEVAQATALPDEEDDL

SEQ ID NO: 81 - protein, 245 aa, Cricetulus griseus
MEKTELILKAKLAEQAERYDDMATCMKAVTEQGAELSNEERNLLSVAYKNVVGGRRSAWRVISSIEQKTDTSDKKLQLIKDYREKVESELRSICTTVLELLDKYLIANATNPESKVFYLKMKGDYFRYLAEVACGDDRKQTIDNSQGAYQEAFDISKKEMQPTHPIRLGLALNFSVFYYEILNNPELACTLAKTAFDEAIAELDTLNEDSYKDSTLIMQLLRDNLTLWTSDSAGEECDAAEGAEN

SEQ ID NO: 82 - protein, 999 aa, Cricetulus griseus
MAATVRRQRPRRLLCWTLVAILLADLLALSDTLAVMSVDLGSESMKVAIVKPGVPMEIVLNKESRRKTPVTVTLKENERFLGDSAAGMAIKNPKATLRYFQHLLGKQADNPHVALYRDRFPEHELNIDPQRQTVRFQISPQLQFSPEEVLGMVLNYSRSLAEDFAEQPIKDAVITVPAFFNQAERRAVLQAARMAGLKVLQLINDNTATALSYGVFRRKDINSTAQNVMFYDMGSGSTVCTIVTYQTVKTKEAGMQPQLQIRGVGFDRTLGGLEMELRLREHLAKLFNEQRRGQKAKDVRENPRAMAKLLREANRLKTVLSANADHMAQIEGLMDDVDFKAKVTRVEFEELCADLFERVPGPVQQALQSAEMSLDEIEQVILVGGATRVPKVQEVLLKAVGKEELGKNINADEAAAMGAVYQAAALSKAFKVKPFVVRDAVIYPILVEFTREVEEEPGVRSLKHNKRVLFSRMGPYPQRKVITFNRYSHDFNFHINYGDLGFLGPEDLRVFGSQNLTTVKLKGVGESFKKYPDYESKGIKAHFNLDESGVLSLDRVESVFETLVEDSPEEESTLTKLGNTISSLFGGGTSSDAKENGTDAVQEEEESPTEGSKDEPGEQGDLKEETEAPVEDTSQPPPPEPKGDAAPEGEKPDEKESGGKSEAQKPEEKGQSGPEGVPPAPEEEKKQKPARKQKMVEEIGVELAVLDLPDLPEDELARSVKKLEDLTLRDLEKQEREKAANSLEAFIFETQDKLYQPEYQEVSTEEQREEISGKLSATSTWLEDEGFGATTVMLKEKLAELKKLCQGLFFRVEERRKWPERLSALDNLLNHSSIFLKGARLIPEMDQIFTEVEMTTLEKVINDTWAWKNATLAEQAKLPATEKPVLLSKDIEAKMMALDREVQYLLNKAKFTKPRPRPKDKNGTRTEPPLNATAGDQEEKVIPPAGQPEEAKPILEPDKEETTTEPTDSEPLELGGPGAESEPKEQTAGQKRSSKNDEL

SEQ ID NO: 83 - protein, 346 aa, Cricetulus griseus
MAAGTLYTYPENWRTFKTLIAAQYSGAQVRVLSAPPHFHFGQTNRTPEFLRKLPAGKVPAFEGDDGFCVFESNAIAYYVINEDLRGSTPEAAAQGVEWVSFADSDIVPPASTWVFPTLGIMHHNKQATKNAKEDVKQILGLLDTHLKTRTFLVGGRVTLADITVVCTLLWPYKQVLEPSFHQAFPNTNRWFLTCINQPQFRAVLGEVKLCEKMAQFDAKKFAESQPKKETPRKEKGSREEKQKPQAERKEEKKAAAPAPEEEMDECEQALAAEHKAKDPFAHLPKSTFVLDEFKRKYSNEDTLSVAMPYFWEHFDKDGWSLWYAEYRFPEELIQTFMSCNLITGMF

SEQ ID NO: 84 - protein, 236 aa, Cricetulus griseus
MLISLLLWLFRFRLNSSCLLILTMSGRGKQGGKARAKAKTRSSRAGLQFPVGRVHRLLRKGNYSERVGAGAPVYLAAVLEYLTAEILELAGNAARDNKKTRIIPRHLQLAIRNDEELNKLLGRVTIAQGGVLPNIQAKPHRYRPGTVALREIRRYQKSTELLIRKLPFQRLVREIAQDFKTDLRFQSSAVMALQEACEAYLVGLFEDTNLCAIHAKRVTIMPKDIQLARRIRGERA

SEQ ID NO: 85 - protein, 262 aa, Cricetulus griseus
MSGRGKQGGKARAKAKTRSSRAGLQFPVGRVHRLLRKGNYSERVGAGAPVYLAAVLEYLTAEILELAGNAARDNKKPPTIPRPLQLAIRNDEELNKLLGRVTIAQGGVLPNIQAVLLPKKTESHHKAKGKSSVRSAACCIKACSQLKAQCFSSQRFTVTMSGRGKGGKGLGKGGAKRHRKVLRDNIQGITKPAIRRLARRGGVKRISGLIYEETRGVLKVFLENVIRDAVTYTEHAKRKTVTAMDVVYALKRQGRTLYGFGG

SEQ ID NO: 86 - protein, 179 aa, Cricetulus griseus
MKEEDVLKFLAAGTHLGGTNLDFQMEQYIYKRKSDGIYIINLKRTWEKLLLAARAIVAIENPADVSVISSRNTGQRAVLKFAAATGATPIAGRFTPGTFTNQIQAAFREPRLLVVTDPRADHQPLTEASYVNLPTIALCNTDSPLRYVDIAIPCNNKVRVLVESSGKPLISVHIVRAWS

SEQ ID NO: 87 - protein, 451 aa, Cricetulus griseus
MRECISIHVGQAGVQIGNACWELYCLEHGIQPDGQMPSDKTIGGGDDSFNTFFSETGAGKHVPRAVFVDLEPTVIDEVRTGTYRQLFHPEQLITGKEDAANNYARGHYTIGKEIIDLVLDRIRKLADQCTGLQGFLVFHSFGGGTGSGFTSLLMERLSVDYGKKSKLEFSIYPAPQVSTAVVEPYNSILTTHTTLEHSDCAFMVDNEAIYDICRRNLDIERPTYTNLNRLIGQIVSSITASLRFDGALNVDLTEFQTNLVPYPRIHFPLATYAPVISAEKAYHEQLSVAEITNACFEPANQMVKCDPRHGKYMACCLLYRGDVVPKDVNAAIATIKTKRSIQFVDWCPTGFKVGINYQPPTVVPGGDLAKVQRAVCMLSNTTAIAEAWARLDHKFDLMYAKRAFVHWYVGEGMEEGEFSEAREDMAALEKDYEEVGVDSVEGEGEEEGEEY

SEQ ID NO: 88 - protein, 401 aa, Cricetulus griseus
MAEEDSRSSSWSTTEDEREEGSDDYRPKFKLFKENKVEIASAITKPFPFLMSLRDRGFLSEQKFQISKKQCKNLDAVRNVVYDILCDLQKDFSLPLLEVIFSPTHLKAYPDLQETRKIFQDDTMETGNNTTLGKSQEKRDTVETRNNTTVGKSQEKTNYRGAGGQAAVRRRQRKSNPEGSVRTVRRRARRLSRNEAVRFKAELLPVTCGRTKGVLHKDKFKLGLCRCRCPPSPVPAAMVNPTVFFDITANGQPLGRVSFELFADKLPKTAENFRALSTGEKGFGYKGSSFHRIIPGFMCQGGDFTRHNGTGGRSIYGEKFEDENFILKHTGPGILSMANAGPNTNGSQFFICTAKTEWLDGKHVVFGKVKEGMSTVEAMERFGSRTGKTSKKITISNCGQL

SEQ ID NO: 89 - protein, 445 aa, Cricetulus griseus
MREIVHIQAGQCGNQIGAKFWEVISDEHGIDPTGSYHGDSDLQLERINVYYNEAAGNKYVPRAILVDLEPGTMDSVRSGPFGQIFRPDNFVFGQSGAGNNWAKGHYTEGAELVDSVLDVVRKESESCDCLQGFQLTHSLGGGTGSGMGTLLISKIREEYPDRIMNTFSVMPSPKVSDTVVEPYNATLSVHQLVENTDETYSIDNKALYDICFRTLKLTTPTYGDLNHLVSATMSGVTTCLRFPGQLNADLRKLAVNMVPFPRLHFFMPGFAPLTSRGSQQYRALTVPELTQQMFDSKNMMAACDPRHGRYLTVAAIFRGRMSMKEVDEQMLNVQNKNSSYFVEWIPNNVKTAVCDIPPRGLKMSATFIGNSTAIQELFKRISEQFTAMFRRKAFLHWYTGEGMDEMEFTEAESNMNDLVSEYQQYQDATADEQGEFEEEEGEDEA

SEQ ID NO: 90 - protein, 801 aa, Cricetulus griseus
MQDAENVAAPEAAEERAEPARQQPASESPPADETVGSGGSEVGQTEDAEEEAGPEPEVRAKRAAQPEEETATSPAVSPPPQPAERSSAQEPSAPGKAEASGEQAREHSVAGAEEEGGSDGSSPEAEPRALENGEADEPSFSDPEDFVDDVSEEELLGDILKDRPQEADGIDSVIVVDNVPQVGPDRLEKLKNVIHKIFSKFGKIINDYYPEEDGKTKGYIFLEYASPAHAVDAVKNADGYKLDKQHTFRVNLFTDFDKYMTISDEWDIPEKQPFKDLGNLRYWLEEAECRDQYSVIFESGDRTSIFRNDVKDPVSIEERARWTETYVRWSPKGTYLATFHQRGIALWGGEKFKQIQRFSHQGVQLIDFSPCERYLVTFSPLMDTQDDPQAIIIWDILTGHKKRGFHCESSAHWPIFKWSHDGKFFARMTLDTLSIYETPSMGLLDKKSLKISGIKDFSWSPGGNIIAFWVPEDKDIPARVTLMQLPTRQEIRVRNLFNVVDCKLHWQKNGDYLCVKVDRTPKGTQGVVTNFEIFRMREKQVPVDVVEMKETIIAFAWEPNGSKFAVLHGEAPRISVSFYHVKSNGKIELIKMFDKQQANTIFWSPQGQFVVLAGLRSMNGALAFVDTSDCTVMNIAEHYMASDVEWDPTGRYVVTSVSWWSHKVDNAYWLWTFQGRLLQKNNKDRFCQLLWRPRPPTLLSQDQIKQIKKDLKKYSKIFEQKDRLSQSKASKELVERRRTMMEDFRQYRKMAQELYMKQKNERLELRGGVDTDELDSNVDDWEEETIEFFVTEEIIPLGSQE

SEQ ID NO: 91 - protein, 490 aa, Cricetulus griseus
MASRASELPPGRSVTAGIIIVGDEILKGHTQDTNTYFLCRTLRSLGVQVCRVSVVPDEVATIAAEVTSFSSRFTHVLTAGGIGPTHDDVTFEAVAQAFGEELKPHPELQAAIKTLGGVGWEKLSLVPSSASLHYGTDPRTGQPFTFPLVSVRNVYLFPGIPELLRRAMEGLKGLFQNTAVQFHVKELYVAAPEGSIASILTEAQAHFGRRLSLGSYPDWGSNYYQVKLILDSEEKEPLEECLAYLTARLPQGSLVPYLPNAVEQAGEAVYKLAQSGSCLGKKVASALQTIETALDQYHLSKLCVGFNGGKDCTALLHLFHAAVQRKFPDVPKPLQILYIRSISPFPELEQFLQDTIKRYNLQVLEAEGNMKQALGELQEKHPQLEAVLMGTRRTDPYSCSLSHFSPTDPGWPSFMRINPLLDWTYRNIWDFLRQLFVPYCILYDRGYTSLGSRENTMQNPALKCLSPGGHPVYRPAYLLENEDEERNSRT

SEQ ID NO: 92 - protein, 1069 aa, Cricetulus griseus
MADMASYKDAASSRHLRFKLQSLSRRLDELEEATKNLQKAEDELLDLQEKVIQAEGSNSSMLAEIEVLRQRVLKIEGKDEEIKRAEDLCHTMKEKLEEEENLTRELKSEIEWLQKRMADLEKLEEALSRSKNECSQLCLSLNEERNLTKKISSELEMLRVKVKELESSEDRLDKTEQSLVSELEKLKSLTLSFVNERKYLNEKEKENEKLIKELTQKLEQNKKMSRDHTRNASTLLERNDLRIEDGISSTLPSKELRRKGSLDYLKQVENETRDKSENEKNQNQEDNKVKDLNQEIQKLKTQIKHFESLEEELKKMRAKNNDLQDNYLTELNKNKILASQLEEIKLQVKKQKELGNGDIEGEDAFLLGRGRHERTKLRGHGGEASVSRHIPRELSPQHKRERIRNREFALNNENYSLSNKQASSIFTNRRAAKASNMGVGADNGSQETKRAEDRFLPGSSQSEGKKCREQPSVLSRYPPAAQEHNKVWKGTLKPGTESGLKGKVEKTTRTFSDSTHGPVPNDTMGRGDKTSEISEAHYGKRGQVPGNGSQVTQAAESGCSKATGALSSSQRASSEGISKSKRAANGLEADANFPNSKAPILSKYPYSSRSQENIPQGFSVPNKEGLDQSVAVVMEDSSQHEALRCRVIKSSGKEKPDSDDDLDIESLVTAKLVNTTITPEPEPKQQPNSREKVKSRGPRTALFENDKNAATENESMKSTRASSSAVEFPDANGVGAKNQRLFSPREALRSRAIIKPVIIDKDVKKIMGGSGTEVVLEKQRSTSNPVPSKVTSSITIYPSESSGPRAVQGEAPRERHTSTSNIQVGHPELTSVSNHVNSPLELSIHKHDITLQLTEAERMGDGSPKNRPETVVSRSSILIKPSDSVERNSHAPQAETVRWKSHNASSEVGSSDTRHVTVRNAWKSKRDFKCSEDVPTRVGRHMESTNAYTQRSSTDFLELEQPRSLPSEQGTRKVGDAGDAPELSSRRTQSSLTASEVITRRNRIGDAITATTWNHSASLEEGEDGTSVTSRRMHNTLEHSELPGKQGLPEPGIWAEERLQPARPYAEED

SEQ ID NO: 93 - protein, 417 aa, Cricetulus griseus
MRSLLLASFCLLAVALAAEVKKPVEAAAPGTAEKLSSKATTLAERSTGLAFSLYQAMAKDQAVENILLSPLVVASSLGLVSLGGKATTASQAKAVLSAEKLRDEEVHTGLGELLRSLSNSTARNVTWKLGSRLYGPSSVNFAEDFVHSSKQHYNCEHSKINFRDKRSALQSINEWASQTTDGKLPEVTKDVERTDGALLVNAMFFKPHWDEKFHHKMVDNRGFMVTRSYTVGVTMMHRTGLYNYYDDEKEKLQILEMPLAHKLSSLIILMPHHVEPLERLEKLLTKEQLKAWMGKMQKKAVAISLPKGVVEVTHDLQKHLAGLGLTEAIDKNKADLSRMSGKKDLYLASVFHATAFEWDTDGNPFDQDIYGREELRSPKLFYADHPFIFLVRDNQSGSLLFIGRLVRPKGDKMRDEL

SEQ ID NO: 94 - protein, 351 aa, Cricetulus griseus
MSPRSCLRSLRLLVFAVFSAAASNWLYLAKLSSVGSISEEETCEKLKGLIQRQVQLCKRNLEVMDSVRRGAQLAIEECQYQFRNRRWNCSTLDSLPVFGKVVTQGTREAAFVYAISSAGVAFAVTRACSSGELEKCGCDRTVHGVSPQGFQWSGCSDNIAYGVAFSQSFVDVRERSKGASSSRALMNLHNNEAGRKAILTHMRVECKCHGVSGSCEVKTCWRAVPPFRQVGHALKEKFDGATEVEPRRVGSSRALVPRNAQFKPHTDEDLVYLEPSPDFCEQDMRSGVLGTRGRTCNKTSKAIDGCELLCCGRGFHTAQVELAERCGCRFHWCCFVKCRQCQRLVEMHTCR

SEQ ID NO: 95 - protein, 263 aa, Cricetulus griseus
MAPYYKKLGRDALLSWDDVLAVQSLYGKPLGRSVATQLPGKLFTDFEAWDPHNSRRIRPETRGPKYCHSSFDAITVDRQWRLYIFKGSYFWEVTADGNVSEPRPLQKRWPGLPPDIEAAAVSLEDGDFYFFKGSRCWRFQGTKSVWGHSQLCRGGRLPRHPDAALFFPPLRRLVLFKGSRYYVLARGGKQVEPYYPRSLRDWAGVPEEVSGALPRPDGSVVFFRDDHYWQLDQAKLRVTSSGRWATELSWMGCWNANSGGALF

SEQ ID NO: 96 - protein, 442 aa, Cricetulus griseus
MPAIAVLAAAAAAWCFLQVDSRHLDALAGGAALNNANFLDNDQWLSTVSQYDRDKYWNRFRDEVEDDYFRNWNPNKPFDQALDPSKDPCLKVKCSPHTVCVTQDYQTALCVSHKHLLPRQKKGNVAHKHWAGPSNLVKCKPCPVAQSAMVCGSDGHTYTSKCKLEFHACSTGKSLSSLCDGPCPCLPEPEPPKPKAEKSACTDKELRNLASRLKDWFGALHEDANRVIKPTSSDTAQGRFDTSILPICKDSLGWMFNKLDMNYDLLLDHSEINAIYLDKYEPCIKPLFNSCDSFKDGKLSNNEWCYCFQKPGGLPCQNEMNRIQKLSKGKSLLGAFIPRCNEEGYYKATQCHGSTGQCWCVDKYGNELAGSRKQGAVSCEEEQETSGDFGSGGSVVLLDDLEDERELGPKDQEGKLRVHTRAVREDDEDEDDDKDDEVGYIW

SEQ ID NO: 97 - protein, 417 aa, Cricetulus griseus
MPPRPGRLLPSLAGLPALAALLLLLGSRRGARAQEAAADGGAEQDPHAKHLYTADMFTHGIQSAAHFVMFFAPWCGHCQRLQPTWNDLGDKYNSMEDAKVYVAKVDCTANSDVCSAQGVRGYPTLKFFKPGQEAVKYQGPRDFETLENWMLQTLKEEPPTPEPEAEPPKAPELKQGLYELSANNFELHVSQGDHFIKFFAPWCGHCKALAPTWEQLALGLEHSETVKIGKVDCTQHYGLCSENQVRGYPTLLWFRDGKKVDQYKGKRDLESLRDYVESQMQDPEVAPETVEPSEAPVLAAEPTGDKGTVLALTEKNFEDTIAQGITFVKFYAPWCGHCKNLAPTWEELSKKEFPGLAEVTVAKVDCTAERNVCTKYSVRGYPTLLLFRGGEKVGEHNGGRDLDSLHSFVLRQAKDEL

SEQ ID NO: 98 - protein, 390 aa, Cricetulus griseus
MPPSGLRLLPLLLPLPWLLVLTPGRPAVGLSTCKTIDMELVKRKRIEAIRGQILSKLRLASPPSQGEVPPGPLPEAVLALYNSTRDRVAGESADPEPEPEADYYAKEVTRVLMVDRSNPIYDKTKDIPHSVYMFFNTSDIREAVPEPPLLSRAELRLQRFKSSVEQHVELYQKFSNNSWRYLGNRLLSPTDTPEWLSFDVTAVVRQWLNQGDGIQGFRFSAHCSCDSKDNVLHVEINGISPKRRGDLGTIHDMNRPFLLLMATPLERAQHLHSSRHRRALDTNYCFSSTEKNCCVRQLYIDFRKDLGWKWIHEPKGYHANFCLGPCPYIWSLDTQYSKVLALYNQHNPGASASPCCVPQALEPLPIVYYVGRKPKVEQLSNMIVRSCKCS

SEQ ID NO: 99 - protein, 1888 aa, Cricetulus griseus
MEEKKKKKQEDKKKKEGAQKKAADQKTKVPELTKTCSSQPQPAGTGTASTSTISSSSNGKRASACGQQPAASRYLPREVPPRFRQQEQKQLLKRGQPLPTGTLTSVSPAGASPPPLPGAGTQQHPSKLQPDPGHSGLADHYENSHWGQQPSYRSEANCGWDKVTLDRTDQEVWPSIPVTETESASECPADTDSASTCGSENSSMATGSTQGSFTGHPKKTNGNNGTNGALVQSPSNQSALGAGGTNGNGGVARVWGVATGSSSGLTHCSVGGGDGKMDNMIGDGRSQNCWGASNSNAGINLNLNPNANPAAWPVLGHEGTVATGNPSSICSPVSAIGQNMGSQNGNPVGTVGAWGNLLPQESTEPQTSTCQNVSFSVQPQNLNTDGSNNTNPMNSSPNPINAMQTNGLPNWGMAVGMGAIIPPHLQGLPGANGSSVSQGSGSGGEGMGSSVWGLSPGNPATGNNNSGFSQGNGDTVNSALSAKQNGSSSAVQKEGNGGNAWDSGPPAGPGILAWGRGSGNNGIGNIHSGAWGHPSRSSSNGMNGEWGKLPNQHSSSDISGKGSTGWDSPSAASQPPALQPGSEHVSSWAKATSSGTTPSEGSSDGSGHHSEGGAGREAMGEGRRRDQGHIQLPRGDLDPRVLSNTGWGQTPVKQNTAWEFEESPRSERKNDNGTEAWGSAATQPSNSGGKSDGSLMNSTNTSSVSGWVSSPPAAVPANTSWGDSNNKAPSGPGVWGDSISSTAVNNAAATKSGHAWSGTVNQEDKSPTWGEPQKPKSQNWGDGQRANPAWSAGAGDWADSSSVLGHLGDGKKNGPGWDADGNRSGSGWNDASRCGTSGWASGASAKVNPGTNWGESLKPGPQQSWAHKPQDSNVSNWGGAASVKQTGTGWIGGPLPVKQKDSCEATGWEEPSPPSIRRKMEIDDGTSAWGDPSTYNNKTVNMWDRNNPVIQSSTTTPATPTTPTSSSTTHQAETPPSHQAGTQLNRSPLLGPVSSGWGEMPSVHSKAENSWGEPSSPSPLVDNGTAAWGKPPSSGSGWDHPAEPVVPFGRASAPAAAPALCKPASKSMQEGWGSGGDEMNLGASQWEDEDGDMWNNGVSQEGSSSCSSWGNASKKGLQKGMKTPGKQDEAWIMSRLIKQLTDMGFPREPAEEALKSNSMNLDQAMSALLEKKVDMDKRGLGMTDYNGMVTKTLGCRPPISKESSMDRPTFLDKLTLSFSNQDGGLVEEPTTSPFLPSPSLKLPLSNSALPNQALGGIASGLGMQNLNSSRQIPSGNLGVFGNSGAAQARTMQQPPVQPLNSSQPSLRAQVPQFLSPQVQAQLLQFAAKNIGLSPALLTSPINPQHMTMLNQLYQLQLAYQRLQIQQQMLQAQRNVSGPMRQQEQQVARTITNLQQQIQQHQRQLAQALLVKQPPPPPPPPHLSLHPSAGKSAMDSFPPHPQTPGLPDLQTKEQQSSPNTFAPYPLAGLNPNMNVNSIDVSSGLSVKDSSQSQSRLPQWTHPNSMGNLSSAASPLDQNPSKHGAIPGGLSIGPPGKSSIDDSYGRYDLIQNSESPASPPVAVPHSWSRAKSDSDKISNGSSISWPPEFHPGVPWKGLQNIDPENDPDVTPGSVPTGPTINTTIQDVNRYLLKSGGKLSDIKSTWSSGPASHTQASLSHELWKVPRNTTAPTRPPPGLANPKPSSTWGTSPLGWTSSYSSGSAWSTDASGRTSSWLVLRNLTPQIDGSTLRTLCLQHGPLITFHLNLTQGNAVVRYSSKEEAAKAQKSLHMCVLGNTTILAEFAGEEEVNRFLAQGQALPPTSSWQPSSGGSQPRLGSSGSTHGLVRSDTAHWSTPCLSGKGSSELLWGGVPQYSSSLWGPPSADDARVIGSPTPLNTLLPGDLLSGESM

SEQ ID NO: 100 - protein, 563 aa, Cricetulus griseus
MDVGELLSYQPNRGTKRPRDDEEEELKTRRKQTGPRERGRYREEEATAAEETDDDKKRLLQIIDRDGEEEEEEEEPLDESSVKKMILTFEKRSYKNQELRIKFPDNPEKFMESELDLNDIIQEMHVVATMPDLYHLLVELSAVQSLLGLLGHDNTDVSIAVVDLLQELTDIDTLHESEEGAEVLIDALVDGQVVALLVQNLERLDESVREEADGVHNTLAIVENMAEFRPEMCTEAAQQGLLQWLLKRLKAKMPFDANKLYCSEVLAILLQDNDDNRELLGELDGIDVLLQQLSVFKRHNPSTAEEQEMMENLFDALCSCLMLSSNRERFLKGEGLQLMNLMLREKKISRSSALKVLDHAMIGPEGTDNCHKFVDILGLRTIFPLFMKSPRKIKKVGTTEKEHEEHVCSILASLLRNLRGQQRTRLLNKFTENDSEKVDRLMELHFKYLGAMQVADKKIEGEKHDIVRRGEIIDNDLEDEFYLRRLDAGLFILQHICYIMAEICNANVPQIRQRVHQILNMRGSSIKIVRHIIKEYAENIGDGRSPEFRETEQKRILGLLENF

SEQ ID NO: 101 - protein, 686 aa, Cricetulus griseus
MAEELLLERCDLEIQANGRDHHTADLCHEKLVLRRGQRFRLTLYFVGRGYEASVDSLTFGAVTGPAPSEETGTKVRFPLSDDVQEGSWTASVLDQRDNVLALQLCTPANAPVGQYRLSLEVSSGYQGSSYVLGHFILLFNAWCPADDVYLDSEEQRREYVLTQQGFIYQGSVKFIKSVPWNFGQFEDGILDICLMLLDVNPKFLKDSARDCSRRRSPIYVGRVVSGMVNCNDDQGVLLGRWDNNYGDGVSPMAWIGSVDILRRWKEHGCQQVKYGQCWVFAAVACTVLRCLGIPTRVVTNYNSAHDQNSNLLIEYFRNEFGELESNKSEMIWNFHCWVESWMTRPDLEPGYEGWQAIDPTPQEKSEGTYCCGPVSVRAIKEGDLSTKYDAPFVFAEVNADVVDWIRQEDGSVHKSINRSLIVGQKISTKSVGRDEREDITHTYKYPEGSPEEREAFTRANHLNKLAEKEETGVAMRIRVGESMNMGNDFDVFAHIGNDTSESRDCHLLLCARTVSYNGVLGPECGTENLNLTLDPFSENTIPLRILYEKYSECLTESNLIKVRGLLVEPASNSYLLAERDLYLENPEIKIRILGEPKQNRKLVAEVSLRNPLSEPLNDCIFTVEGAGLTKEQKSVEVPDPVPAGEVGKVRVDFFPTEIGLHKLVVNFQCDKLKSVKGYRNVIIGPA

SEQ ID NO: 102 - protein, 967 aa, Cricetulus griseus
MDDSEVESTASILASVKEQEAQFEKLTRALEEERRHVSAQLERVRVSPQDANPLMANGTLTRRHQNGRFMGDADLERQKFSDLKLNGPQDHNHLLYSTIPRMQEPGQIVETYTEEDPEGAMSVVSVETSDDGTTRRTETTVKKVVKTVTTRTVQPVPMGPDGLPVDASSVSNNYIQTLGRDFRKNGNGGPGPYVGQAGTATLPRNFHYPPDGYGRHYEDGYPGGSDNYGSLSRVTRIEERYRPSMEGYRAPSRQDVYGPQPQVRVGGSSVDLHRFHPEPYGLEDDQRSMGYDDLDYGMMSDYGTARRTGTPSDPRRRLRSYEDMIGEEVPPDQYYWAPLAQHERGSLASLDSLRKGVPPPPNWRQPELPEVIAMLGFRLDAVKSNAAAYLQHLCYRNDKVKTDVRKLKGIPVLVGLLDHPKKEVHLGACGALKNISFGRDQDNKIAIKNCDGVPALVRLLRKARDMDLTEVITGTLWNLSSHDSIKMEIVDHALHALTDEVIIPHSGWEREPNEDCKPRHIEWESVLTNTAGCLRNVSSERSEARRKLRECDGLVDALIFIVQAEIGQKDSDSKLVENCVCLLRNLSYQVHREIPQAERYQEALPSVANSTGPHAASCFGAKKGKDEWFSRGKKPTEDPANDTVDFPKRTSPARGYELLFQPEVVRIYISLLKESKTPAILEASAGAIQNLCAGRWTYGRYIRSALRQEKALSAIADLLTSEHERVVKAASGALRNLAVDARNKELIGKHAIPNLVKNLPGGQQNSSWNFSEDTVVSILNTINEVIAENLEAAKKLRETQGIEKLVLINKSGNRSEKEVRAAALVLQTIWGYKELRKPLEKEGWKKSDFQVNLNNASRSQSSHSYDDSTLPLIDRNQKSDKKPDREEIPMSNMGSNTKSLDNNYSTLNERGDHNRTLDRSGDLGDMEPLKGAPLMQDEGQESLEEELDVLVLDDEGDQVSYSPMQKI

SEQ ID NO: 103 - protein, 410 aa, Cricetulus griseus
MLLQRALVVLALLNLATVSFSLSTCTTLDFGHIKKKRVEAIRGQILSKLRLTSPPEPSVMTHVPYQVLALYNSTRELLEEMHGEREEGCTQENTESEYYAKEIHKFDMIQGLAEHNELAVCPKGITSKVFRFNVSSVEKNGTNLFRAEFRVLRVPNPSSKRTEQRIELFQILRPDEHIAKQRYIGGKNLPTRGTAEWLSFDVTDTVREWLLRRESNLGLEISIHCPCHTFQPNGDILENVHEVMEIKFKGVDNEDDHGRGDLGRLKKQKDHHNPHLILMMIPPHRLDSPGQGGQRKKRALDTNYCFRNLEENCCVRPLYIDFRQDLGWKWVHEPKGYYANFCSGPCPYLRSADTTHSTVLGLYNTLNPEASASPCCVPQDLEPLTILYYVGRTPKVEQLSNMVVKSCKCS

SEQ ID NO: 104 - protein, 1607 aa, Cricetulus griseus
MTGGGRAELALRPRGRLWPLLAVLAAAAGCVRAAMDECADEGGRPQRCMPEFVNAAFNVTVVATNTCGTPPEEYCVQTGVTGVTKSCHLCDAGQLHLQHGAAFLTDYNNQADTTWWQSQTMLAGVQYPNSINLTLHLGKAFDITYVRLKFHTSRPESFAIYKRTREDGPWIPYQYYSGSCENTYSKANRGFIRTGGDEQQALCTDEFSDISPLTGGNVAFSTLEGRPSAYNFDNSPVLQEWVTATDIRVTLNRLNTFGDEVFNDPKVLKSYYYAISDFAVGGRCKCNGHASECVKNEFDKLVCNCKHNTYGVDCEKCLPFFNDRPWRRATAESASECLPCDCNGRSQECYFDPELYRSTGHGGHCTNCRDNTDGAKCERCRENFFRLGNTEACSPCHCSPVGSLSTQCDSYGRCSCKPGVMGDKCDRCQPGFHSLTEAGCRPCSCNPSGSTDECNVETGRCVCKDNVEGFSCERCKPGFFNLESSNPKGCTPCFCFGHSSVCTNAVGYSVYDISSIFQIDEDGWRVEQRDGSEASLEWSSDRQDIAVISDSYFPRYFIAPAKFLGNQVLSYGQNLSFSFRVDRPDTRLSAEDLVLEGAGLRVSVPLIAQGNSYPSETAVKYIFRLHEATDYPWRPTLSPFEFQKLLNNLTSIKIRGTYSERSAGYLDDVTLASARPGPGVPATWVESCTCPVGYGGQFCETCLSGYRRETPSLGPYSPCVLCTCNGHSETCDPETGVCNCRDNTDGPHCERCSDGYYGDSTLGTSSDCQPCPCPGGSSCAIVPKTKEVVCTHCPTGTAGKRCELCDDGYFGDPLGSNGPVRLCRPCQCNDNIDPNAVGNCNRLTGECLKCIYNTAGFYCDRCKEGFFGNPLAPNPADKCKACACNPYGTVQQQSSCNPVTGQCECLPHVSGRDCGACEPGFYNLQSGQGCERCDCHALGSTNGQCDIQTGQCECQPGITGQHCERCETNHFGFGPEGCKPCDCHHEGSLSLQCKDDGRCECREGFVGNRCDQCEENYFYNRSWPGCQECPACYRLVKDKVAEHRVKLQELESLIANLGTGDETVTDQAFEDRLKEAEREVTDLLREAQDVKDVDQNLMDRLQRVNSSLHSQISRLQNIRNTIEETGILAEQARSRVESTEQLIEIASRELEKAKMAAANVSIAQPESTGEPNNMTLLAEEARRLAERHKQEADDIVRVANTANETSTEAYNLLLRTLEGENQTSLEIEDLNRKYEQAKNISQDLEKQAARVHEEAKRAGDKAVEIYASVAQLTPVDSEALENEANKIKKEAADLDRLIDQKLKDYEDLREDMRGKEHEVKNLLEKGKAEQQTADQLLARADAAKALAEEAAKKGRNTLQEANDILSNLKDFDRRVNDNKTAAEEALRRIPAINRTIAEANEKTREAQLALGNAAADATEAKNKAHEAERIASAVQKNATSTKADAERTFAEVTDLDNEVNVMLRQLEEAESELKEKQQVAEADMMMAGMASQAAQEAELNARKAKNSVSSLLSQLTDLLEQLGQLDTVDLNKLNEIEGTLNKAKDEMKVSDLDRKVADLESEARKQEAAIMDYNRDIEEIIKDIHNLEDIKKTLPSGCFNTPSIEKP

SEQ ID NO: 105 - protein, 4650 aa, Cricetulus griseus
MSEPGGGGGGGGGEDGSAGLEVSAVQNVADVAVLQKHLRKLVPLLLEDGGDAPAALEAALEEKSALEQMRKFLSDPQVHTVLVERSTLKEDVGDEGEEEKEFISYNINIDIHYGVKSNSLAFIKRTPVIDADKPVSSQLRVLTLSEDSPYETLHSFISNAVAPFFKSYIRESGKADRDGDKMAPSVEKKIAELEMGLLHLQQNIEIPEISLPIHPIITNVAKQCYERGEKPKVTDFGDKVEDPTFLNQLQSGVNRWIREIQKVTKLDRDPASGTALQEISFWLNLERALYRIQEKRESPEVLLTLDILKHGKRFHATVSFDTDTGLKQALETVNDYNPLMKDFPLNDLLSATELDKIRQALVAIFTHLRKIRNTKYPIQRALRLVEAISRDLSSQLLKVLGTRKLMHVAYEEFEKVMVACFEVFQTWDDEYEKLQVLLRDIVKRKREENLKMVWRINPAHRKLQARLDHMRKFRRQHEQLRAVIVRVLRPQVTAVAQQNQGEAPEPQDMKVAEVLFDAADANAIEEVNLAYENVKEVDGLDVSKEGTEAWEAAMKRYDERIDRVETRITARLRDQLGTAKNANEMFRIFSRFNALFVRPHIRGAIREYQTQLIQRVKDDIESLHDKFKVQYPQSQACKMSHVRDLPPVSGSIIWAKQIDRQLTAYMKRVEDVLGKGWENHVEGQKLKQDGDSFRMKLNTQEIFDDWARKVQQRNLGVSGRIFTIESARVRGRTGNVLKLKVNFLPEIITLSKEVRNLKWLGFRVPLAIVNKAHQANQLYPFAISLIESVRTYERTCEKVEERNTISLLVAGLKKEVQALIAEGIALVWESYKLDPYVQRLAETVFNFQEKVDDLLIIEEKIDLEVRSLETCMYDHKTFSEILNRVQKAVDDLNLHSYSNLPIWVNKLDMEIERILGVRLQAGLRAWTQVLLGQAEDKAEVDMDTDAPQVSHKPGGEPKIKNVVHELRITNQVIYLNPPIEECRYKLYQEMFAWKMVVLSLPRIQSQRYQVGVHYELTEEEKFYRNALTRMPDGPVALEESYSAVMGIVTEVEQYVKVWLQYQCLWDMQAENIYNRLGEDLNKWQALLVQIRKARGTFDNAETKKEFGPVVIDYGKVQSKVNLKYDSWHKEVLSKFGQMLGSNMTEFHSQISKSRQELEQHSVDTASTSDAVTFITYVQSLKRKIKQFEKQVELYRNGQRLLEKQRFQFPPCWLYIDNIEGEWGAFNDIMRRKDSAIQQQVASLQMKIVQEDRAVESRTTDLLTDWEKTKPVTGNLRPEEALQALTIYEGKFGRLKDDREKCAKAKEALELTDTGLLSGSEERVQVALEELQDLKGVWSELSKVWEQIDQMKEQPWVSVQPRKLRQNLDGLLNQLKNFPARLRQYASYEFVQRLLKGYMKINMLVIELKSEALKDRHWKQLMKRLHVNWVVSELTLGQIWDVDLQKNEAVVKDVLLVAQGEMALEEFLKQIREVWNTYELDLVNYQNKCRLIRGWDDLFNKVKEHINSVSAMKLSPYYKVFEEDALSWEDKLNRIMGLFDVWIDVQRRWVYLEGIFTGSADIKHLLPVETQRFQSISTEFLALMKKVSKSPLVMDVLNIQGVQRSLERLADLLGKIQKALGEYLERERSSFPRFYFVGDEDLLEIIGNSKNVAKLQKHFKKMFAGVSSIILNEDNSVVLGISSREGEEVMFKTPVSITEHPKINEWLTLVEKEMRVTLAKLLAESVTEVEIFGKATSIDPNTYITWIDKYQAQLVVLSAQIAWSENVENALSSVGGGGDMAPLQSVLSNVEVTLNVLADSVLMEQPPLRRRKLEHLITELVHQRDVTRSLIKSKIDNAKSFEWLSQMRFYFDPKQTDVLQQLSIQMANAKFNYGFEYLGVQDKLVQTPLTDRCYLTMTQALEARLGGSPFGPAGTGKTESVKALGHQLGRFVLVFNCDETFDFQAMGRIFVGLCQVGAWGCFDEFNRLEERMLSAVSQQVQCIQEALREHSNPNYDKTSAPITCELLNKQVKVSPDMAIFITMNPGYAGRSNLPDNLKKLFRSLAMTKPDRQLIAQVMLYSQGFRTAEVLANKIVPFFKLCDEQLSSQSHYDFGLRALKSVLVSAGNVKRERIQKIKREKEERGEAVDEGEIAENLPEQEILIQSVCETMVPKLVAEDIPLLFSLLSDVFPGVQYHRGEMTALREELKKVCREMYLTYGDGEEVGGMWVEKVLQLYQITQINHGLMMVGPSGSGKSMAWRVLLKALERLEGVEGVAHIIDPKAISKDHLYGTLDPNTREWTDGLFTHVLRKIIDNVRGELQKRQWIVFDGDVDPEWVENLNSVLDDNKLLTLPNGERLSLPPNVRIMFEVQDLKYATLATVSRCGMVWFSEDVLSTDMIFNNFLARLRSIPLDEGEDEAQRRRKGKEDEGEEAASPMLQIQRDAATIMQPYFTSNGLVIKALEHAFKLEHIMDLTRLRCLGSLFSMLHQACRNVAQYNANHPDFPMQIEQLERYIQRYLVYAILWSLSGDSRLKMRAELGEYIRRITTVPLPTAPNIPIIDYEVSISGEWSPWQAKVPQIEVETHKVAAPDVVVPTLDTVRHEALLYTWLAEHKPLVLCGPPGSGKTMTLFSALRALPDMEVVGLNFSSATTPELLLKTFDHYCEYRRTPNGVVLAPVQLGKWLVLFCDEINLPDMDKYGTQRVISFIRQMVEHGGFYRTSDQTWVKLERIQFVGACNPPTDPGRKPLSHRFLRHVPVVYVDYPGPASLTQIYGTFNRAMLRLIPSLRTYAEPLTAAMVEFYTMSQERFTQDTQPHYIYSPREMTRWVRGIFEALRPLETLPVEGLIRIWAHEALRLFQDRLVEDEERRWTDENIDMVALKHFPNIDKEKAMNRPILYSNWLSKDYIPVDQEELRDYVKARLKVFYEEELDVPLVLFNEVLDHVLRIDRIFRQPQGHLLLIGVSGAGKTTLSRFVAWMNGLSVYQIKVHRKYTGEDFDEDLRTVLRRSGCKNEKIAFIMDESNVLDSGFLERMNTLLANGEVPGLFEGDEYATLMTQCKEGAQKEGLMLDSHEELYKWFTSQVIRNLHVVFTMNPSSEGLKDRAATSPALFNRCVLNWFGDWSTEALYQVGKEFTSKMDLEKPNYIVPDYMPVVYDKLPQPPTHREAIVNSCVFVHQTLHQANARLAKRGGRTMAITPRHYLDFINHYANLFHEKRSELEEQQMHLNVGLRKIKETVDQVEELRRDLRIKSQELEVKNAAANDKLKKMVKDQQEAEKKKVMSQEIQEQLHKQQEVIADKQMSVKEDLDKVEPAVIEAQNAVKSIKKQHLVEVRSMANPPAAVKLALESICLLLGESTTDWKQIRSIIMRENFIPTIVNFSAEEISDAIREKMKKNYMSNPSYNYEIVNRASLACGPMVKWAIAQLNYADMLKRVEPLRNELQKLEDDAKDNQQKANEVEQMIRDLEASIARYKEEYAVLISEAQAIKADLAAVEAKVNRSTALLKSLSAERERWEKTSETFKNQMSTIAGDCLLSAAFIAYAGYFDQQMRQNLFTTWSHHLQQANIQFRTDIARTEYLSNADERLRWQASSLPADDLCTENAIMLKRFNRYPLIIDPSGQATEFIMNEYKDRKITRTSFLDDAFRKNLESALRFGNPLLVQDVESYDPVLNPVLNREVRRTGGRVLITLGDQDIDLSPSFVIFLSTRDPTVEFPPDLCSRVTFVNFTVTRSSLQSQCLNEVLKAERPDVDEKRSDLLKLQGEFQLRLRQLEKSLLQALNEVKGRILDDDTIITTLENLKREAAEVTRKVEETDIVMQEVETVSQQYLPLSTACSSIYFTMESLKQVHFLYQYSLQFFLDIYHNVLYENPNLKGATDHTQRLSVITKDLFQVAFNRVARGMLHQDHITFAMLLARIKLKGTLGEPTYDAEFQHFLRGNEIVLSAGSTPKIQGLTVEQAEAVMRLSCLPAFKDLIAKVQADEQFGIWLDSSSPEQTVPYLWSEETPSTPIGQAIHRLLLIQAFRPDRLLAMAHMFVSTNLGESFMSIMEQPLDLTHIVGTEVKPNTPVLMCSVPGYDASGHVEDLAAEQNTQITSIAIGSAEGFNQADKAINTAVKSGRWVMLKNVHLAPGWLMQLEKKLHSLQPHACFRLFLTMEINPKVPVNLLRAGRIFVFEPPPGVKANMLRTFSSIPVSRMCKSPNERARLYFLLAWFHAIIQERLRYAPLGWSKKYEFGESDLRSACDTVDTWLDDTAKGRQNISPDKIPWSALKTLMAQSIYGGRVDNEFDQRLLNTFLERLFTTRSFDSEFKLACKVDGHKDIQMPDGIRREEFVQWVELLPDTQTPSWLGLPNNAERVLLTTQGVDMISKMLKMQMLEDEDDLAYAETEKKTRTDSTSDGRPAWMRTLHTTASNWLHLIPQTLSPLKRTVENIKDPLFRFFEREVKMGAKLLQDVRQDLADVVQVCEGKKKQTNYLRTLINELVKGILPRSWSHYTVPAGMTVIQWVSDFSERVKQLQSISQAAASGGAKELKNIHVCLGGLFVPEAYITATRQYVAQANSWSLEELCLEVNVTASQSATLDACSFGVTGLKLQGATCTNNKLSLSNAISTVLPLTQLRWVKQTNAEKKANVVTLPVYLNFTRADLIFTVDFEIATKEDPRSFYERGVAVLCTE

SEQ ID NO: 106 - protein, 2941 aa, Cricetulus griseus
MRLRLLVAALCTAEVLVGAPGVWAQSRDRVTCTRLYAADIVFLLDGSSSIGRSNFREVRGFLEGLVLPFSGAASAQGVRFATVQYSDDPQTEFGLDALGSGGDTIRAIRELNYKGGNTRTGAALHHVSDRVFLPHLTRPNIPKVCILITDGKSQDLVDTAAQKLKGQGVKLFAVGIKNADPEELKRVASQPTSDFFFFVNDFSILRTLLPLISRRVCTTAGGVPVTLPFDDTPSGPRDLVLSEPSSQSLQVKWTAASGPVTGYKIQYTPLTGLGQPLPSERQEVNVPAGETSTRLQGLRPLTEYQVTVVALYANSIGEAVSGTARTTAEEGLELSVQNITSHSLLVAWRRVPGVTGYRVAWRDLSGGTTQQQDLSPGQGSVFLYHLEPGTDYEVTVSALYGHSVGPATSLTARTDSSVEQTLHPVILSPTSILLSWNLVPEARGYRLEWRRESGLEPPQKVVLPSDVTRHQLDGLQPGTEYRLTLYTLLEGREVATPATIVPTGPEQPVSEVMNLQAIELSGQRVRVSWNPVPSATEYRVTVRSTQGVERTLLLPGSQTSFNLDDVQAGISYTVRVSARVGSREGGASVLTIRRDPETQLTVPGLRVVASDSTRIRVTWGPVPGASGFRISWRTGSGPESSQTLPPDSTATDILGLQPGTSYHVAVSALRGREEGPPVVIVARTDPLGPVRRVHLTQAGSSSISIAWTGVPGATGYRVSWHSGHGPEKSQLVSGEATVAEIDGLEPDTEYTVRVRTHVAGVDGAPASVVVKTAPEPVGSVSKLQILNASSDVLRVTWVGVPGATAYRLAWGRSEGGPMRHQILPGNKDSAEIRGLEGGVSYSVRVTALVGDREGAPVSIVVTTPPEAPTPLESLQVVQRGEHSLRLRWERVPGALGFRLHWQPEGGQEQSLTLRPESNSYNLDGLEPATLYHIWLSVLGQTGEGPPRKVSAHTEPSPVLSTDLRVVDISTDSVTLAWTPVPDASSYILSWRPLRGTGQEVPGAPQTLPGTSSSHRVTGLDPGVSYVFSLAPIQRGVRGPEVSVTQKPACPHGQVDVVFVLHATRDNAHNAEAVRRALERLVSALGPLGPQAAQVGLLSYSHRPSPLFPLNSSRDLGIILQKIRDIPYVDPSGNNLGTAVITAHSHLLAPNAPGRRQRVPGVMVLLVDEPLRGDIFSPIREVQASGLKVMTLGLAGADPEQLRRLAPGLDPIQNFFATDNGPSLDRAVSDLAVALCQAAVATQPQPEPCAVHCPKGQKGEPGATGLQGQAGPPGPPGLPGRTGAPGPQGPPGSTQAKGERGFPGPVGPPGSPGLTGAPGSPGIKGSPGWPGPRGEPGERGPRGPKGEPGEPGEVIGGEGPGLPGKKGDPGPSGPPGPRGPLGDPGPRGSPGIPGTSVKGDKGDRGERGPPGPGIGGTGQGEPGLPGLPGSPGPQGPAGRAGEKGEKGDCEDGAPGLPGQPGAPGEPGLRGTPGITGPKGDRGQTGTPGEPGEKGERGPPGPVGPQGLPGVAGHPGVEGPEGPPGPAGRRGEKGEPGRPGDPAVGPGGAGAKGEKGDAGLPGPRGAAGIKGEQGPPGLALPGDPGPKGDPGDRGPIGLTGRAGPTGDSGPPGEKGDPGRPGPPGPVGPRGRDGEVGEKGVEGNPGDPGLPGKAGERGLRGAPGVRGPAGEKGDQGDPGEDGRNGSPGPSGPKGDRGEPGPPGPPGRLVDAGIGSRDKGEPGQEGPRGPKGDPGPPGASGERGIEGLRGPPGPQGDPGVRGPAGDKGDRGPPGLDGRNGVDGKPGAPGPPGPHGASGKAGDPGRDGLPGLRGEHGPAGPPGPPGVPGKTGEDGKPGLNGKNGEPGDPGEDGRKGEKGDSGAPGREGPDGPKGERGAPGDPGLRGPPGLPGQVGPPGQGFPGVPGSMGPKGDRGETGSKGEQGLPGERGLRGEPGSLPNAERLLETAGIKVSALRDIVETWGESSGSFLPVPERRPGPKGDPGERGPPGKEGSIGFPGERGLKGDRGDPGPQGPPGLALGERGPPGPPGLAGEPGKPGIPGLPGRAGSAGEAGRPGERGERGEKGDRGEQGRDGLPGLPGPPGPPGPKVAIDEQGPGLSREQGPPGLKGAKGEPGSDGDHGPKGDKGAPGIKGDQGEPGKRGHDGSPGLPGERGVAGPEGKPGLQGPRGTPGPAGGHGDPGPSGAPGLAGPAGPQGPSGLKGEPGETGPPGRGLPGPTGAVGLPGPPGPSGLVGPQGSPGLPGQVGETGKPGPPGRDGTSGKDGERGGPGVPGLPGLPGPVGPKGEPGPVGAPGQVMVGPPGAKGEKGAPGDLAGDLLGEPGAKGDRGLPGPRGEKGEAGRAGEPGDPGEDGQKGAPGLKGLKGEPGIGVQGPPGPTGPPGMKGDVGSPGAPGVVGFPGQTGPRGETGQPGPVGERGLAGPPGREGAPGPLGPPGPPGSVGAPGASGLKGDKGDPGTGLPGPRGERGEPGVRGEDGHPGQEGPRGLMGPPGSRGDRGEKGDTGPAGLKGDKGDSAVIEGPPGIRGAKGDMGERGPRGIDGDKGPRGDNGNPGDKGSKGEPGDKGSAGSIGVRGLPGPKGETGATGIPGEPGAPGKDGAPGFRGDKGDIGFMGPRGLKGERGMKGACGLDGEKGAKGEAGFPGRPGLAGRKGDAGEPGVPGQSGSPGKEGLIGPKGDRGFDGQSGPKGDQGEKGERGPPGVGGFPGPRGNDGSSGPPGPPGGVGPKGPEGLQGQKGERGPPGESVVGAPGAPGAPGERGEQGRPGPAGPRGEKGEAALTEDDIRGFVRQEMSQHCACQGQFIASGSRPLPSYAADTAGPQLHHVPVLRVSHVEEEGQVPPEDDDDFSEYSVYSVEDYHDPEVPWDGDGDIKGWDQRGSDPCSLPLDEGSCTAYTLRWYHRAVPGGTACHPFVYGGCGGNANRFGTREACERRCPPQVVHSQRTGAA

SEQ ID NO: 107 - protein, 781 aa, Cricetulus griseus
MATQADLMELDMAMEPDRKAAVSHWQQQSYLDSGIHSGATTTAPSLSGKGNPEEEDVDTSQVLYEWEQGFSQSFTQEQVADIDGQYAMTRAQRVRAAMFPETLDEGMQIPSTQFDAAHPTNVQRLAEPSQMLKHAVVNLINYQDDAELATRAIPELTKLLNDEDQVVVNKAAVMVHQLSKKEASRHAIMRSPQMVSAIVRTMQNTNDVETARCTAGTLHNLSHHREGLLAIFKSGGIPALVKMLGSPVDSVLFYAITTLHNLLLHQEGAKMAVRLAGGLQKMVALLNKTNVKFLAITTDCLQILAYGNQESKLIILASGGPQALVNIMRTYTYEKLLWTTSRVLKVLSVCSSNKPAIVEAGGMQALGLHLTDPSQRLVQNCLWTLRNLSDAATKQEGMEGLLGTLVQLLGSDDINVVTCAAGILSNLTCNNYKNKMMVCQVGGIEALVRTVLRAGDREDITEPAICALRHLTSRHQEAEMAQNAVRLHYGLPVVVKLLHPPSHWPLIKATVGLIRNLALCPANHAPLREQGAIPRLVQLLVRAHQDTQRRTSMGGTQQQFVEGVRMEEIVEGCTGALHILARDVHNRIVIRGLNTIPLFVQLLYSPIENIQRVAAGVLCELAQDKEAAEAIEAEGATAPLTELLHSRNEGVATYAAAVLFRMSEDKPQDYKKRLSVELTSSLFRTEPMAWNETADLGLDIGAQGEALGYRQDDPSYRSFHSGGYGQDALGMDPMMEHEMGGHHPGADYPVDGLPDLGHAQDLMDGLPPGDSNQLAWFDTDL

SEQ ID NO: 108 - protein, 967 aa, Cricetulus griseus
MQPTVPLGSRKQRPRSDVGHVQRAAKSRSSLPSPMLLLIASVAMLLCVRGAQGRPAEEDEELVLPSLERSPGHDSTTSLRLDAFGQQLHLKLQPDSGFLAPGFTLQTVGRSPGSEAQRLDPTGDLAHCFYSGTVNGDPSSAAALSLCEGVRGAFYLQGEEFFIQPAPEVATERLVPAGPEEESPAAPQFHILRRRRRGSGGAKCGVMDDETLPTSDSRPPESQDPRNQWPLRDPTPQGAGKPTGPGSIRKKRFVSSPRYVETMLVADQSMADFHGSGLKHYLLTLFSVAARFYKHPSIRNSISLVVVKILVIYEEQKGPEVTSNAALTLRNFCSWQKQHNPPSDRDAEHYDTAILFTRQDLCGSHTCDTLGMADVGTVCDPSRSCSVIEDDGLQAAFTTAHELGHVFNMPHDDAKHCASFNGVSGDSHLMASMLSSLDHSQPWSPCSAYMVTSFLDNGHGECLLDKPQNPIKLPSDLPGTMYDANRQCQFTFGEESKHCPDAASTCTTLWCTGTSGGLLVCQTKHFPWADGTSCGEGKWCVSGKCVNKTDMKHFSTPVHGSWGAWGPWGECSRTCGGGVQYTMRECDNPVPKNGGKYCEGKRVRYRSCNIEDCPDNNGKTFREEQCEAHNELSKAPFGNEPTVEWTPKYAGVSPKDRCKLICQAKGIGYFYVLQPKVVDGTPCSPDSTSVCVQGQCVKAGCDHIIDSKKKFDKCGVCGGNGSTCKKISGSVTSTRPGYHDIVTIPAGATNIEVKHRNQRGSRNNGSFLAIRAADGTYILNGNFTLSTLEQDLTYRGTVLRYSGSSAALERIRSFSPLKEPLTIQVLMVGHALRPKIKYTYFVKKKKESFNAIPTFSEWVIEEWGECSKSCGSGWQRRVVECRDINGHPASECAKEVKPASTRPCADLPCPHWQVGDWSPCSKTCGKGYKKRALECLSHDGGVLANESCDPLKKPKHYIDFCTLAECS

SEQ ID NO: 109 - protein, 1662 aa, Cricetulus griseus
MHGGTSLFLILCALASNVPGPASGLETEGRSALDIVHPVRVDAGGSFLSYELWPPRVLHKRDVSATQASSAFYQLQYQGRELLFNLTTNPYLLAPGFVSEIRRRSSLGQMHIRTHVPTCHLLGDVQDPELEGGFAAISACDGLRGVFQLSNEDYFIEPLHGVPAQAGHAQPHVVYKHQVPEQRAQQDGSRAPDTCGVQELEHRRERWEQRQQRRRQQRSVSKEKWVETLVVADAKMVEYHGQPQVESYVLTIMNMVAGLFHDPSIGNPIHITVVRLILLEDEEEDLKITHHADNTLRSFCKWQRNINTKGDAHPQHHDTAILLTRKDLCAAMNHPCETLGLSHVAGMCHPQLSCSVSEDTGMPLAFTVAHELGHSFGIQHDGTGNDCESIGKRPFIMSPQLLYDGGIPLTWSRCSREYITRFLDRGWGLCLDDSPAKNVIGFPSVLPGVLYDVNHQCRLQYGAYSVFCEDMDNVCHTLWCSVGTTCHSKLDAAVDGTSCGKNKWCLNGECVPEGFQPEAVDGGWSGWSAWSVCSRSCGVGVRSAERQCTQPVPKHRGKYCVGERKRFRLCNLSPCPAGQPSFRHTQCSQFDAMLYKGQLHTWVPVVNDENPCALHCRPANQSNTEKLRDAVVDGTPCYQGRVSRDICINGICKNVGCDFEIDSGATEDRCGVCQGNGSTCHTVSRTFEEAEGLGYVDIGLIPAGAREILIKEVAEAANFLALRSEDPDKYFLNGGWTIQWNGDYQVAGTTFTYARTGNWENLTSPGPTKEPVWIQLLFQESNPGVHYEYTIHRDSHDEVQPPEFSWHYGPWSKCTVTCGTGVQRQSLYCMERQAGLVDEEHCDHLNRPDDRQRKCSEEPCPARWWAGEWQMCSRSCGPGGFSRRTVLCIRSVGLDEQRALAPLACEHLPRPLAETPCNRHVPCPSNWGVGNWSQCSVTCGVGVRQRTTLCINDTYVPCDEAERPVTKAICLLPPCPRPVYMTGTDGSGSGSSSPELFNEVDFIPHRLTPRPSPASSPKPVSISNAIDEEDLEPGPPGPVFVDDFYYDYNFINFHEDLSYGSFEEPHSDLVDTGGWTAPPHIRLTEPPSDTPVPTAGTPGVKEDGVQGGWSPSPSLSQDSHSPPVFLEQTPVNPLANFLSEEDMLMGTPEVGLPSLPWPPASADDMVTPVDPGNPDELLVREDRQGQPPTPWSDRNKASKDEDTLGHTLPAPAQIPIPTQPPSPSISTTQVSHGPDMVEVWTGGPVAWDSVLEGDLKHSEQWPTIEAAPPLLPPMATVPGIWDRDSPLEPGTPTFSTPGLGSQNPKTVALPGTLFLTAPTDLSSLGPVGQPQPTNPEGTLSPVLLPRPAQETHNNSSKFPEAQPLQPSLVEDGSPTDPLPAKNASWQVGNWSQCSTTCGLGATWRLVRCSSGRDEDCIPSSRPQPARHCHLRPCAAWRMGNWSKCSRNCGGGSATRDVQCVDTRDLRPLRPFHCQPGPTKPPTRQLCGTQPCLSWYTSSWRECSEACGGGEQQRLVTCPEPGLCEESLRPNSTQPCNTHPCTQWVVGPWGQCSAPCGGGVQRRLVKCVNTQTGLAEEDSELCGHEAWPESSRPCATEDCELVEPPREYLTWTWQSLKWVEIAPRKASTEGYVGRARRSSLQGVRVGRGTGSPLHCLHSFCTPA

SEQ ID NO: 110 - protein, 1903 aa, Cricetulus griseus
MRELEAKATKDVERNLSRDLVQEEEQLMEEKKKKKDDKKKKEAAQKKATEQKIKVPEQIKPSVSQPQPANSDNGTSTATSTNNNAKRATASNQQPPPQQQQQQQQQQQQQQEQQQQPQALPRYPREVPPRFRHQEHKQLLKRGQHFPVIAANLGSAVKVLNSQSESSAVTNQQPQNNGEVQNSKNQSDINHNTSGSHYENCQRGPVSSTSDCSTSCKNAVKDLLEKEAWPSVPGSDPELASECMDADSASSSESERNITVMASGNTGGEKDGLRNSTGLSSQSKFVVGSSSNNVGHGSSTGPWGFPHGAIISTCQVSVDAPESKSESSNNRMNAWGTVSSSSNGGLNPSTLNSASNHGAWPVLENNGLALKGPVGSGSSGINIQCSTIGQMPNNQSINSKVSGSSTHGTWGSLQETCDPEVSGTQKVSFSGQPQNITTETTGPNNTTNFMTSSLPNSGSVQNNELPTSNPGAWRVSTMNHPQIQAPSVMNGTSLSHLSNGESKTGGSYGTTWGAYGSNYSGDKCAGPNGQANGDTVNATLMQPGINGPMGTNFQINTNKGGGVWEPGTTNSQSSPWGSGNGANSGGSRRGWGSPAQNTGTSLPSVEWNKLPSNQHSNDSANGNGKKFTNGWKSTEEEDQGSATSQTNEQNSVWAKTGGTVESDGSTESTGRLDEKVTGESQSRDRRKIDQHTLLQSIVNRTDLDPRVLSNSGWGQTPIKQNTAWDTETSPRGERKTDNGTEAWGSSATQTFNSGACIDKTSPNSNDTSSVSGWGDPKPTLRWGDSKGSNCQGGWEDDSAATGMIKSNQWGNCKEEKSAWNDSQKNKQGWGDGQKSNQGWSISASDNWGETSRSNHWGETNKKSSSGGSDSDRSISGWNELGKTSSFTWGNNINPNNSSGWDDSSKPNSSQGWGDPPKCNQSLGWGDSSKPVSSPDWNKQQDIVGSWGIPPATGKPPGTGWLGGPIPAPTKEEEPTGWEEPSPESIRRKMEIDDGTSAWGDPSKYNYKNVNMWNKNIPDGSSRSDQQAQMHRLLPSANTVSSKEASSGSGWGEPWGEPSTPATTVDNGTSAWGKPTDSGPSWGEPISAASNTSTWGSSSVGPQSLSKSGPKSMQDGWCGDDMPLPGSRPTGWEEEEDVEIGMWNSNSSQELNSSLNWPPYTKKMSSKGLSGKKRRRERAMMKGGNKQEDAWINPFVKQFSNISFSRDSPEENVQSNKMDLSGGMLQDKRMEIDKHSLNIGDYNRTVGKGPGSRPQISKESSMERNPYFDKNGNPSMFGVGNTAAQPRGMQQPPAQPLSSSQPNLRAQVPPPLLSPQVPVSLLKYAPNNGGLNPLFGPQQVAMLNQLSQLNQLSQISQLQRLLAQQQRVQQSQRSVPSANRQQQDQQGRPLSVQQQMMQQSRQLDPSLLVKQQTPPSQQPLHQPAMKSFLDNVMPHTTPELQKGPSPVNAFSNFPIGLNSNLNVNMDMNSIKEPQSRLRKWTTVDSISVNTSLDQNSSKHGAISSGFRLEETPFVPYDFMNSSTSPASPPGSIGDGWPRAKSPNGSSSVNWPPEFRPGEPWKGYPNIDPETDPYVTPGSVINSLSINTVREVDHLRDRNSGSSSSLNTTLPSTSAWSSIRASNYNVPLSSTAQSTSARNSDSKLTWSPGSVTNTSLAHELWKVPLPPKNITAPSRPPPGLTGQKPPLSTWDNSPLRVGGGWGNSDARYTPGSSWGESSSGRITNWLVLKNLTPQIDGSTLRTLCMQHGPLITFHLNLQHGNALVRYSSKEEVVKAQKSLHMCVLGNTTILAEFASEEEISRFFAQSQSLTPSPGWQSLGTSQSRLGSLDCSHSFSSRTDLNHWNGAGLSGTNCGDLHGTSLWGTPHYSTSLWGPPSSSDPRGISSPSPINAFLSVDHLGGGGESM

SEQ ID NO: 111 - protein, 443 aa, Cricetulus griseus
MLPFASCLPGSLLLWALLLLLLGAASPQDSEEPDSYTECTDGYEWDADSQHCRDVNECLTIPEACKGEMKCINHYGGYLCLPRSAAVINDLHGEGPPPPVPPAQHPNPCPPGYEPDEQESCVDVDECAQALHDCRPSQDCHNLPGSYQCTCPDGYRKVGPECVDIDECRYRYCQHRCVNLPGSFRCQCEPGFQLGPNNRSCVDVNECDMGAPCEQRCFNSYGTFLCRCNQGYELHRDGFSCSDIDECSYSSYLCQYRCVNEPGRFSCHCPQGYQLLATRLCQDIDECETGAHQCSEAQTCVNFHGGYRCVDTNRCVEPYVQVSDNRCFCPVSNPLCREQPSSIVHRYMSITSERSVPADVFQIQATSVYPGAYNAFQIRAGNTQGDFYIRQINNVSAMLVLARPVTGPREYVLDLEMVTMNSLMSYRASSVLRLTVFVGAYTF

SEQ ID NO: 112 - protein, 461 aa, Cricetulus griseus
MPLSRALAVLCGVLLCASGLFAVSGDFCDSSLCQNGGTCLISQDNDVYCLCPEGFTGLVCSETEKGPCSPNPCYNDGKCQVTENTQRGDIFTQYICQCSLGYSGTHCEIMNETIYYNLEGDYLSTTAVPIPVPNPGLSNSLASSCTSTLGMEGGAIANSQISASSVYVGFLGVQRWGPELARLHSSGLVNAWTASDYDSKPWIQVNLLRKMRVSGVITQGASRAGRAEYLKTFKVAYSLDGLKFKFIQNASGSGDKVFWGNMDNNGLKVNMFSPSLEAQYIRLYPVSCYRACTLRFELLGCELNGCSEPLGLKNNSIPDSHMTASSTYKTWNLRAFGWYPHYGRLDMQGKINAWTAQSNSNKEWLQVDLCTQRHVTGIITQGARDFGQVQYVASYKVAHSNDGVEWTIYKEQGTDKVFLGNSDNNSHKKNIFETPIVARYVRVLPVSWHKRITLRLELLGC

SEQ ID NO: 113 - protein, 1253 aa, Cricetulus griseus
MPGPRGAARGLAPAMRRAGASGLLALLLLALLGPGGGAEGGPAGERSTGGGGALARERFKVVFAPVICKRTCLKGQCRDSCQQGSNMTLIGENGHSTDTLTGSGFRVVVCPLPCMNGGQCSSRNQCLCPPDFTGRFCQVPAAGTGAGTGSSGPGLARTGAMSTGPLPPLAPEGESVASKHAIYAVQVIPDPPGPGEGSPAQHAAFLVPLGPGQISAEVQAPPPVVNVRVHHPPEASVQVHRIEGPNAEGQASSQHLLPHPKPPHPRPPTQKPLGRCFQDTLPKQPCGSNPLPGLTKQEDCCGSIGTAWGQSKCHKCPQLQYTGVQKPGPVRGEVGADCPQGYKRLNSTHCQDINECAMPGMCRHGDCLNNPGSYRCVCPSGHSLGPSRTQCIADKPEEKSLCFRLVSTEHQCQHPLTTRLTRQLCCCSVGKAWGARCQRCPADGTAAFKEICPAGKGYHILTSHQTLTIQGESDFSLFLHPDGPPKPQQLPESPSRAPPPEDTEEERGVTMDPPVSEERSVQQSHPTATTSPARPYPELISRPSPPTFHRFLPDLPPSRSAVEIAPTQVTETDECRLNQNICGHGQCVPGPSDYSCHCNPGYRSHPQHRYCVDVNECEAEPCGPGRGICMNTGGSYNCHCNRGYRLHVGAGGRSCVDLNECAKPHLCGDGGFCINFPGHYKCNCYPGYRLKTSRPPVCEDIDECRDPSTCPDGKCENKPGSYKCIACQPGYRSQGGGACRDINECSEGSPCSPGWCENLPGSFRCTCAQGYEPAPDGRSCLDMDECEAGNVCSNGICANTPGSFQCQCLSGYHLSRDRSHCEDIDECDFPAACIGGDCINTNGSYRCLCPQGHRLVGGRKCQDIDECSQDPGLCLPHGACENLQGSYVCVCDEGFTLSQDQHGCEEVEQPHHKKECYLNFDDTVFCDSVLATNVTQQECCCSLGAGWGDHCEIYPCPVYSSAEFHSLCPDGKGYTQDNNIINYGIPAHRDIDECILFGAEICKEGKCVNTQPGYECYCKQGFYYDGNLLECVDVDECLDESNCRNGVCENTRGGYRCACTPPAEYNPAQRQCLSPEEMEHAPERREVCWGQRGEDGMCMGPLAGPALTFDDCCCRQGRGWGTQCRPCPPHGTGAQCPTSQSESNSFWDTSPLLLGKSPRDEDSSEEDSDECRCVSGRCVPRPGGAVCECPGGFQLDASRARCVDIDECRELNQRGLLCKSERCVNTSGSFRCVCKAGFTRSRPHGACVPQRRR

SEQ ID NO: 114 - protein, 214 aa, Cricetulus griseus
MSKPPPKPVKPGQVKVFRALYTFEPRTPDELYFEEGDIIYITDMSDTSWWKGTCKGRTGLIPSNYVAEQAESIDNPLHEAAKRGNLSWLRECLDNRVGVNGLDKAGSTALYWACHGGHKDIVEVLFTQPNVELNQQNKLGDTALHAAAWKGYADIVQLLLAKGARTDLRNNEKKLALDMATNAACASLLKKKQATDGVRTLSNAEDYIDEEDSD

SEQ ID NO: 115 - protein, 1217 aa, Cricetulus griseus
MFLYNLTLQRATGISFAIHGNFSGTKQQEIVVSRGKILELLRPDPNTGKVHTLLTVEVFGVIRSLMAFRLTGGTKDYIVVGSDSGRIVILEYQPSKNMFEKIHQETFGKSGCRRIVPGQFLAVDPKGRAVMISAIEKQKLVYILNRDAAARLTISSPLEAHKANTLVYHVVGVDVGFENPMFACLEMDYEEADNDPTGEAAANTQQTLTFYELDLGLNHVVRKYSEPLEEHGNFLITVPGGSDGPSGVLICSENYITYKNFGDQPDIRCPIPRRRNDLDDPERGMIFVCSATHKTKSMFFFLAQTEQGDIFKITLETDEDMVTEIRLKYFDTVPVAAAMCVLKTGFLFVASEFGNHYLYQIAHLGDDDEEPEFSSAMPLEEGDTFFFQPRPLKNLVLVDELDSLSPILFCQIADLANEDTPQLYVACGRGPRSSLRVLRHGLEVSEMAVSELPGNPNAVWTVRRHIEDEFDAYIIVSFVNATLVLSIGETVEEVTDSGFLGTTPTLSCSLLGDDALVQVYPDGIRHIRADKRVNEWKTPGKKTIVKCAVNQRQVVIALTGGELVYFEMDPSGQLNEYTERKEMSADVVCMSLANVPPGEQRSRFLAVGLVDNTVRIISLDPSDCLQPLSMQALPAQPESLCIVEMGGTEKQDELGERGSIGFLYLNIGLQNGVLLRTVLDPVTGDLSDTRTRYLGSRPVKLFRVRMQGQEAVLAMSSRSWLSYSYQSRFHLTPLSYETLEFASGFASEQCPEGIVAISTNTLRILALEKLGAVFNQVAFPLQYTPRKFVIHPESNNLIIIETDHNAYTEATKAQRKQQMAEEMVEAAGEDERELAAEMAAAFLNENLPESIFGAPKAGNGQWASVIRVMNPIQGNTLDLVQLEQNEAAFSVAVCRFSNTGEDWYVLVGVAKDLILSPRSVAGGFVYTYKLVNNGEKLEFLHKTPVEEVPAAIAPFQGRVLIGVGKLLRVYDLGKKKLLRKCENKHIANYISGIQTIGHRVIVSDVQESFIWVRYKRNENQLIIFADDTYPRWVTTASLLDYDTVAGADKFGNICVVRLPPNTNDEVDEDPTGNKALWDRGLLNGASQKAEVIMNYHVGETVLSLQKTTLIPGGSESLVYTTLSGGIGILVPFTSHEDHDFFQHVEMHLRSEHPPLCGRDHLSFRSYYFPVKNVIDGDLCEQFNSMEPNKQKNVSEELDRTPPEVSKKLEDIRTRYAF

SEQ ID NO: 116 - protein, 424 aa, Cricetulus griseus
MSPCSPFIAPPSTVSQRVPASIHGHGPASNSLTSPPRPPAPPWRTWVRGLGFPTLKPDSLLSLSTVCKPRSPKPVAPVAPPFSSSSGVLGNGLCELDRLLQELNATQFNITDEIMSQFPSSKMAEGEEKEDQTEDKNTPTVPPSTFPVPSKPSATSATLELDRLMASLSDFRVQNHLPASGPSQPPVASSTQEGCPSPPGQTSKGSLDTMLGLLQSDLSRRGVPTQAKGLCGSCNKPIAGQVVTALGKAWHPEHFLCSGCSTTLGGSSFFEKDGAPFCPECYFERFSPRCGFCNQPIRHVSSTDALWHPDCFVCRVRGCGERARSPGLVWLALSGSASSRFCSFGSFFEHEGRPLCENHFHAQRGSLCATCGLPVTGRCVSALGRRFHPDHFTCTFCLRPLTKGSFQERAGKPYCQPCFLKLFG

SEQ ID NO: 117 - protein, 348 aa, Cricetulus griseus
MTEMSFLNSEVLAGDLMSPFDQSGLGAEESLGLLDDYLEVAKHFKPHGFSSDKAKAGSSEWLAVDGLVSASDTGKEDAFSGTDWMLEKMDLKEFDFDALFRMDDLDTMPDELLATLDDTCDLFAPLVQETNKEPMTVNPIGHLPESATKIDQVAPFAFLQPFPCSPGVLSSTPDHSFSLELGSEVDISEGDRKPDSAYITLIPQCVKDEDTPSDNDSGICMSPESYLGSPQHSPSTSRGSPSSLPSPVVTRGSPRPKPYDPPGVTLTAKVKIEKLDKKLKKMEQNKTAATRYRQKKRAEQEALTGECRELEKKNEALKEKADSLAKEIQYLKDLIEEVRKARGKKRAP

SEQ ID NO: 118 - protein, 732 aa, Cricetulus griseus
MSRFFTTGSDSESESSLSGEELDTKPVSGNYGRRPLLLSEDEEDTKRVVRSAKDKRFEELTNLIRTIRNAMKIRDVTKCLEEFELLGKAYGKAKSIVDKEGVPRFYIRILADLEDYLNELWEDKEGKKKMNKNNAKALSTLRQKIRKYNRDFESHITNYKQNPEQSADEDAEKNEEDSEGSSDEDEDDDGVSAAAFLKKKPESSGDSRKFLKKMDDDDEDSEDSEDDEEWDTSSTSSDSDSEEEEGKQTVLASKFLKKAPTTEEDKKAAEKKREDKAKKKHDRKSKRLDEEEEDNEGGEWERVRGGVPLVKEKPKMFAKGTEITHAVVIKKLNEILQARGKKGTDRATQIELLQLLVQIASENNLGEGVIVKIKFNIIASLYDYNPNLATYMKPEMWQMCLDCINELMDILVAHSNIFVGENILEESENLHNFDQPLRVRGCILTLVERMDEEFTKIMQNTDPHSQEYVEHLKDEAQVCAIIERVQRYLEEKGTTEEICQIYLRRILHTYYKFDYKAHQRQLTPPEGSSKSEQDQAENEGEDSAVLMERLCKYIYAKDRTDRIRTCAILCHIYHHALHSRWYQARDLMLMSHLQDNIQHADPPVQILYNRTMVQLGICAFRQGLTKDAHNALLDIQSSGRAKELLGQGLLLRSLQERNQEQEKVERRRQVPFHLHINLELLECVYLVSAMLLEIPYMAAHESDARRRMISKQFHHQLRVGERQPLLGEYGVL

SEQ ID NO: 119 - protein, 417 aa, Cricetulus griseus
MLLSVPLLLGLLGLAAAEPAVYFKEQFLDGDDWTNRWVESKHKSDFGKFVLSSGKFYGDQEKDKGLQTSQDARFYALSARFEPFSNKGQTLVVQFTVKHEQNIDCGGGYVKLFPGSLDQKDMHGDSEYNIMFGPDICGPGTKKVHVIFNYKGKNVLINKDIRCKDDEFTHLYTLIVRPDNTYEVKIDNSQVESGSLEDDWDFLPPKKIKDPDAAKPEDWDERAKIDDPTDSKPEDWDKPEHIPDPDAKKPEDWDEEMDGEWEPPVIQNPEYKGEWKPRQIDNPDYKGTWIHPEIDNPEYSPDANIYAYDSFAVLGLDLWQVKSGTIFDNFLITNDEAYAEEFGNETWGVTKASEKQMKDKQDEEQRLKEEEEDKKRKEEEEAEDKEDEDDRDEDEEDEDEKEEDEEDTTPGQTKDEL

SEQ ID NO: 120 - protein, 2154 aa, Cricetulus griseus
MSGALDVLQMKEEDVLKFLAAGTHLGGTNLDFQMEQYIYKRKSDGIYIINLKRTWEKLLLAARAIVAIENPADVSVISSRNTGQRAVLKFAAATGATPIAGRFTPGTFTNQIQAAFREPRLLVVTDPRADHQPLTEASYVNLPTIALCNTDSPLRYVDIAIPCNNKGAHSVGLMWWMLAREVRRMRGTISREHPWEVMPDLYFYRDPEEIEKEEQAAAEKAVTKEEFQGEWTAPAPEFTAAQPEVADWSEGVQVPSVPIQQFPTEDWSAQPATEDWSAAPTAQATEWVGATTEWSGHWTRINUCLEOTIDEREPEATCONTAININGGENEBPROTEINTNRCBMQTNEGEVEEESCSKVEQEDFVMEGHGKTPPPGEESKQEKEQEREEQLMEDKKRKKEDKKKKEATQKVTEQKTKVPEVTKPSLSQPTAASPIGSSPSPPVNGGNNAKRVAVPNGQPPSAARYMPREVPPRFRCQQDHKVLLKRGQPPPPSCMLLGGGAGPPPCTAPGANPNSNAQVTGTLLQNESGTAPESTLGGAAASNYANSTWGPGASSNNGASPNPIHIWDKVIVDGSDMEEWPCIASKDTESSSENTTDNNSASNPGSEKSTLPGSTTSNKGKGSQCQSANSGNECNLGVWKSDPKAKSVQSSNSTSDSSSGLGNWRNVSGQDRIGPGSGFSNFNPNSNPSAWPALVQEGTSRKGVLETENSNSGAQVSTVGQASREQQSKMENAGVNFVVSGREQAQIHNTDGPKNGNTNSLNLSSPNPMENKGIPFGMGLGNTSRSTDAPSQSTGDRKTGSVGSWGAARGPSGTDTVSGQSNSGNNGNNGKDREDSWKGAPVPKSTGSKNDSWDNNNRSTGGSWNFGPQDSNDNKWGEGNKMTSGVSQGEWKQPTGSDELKIGEWSGPNQPNSSTGAWDNQKGHPLPENQGNAQAPCWGRSSSSAGSEVGGQSTGSNHKAGSSDSHNSGRRSYRPTHPDCQAVLQTLLSRTDLDPRVLSNTGWGQTQIKQDTVWDIEEVPRPEGKSDKGTEGWESAATQTKNSGGWGDAPSQSNQMKSGWGELSASTEWKDPKSTGGWNDYKNNNSSNWGGRADEKTPSSWNESSCKDQGWGGGRQPNQGWTSGKNGWGEEVEQVKNNNWESSANKPVSGWGEGGQNEIGTWGNGGNANLASKGGWEDCKRSPAWNETGRQPNSWNKQHQQQQQPPPPPQPEASGSWGGPPPPPPGNVRPSNSNWSSGPQPTTPKDDEPSGWEEPSPQSISRKMDIDDGTSAWGDPNSYNYKNVNLWDKNSQGGPPPREPNLPTPMAGKSASVWSKSTPPAPDNGTSAWGEPNESSPGWGEMDDSGASTTGWGNTPASAPNAMKPNTKSMQDGWGESDGPVTGTRHPSWEEEDDGGVWNTAGSQGSTSSHNSASWGQGGKKQMKCSLKGGNNDSWMNPLAKQFSNMGLLSQTEDNPSSKMDLSVDKKFDVDKRTMNLGDFNDIMRKDRPGFRPPNSKDLGTADSGPYFEKGGNHGLFGNSTAQSRGLHTPVQPLSSSPGLRAQVPPQFISPQVSASMLKQFPNSGLNPGLFNVGPQLSPQQIAMLSQLPQIPQFQLACQLLLQQQQQQQLLQNQRKISQAVRQQQEQQLARMVSALQQQQQQQQQQQQRQPSMKHSPSHPVGPKPHLDNMVPNALNVGLPDLQNKGPIPGYGSGFSSGGMDYGMVGGKEAGTESRFKQWTSMMEGLPSVATQEATMHKNGSIVAPGKTRGGSPYNQFDIIPGDTLGGHTGPAGDSWLPAKSPPTNKIGSKSSNASWPPEFQPGVPWKGIQNIDPESDPYVTPGSVLGGTATSPIVDTDHQLLRDNTTGSNSSLNTSLPSPGAWPYSASDNSFTNVHSTSAKFPDYKSTWSPDPIGHNPTHLSNKMWKNHISSRNTTPLPRPPPGLTNPKPASPWSSTAPRSVRGWGTQDSRIASASTWSDGGSVRASYWLVLHNLTPQIDGSTLRTICMQHGPLLTFHLNLTQGTALIRYSTKQEAAKAQTALHMCVLGNTTILAEFATEDEVSRFLAQAQPPTPAATPSAPATGWQSLETSQNQADPVGPALNLFGGSTGLGQWSSSAGGSSGADLAGTSLWGPPNYSSSLWGVSTVEDPHRMGSPAPLLPGDLLGGGSDSI

SEQ ID NO: 121 - protein, 1810 aa, Cricetulus griseus
MQTNEGEVEEESCSKVEQEDFVMEGHGKTPPPGEESKQEKEQEREEQLMEDKKRKKEDKKKKEATQKVTEQKTKVPEVTKPSLSQPTAASPIGSSPSPPVNGGNNAKRVAVPNGQPPSAARYMPREVPPRFRCQQDHKVLLKRGQPPPPSCMLLGGGAGPPPCTAPGANPNSNAQVTGTLLQNESGTAPESTLGGAAASNYANSTWGPGASSNNGASPNPIHIWDKVIVDGSDMEEWPCIASKDTESSSENTTDNNSASNPGSEKSTLPGSTTSNKGKGSQCQSANSGNECNLGVWKSDPKAKSVQSSNSTSDSSSGLGNWRNVSGQDRIGPGSGFSNFNPNSNPSAWPALVQEGTSRKGVLETENSNSGAQVSTVGQASREQQSKMENAGVNFVVSGREQAQIHNTDGPKNGNTNSLNLSSPNPMENKGIPFGMGLGNTSRSTDAPSQSTGDRKTGSVGSWGAARGPSGTDTVSGQSNSGNNGNNGKDREDSWKGAPVPKSTGSKNDSWDNNNRSTGGSWNFGPQDSNDNKWGEGNKMTSGVSQGEWKQPTGSDELKIGEWSGPNQPNSSTGAWDNQKGHPLPENQGNAQAPCWGRSSSSAGSEVGGQSTGSNHKAGSSDSHNSGRRSYRPTHPDCQAVLQTLLSRTDLDPRVLSNTGWGQTQIKQDTVWDIEEVPRPEGKSDKGTEGWESAATQTKNSGGWGDAPSQSNQMKSGWGELSASTEWKDPKSTGGWNDYKNNNSSNWGGRADEKTPSSWNESSCKDQGWGGGRQPNQGWTSGKNGWGEEVEQVKNNNWESSANKPVSGWGEGGQNEIGTWGNGGNANLASKGGWEDCKRSPAWNETGRQPNSWNKQHQQQQQPPPPPQPEASGSWGGPPPPPPGNVRPSNSNWSSGPQPTTPKDDEPSGWEEPSPQSISRKMDIDDGTSAWGDPNSYNYKNVNLWDKNSQGGPPPREPNLPTPMAGKSASVWSKSTPPAPDNGTSAWGEPNESSPGWGEMDDSGASTTGWGNTPASAPNAMKPNTKSMQDGWGESDGPVTGTRHPSWEEEDDGGVWNTAGSQGSTSSHNSASWGQGGKKQMKCSLKGGNNDSWMNPLAKQFSNMGLLSQTEDNPSSKMDLSVDKKFDVDKRTMNLGDFNDIMRKDRPGFRPPNSKDLGTADSGPYFEKGGNHGLFGNSTAQSRGLHTPVQPLSSSPGLRAQVPPQFISPQVSASMLKQFPNSGLNPGLFNVGPQLSPQQIAMLSQLPQIPQFQLACQLLLQQQQQQQLLQNQRKISQAVRQQQEQQLARMVSALQQQQQQQQQQQQRQPSMKHSPSHPVGPKPHLDNMVPNALNVGLPDLQNKGPIPGYGSGFSSGGMDYGMVGGKEAGTESRFKQWTSMMEGLPSVATQEATMHKNGSIVAPGKTRGGSPYNQFDIIPGDTLGGHTGPAGDSWLPAKSPPTNKIGSKSSNASWPPEFQPGVPWKGIQNIDPESDPYVTPGSVLGGTATSPIVDTDHQLLRDNTTGSNSSLNTSLPSPGAWPYSASDNSFTNVHSTSAKFPDYKSTWSPDPIGHNPTHLSNKMWKNHISSRNTTPLPRPPPGLTNPKPASPWSSTAPRSVRGWGTQDSRIASASTWSDGGSVRASYWLVLHNLTPQIDGSTLRTICMQHGPLLTFHLNLTQGTALIRYSTKQEAAKAQTALHMCVLGNTTILAEFATEDEVSRFLAQAQPPTPAATPSAPATGWQSLETSQNQADPVGPALNLFGGSTGLGQWSSSAGGSSGADLAGTSLWGPPNYSSSLWGVSTVEDPHRMGSPAPLLPGDLLGGGSDSI

SEQ ID NO: 122 - protein, 737 aa, Cricetulus griseus
MAASPVPGGGGGGGGGGAGAVHSSSTSGFAFDSGLEIRTRSVEQTLLPLVSQITTLINHKDNTKKSDKTLQAIQRVGQAVNLAVGRFVKVGEAIANENWDLKEEINIACIEAKQAGETIAALTDVTKLNHVESSGQITILTDKTGVVQAARLLLSSVTKVLLLADRVVIKQIVTSRNKVLATMERLEKVNSFQEFVQIFSQFGNEMVEFAHLTGDRQNDLKDEKKKASMAVARAVLEKGTMMLLTASKTCLRHPSCDSAHKNKEGVFDRMRVALDKVIEIVTESKPNGETDRSSVSVFTGIKELKLNIEALWENLYFESKENLAAALEVILERVEDFTDSAYTSHEHRERILELSTQARTELQQFISVWMQAQSRKTKSAAEELELTVLRVSHSLNQLRKELHHTAMQLAADLLKFHADHVVLKALKLTGVEGNLEALAEYACKLSEQKEQLVETCRLLRHVSGTEPLEITCIHAEETFQVTGPQIISAAETLTLHPSSKIAKENLDVFCEAWESQISDMATLLREISDVFKGRRGEKYDHLSLPRPMKNNANLKSLKPDKPDSEEQAKIAKLGLKLALLTSDTDCELEKWEDQENEIARHGRNMSRMAYSLYLFTRGEGPLKTSHDLIHFLEGFAAEGLKLTSNVQSFSKQLKDDDKLMLLLEINKLIPLCHQLQTITKTSLQNKVFLKVDKCITKIRSMMALVVQLLSLCYKLLKKVESNRWVSVTKKDIMDGKT

SEQ ID NO: 123 - protein, 906 aa, Cricetulus griseus
MTAVHTGNINFKWDPKSLEIRTLAVERLLEPLVTQVTTLVNTNSKGPSNKKRGRSKKAHVLAASVEQATENFLEKGDKIAKESQFLKEELVAAVEDVRKQGDLMKSAAGEFADDPCSSVKRGNMVRAARALLSAVTRLLILADMADVYKLLVQLKVVEDGILKLRNAGNEQDLGIQYKALKPEVDKLNIMAAKRQQELKDVGHRDQMAAARGILQKNVPILYTASQACLQHPDVAAYKANRDLIYKQLQQAVTGISNAAQATASDDASQHQGAGGGELAYALNNFDKQIIVDPLSFSEERFRPSLEERLESIISGAALMADSSCTRDDRRERIVAECNAVRQALQDLLSEYMGNAGRKERSDALNSAIDKMTKKTRDLRRQLRKAVMDHVSDSFLETNVPLLVLIEAAKNGNEKEVKEYAQVFREHANKLIEVANLACSISNNEEGVKLVRMSASQLEALCPQVINAALALAAKPQSKLAQENMDLFKEQWEKQVRVLTDAVDDITSIDDFLAVSENHILEDVNKCVIALQEKDVDGLDRTAGAIRGRAARVIHVVTSEMDNYEPGVYTEKVLEATKLLSNTVMPRFTEQVEAAVEALSSDPAQPMDENEFIDASRLVYDGIRDIRKAVLMIRTPEELDDSDFETEDFDVRSRTSVQTEDDQLIAGQSARAIMAQLPQEQKAKIAEQVASFQEEKSKLDAEVSKWDDSGNDIIVLAKQMCMIMMEMTDFTRGKGPLKNTSDVISAAKKIAEAGSRMDKLGRTIADHCPDSACKQDLLAYLQRIALYCHQLNICSKVKAEVQNLGGELVVSGVDSAMSLIQAAKNLMNAVVQTVKASYVASTKYQKSQGMASLNLPAVSWKMKAPEKKPLVKREKQDETQTKIKRASQKKHVSPVQALSEFKAMDSI

SEQ ID NO: 124 - protein, 1498 aa, Cricetulus griseus
MMANWVVARPLLILTVLLGHCVSIKAQEQENDEYDEEIACTQGGQMYLNRDIWKPSPCQICVCDNGAILCDKIECPEMLTCANPITPAGECCPVCPQTPGGGDTNFGRGRKGQKGEPGLVPVVTGIRGRPGPAGPPGSQGPRGDRGPKGRPGPRGPQGIDGEPGVPGQPGAPGPPGHPSHPGPDGMSRPFSAQMAGLDEKSGLGSQVGLMPGSVGPVGPRGPQGLQGQQGGVGPTGPPGEPGEPGPMGPIGARGPEGPPGKPGEDGEPGRNGNTGEVGFSGSPGARGFPGAPGLPGLKGHRGHKGLEGPKGEVGATGAKGEAGPTGPMGAMGPLGPRGMPGERGRLGPQGAPGQRGAHGMPGKPGPMGPLGIPGSSGFPGNPGMKGEAGPTGARGPEGPQGQRGETGPPGPVGSHGLPGAVGTDGTPGAKGPTGSAGTSGPPGLSGPPGSPGPQGSTGPQGIRGQPGDPGVPGFKGEAGPKGEPGPHGVQGPIGPPGEEGKRGPRGDPGTVGPPGPMGERGAPGNRGFPGSDGLPGPKGAQGERGPVGSSGPKGGQGDPGRPGEPGLPGARGLTGNPGVQGPEGKLGPLGAPGEDGRPGPPGSVGIRGQPGSMGLPGPKGSSGDLGKPGEAGNAGVPGQRGAPGKDGEVGPSGPVGPPGLAGERGEQGPPGPTGFQGLPGPPGPPGEGGKSGDQGVPGEPGAVGPLGPRGERGNPGERGEPGITGLPGEKGMAGGHGPDGPKGNPGPTGTIGDTGPPGLQGMPGERGIAGTPGPKGDRGGIGEKGAEGTAGNDGARGLPGPLGPPGPAGPTGEKGEPGPRGLVGPPGSRGNPGSRGENGPTGAVGFAGPQGPDGQPGVKGEPGEPGQKGDAGSPGPQGLAGSPGPHGPHGVPGLKGGRGTQGPPGATGFPGSAGRVGPPGPAGAPGPAGPIGEPGKEGPPGLRGDPGSHGRVGDRGPAGPPGGPGDKGDPGEDGQPGPDGPPGPAGTTGQRGIVGMPGQRGERGMPGLPGPAGTPGKVGPTGATGDKGPPGPVGPPGSNGPVGEPGPEGPAGNDGTPGRDGAVGERGDRGDPGPAGLPGSQGAPGTPGPVGAPGDAGQRGDPGSRGPVGPPGRAGKRGLPGPQGPRGDKGDNGDRGDRGQKGHRGFTGLQGLPGPPGPNGEQGSAGIPGPFGPRGPPGPVGPSGKEGNPGPLGPIGPPGVRGSVGEAGPEGPPGEPGPPGPPGPPGHLTAALGDIMGHYDENMPDPLPEFTEDQAAPDDTNKTDPGVHATLKSLSSQIETMRSPDGSKKHPARTCDDLKLCHSTKQSGEYWIDPNQGSSEDAIKVYCNMETGETCISANPASVPLKTWWASKSPDSKPVWYGLDMNRGSQFTYGDYQSPNTAITQMTFLRLLSKEASQNITYVCRNTVGYMDDQAKNLKKAVVLKGSNDLEIKGEGNIRFRYTVLQDTCSKRNGNVGKTIFEYRTQNVARLPIIDLAPVDIGNTDQEFGIEIGPVCFM

SEQ ID NO: 125 - protein, 1112 aa, Cricetulus griseus
MEPSGGGLGPGRGTRDKKKGRSPDELPATGGDGGKPKKFTLKRLMADELERFTSMRIKKEKEKPNSAHRNSSAMYGDDPTVQPLHDITDEQVLVFFEQMLVDMNLNEEKQQPLREKDIVIKREMVSQYLHTSSAGMNQKESSRSAMMYIQELRSGLRDMHLLSCLESLRVSLNNNPVSWVQTFGAEGLASLLDILKRLHDEKEETSGSYDSRNQHEIIRCLKAFMNNKFGIKTMLETEEGILLLVRAMDPAVPNMMIDAAKLLSALCILPQPEDMNERVLEAMTERAEMDEVERFQPLLDGLKSGTSIALKVGCLQLINALITPAEELDFRVHIRSELMRLGLHQVLQELREIENDDMRVQLSVFDEQAEEDFFDLKGRLDDILFQILLNTVKDSKAEPHFLSILQHLLLVRNDYEARPQYYKLIEECVSQIVLHKNGTDPDFKCRHLQIDIEGLIDQMIDKTKVEKSEAKATELEKKLDSELTARHELQVEMKKMENDFEQKLLDLQGEKDALDSEKQQIATQKQDLEVEVSKLTGEVAKLSKELEDAKKEMASLSAVVVSSSAAVPPAPPLPGGPGTVIPPPPPPPPLPGGTFPPPAPPLPGVAAISPPPPVPGGASVPPPPPLPGSTAIPPPPPLPGGCVIPPPPPLPGGCVIPPPPPLPGSASVPALPPSXXXXXXXXXXXXXXXXXXXXXXXXXXXXXXXXXXFTKKDQEGGEEKKSVQKKKVKELKVLDSKTAQNLSIFLGSFRMPYQEIKSVILEVNEAVLTESMIQNLIKQMPEPEQLKMLSELKDEYDDLAESEQFGVVMGTVPRLRPRLNAILFKLQFSEQVENIKPEIVSVTAACEELRKSESFSSLLEITLLVGNYMNAGSRNAGAFGFNISFLCKLRDTKSADQKMTLLHFLAELCENDYPDVLKFPDELAHVEKASRVSAENLQKNLDQMKKQIADVERDVQNFPAATDEKDNFVKDAQEQYNKLRMMHSNMETLYKELGDYFIFDPKKLSVEEFFMDLHNFRNMFLVSKGKLLIFHGGDETGVMDSLLEALQSGAAFRRKRGPRQVNRKAGCAVTSLLASELTKDDAMSAGPAKVPKKSEGVPTILEEAKELVGRAS

SEQ ID NO: 126 - protein, 380 aa, Cricetulus griseus
MARARVSLWAICVLRVALATVYFQEEFLDGERWRNRWVQSTNDSQFGHFRVSSGKFYGHIEKDKGLQTTQNSRFYAISASFKPFSNKGKTLVIQYTVKHEQKMDCGGGYIKVFPSDLDQKNMNGKSQYYIMFGPDICGFDIKKVHVILYFKNQYHSNKKTIRCKVDGFTHLYTLILRPDLSYEVKIDGQSIESGSIEYDWNLMSLKKMEKTSAESRDWDQVESDKAQDWEKHFLDAGASKPSDWNSELDGDWLQKPPYQDGLKAEGIDKDVWLHREMKPANYLTQYDLSEFENIGAVGLELWQVRSGTIFDNFLITDDEEYAERFGKATWGETKGPEKEMDAIQAKEEVKKAREEDEELLVGKFHSHSSHFSRFHRQGEL

SEQ ID NO: 127 - protein, 450 aa, Cricetulus griseus
MAAADGGRDFTDIESKFALRTPDDTAEDNCHLIPGIAESVSNCHFNHSSKTFVVIHGWTVTGMYESWVPKLVAALYKREPDSNVIVVDWLYRAQQHYPVSAGYTKLVGNDVARFINWMEEEFNYPLDNVHLLGYSLGAHAAGVAGSLTNKKVNRITGLDPAGPNFEYAEAPSRLSPDDADFVDVLHTFTRGSPGRSIGIQKPVGHVDIYPNGGTFQPGCNIGEAIRVIAERGLGDVDQLVKCSHERSIHLFIDSLLNEENPSKAYRCNSKEAFEKGLCLSCRKNRCNNVGYEINKVRAKRSSKMYLKTRSQMPYKVFHYQVKIHFSGTESDKQLNQAFEISLYGTVAESENIPFTLPEVSTNKTYSFLIYTEVDIGELLMMKLKWKSDSYFSWSDWWSSPGFVIEKIRVKAGETQKKVIFCAREKVSHLQKGKDSAVFVKCHDKSLKKSG

SEQ ID NO: 128 - protein, 369 aa, Cricetulus griseus
MSPLWLLTLLLALSQALPFEQKGFWDFTLDDGLLMMHDEEASGSDTTSGVPDLDSLTPTFSAMCPFGCHCHLRVVQCSDLGLKTVPKEISPDTTLLDLQNNDISELRKDDFKGLQHLYALVLVNNKISKIHEKAFSPLRKLQKLYISKNHLVEIPPNLPSSLVELRIHDNRIRKVPKGVFSGLRNMNCIEMGGNPLENSGFEPGAFDGLKLNYLRISEAKLTGIPKDLPETLNELHLDHNKIQAIELEDLLRYSKLYRLGLGHNQIRMIENGSLSFLPTLRELHLDNNKLSRVPAGLPDLKLLQVVYLHSNNITKVGINDFCPMGFGVKRAYYNGISLFNNPVAYWEVQPATFRCVTDRLAIQFGNYKK

SEQ ID NO: 129 - RNA, 20 nt, synthetic construct
  source 1..20: mol_type = other RNA
gagcaaagccctgctcctgg

SEQ ID NO: 130 - RNA, 20 nt, synthetic construct
  source 1..20: mol_type = other RNA
cagagtttgaccgcctccca

SEQ ID NO: 131 - RNA, 20 nt, synthetic construct
  source 1..20: mol_type = other RNA
ctgctgcggccatccttggg

SEQ ID NO: 132 - RNA, 20 nt, synthetic construct
  source 1..20: mol_type = other RNA
atccagcttccagaatgtgg

SEQ ID NO: 133 - RNA, 20 nt, synthetic construct
  source 1..20: mol_type = other RNA
ttaatcaggtcatccgacag

SEQ ID NO: 134 - RNA, 20 nt, synthetic construct
  source 1..20: mol_type = other RNA
caaacggaatacgacatggc

SEQ ID NO: 135 - RNA, 20 nt, synthetic construct
  source 1..20: mol_type = other RNA
agtttgaccgcctcccaagg

SEQ ID NO: 136 - RNA, 20 nt, synthetic construct
  source 1..20: mol_type = other RNA
gaccgcctcccaaggagggg

SEQ ID NO: 137 - RNA, 20 nt, synthetic construct
  source 1..20: mol_type = other RNA
tgcggccacccctccttggg

SEQ ID NO: 138 - RNA, 20 nt, synthetic construct
  source 1..20: mol_type = other RNA
agcaaggtgagtagccacag

SEQ ID NO: 139 - RNA, 20 nt, synthetic construct
  source 1..20: mol_type = other RNA
cattcaccatgagtcccctg

SEQ ID NO: 140 - RNA, 20 nt, synthetic construct
  source 1..20: mol_type = other RNA
gctgctcatgatgcatgatg

SEQ ID NO: 141 - RNA, 20 nt, synthetic construct
  source 1..20: mol_type = other RNA
gggggtcagtcctacaagat

SEQ ID NO: 142 - RNA, 20 nt, synthetic construct
  source 1..20: mol_type = other RNA
atgtaaccaccagtttcatg

SEQ ID NO: 143 - RNA, 20 nt, synthetic construct
  source 1..20: mol_type = other RNA
aggaggccacatgaaactgg

SEQ ID NO: 144 - RNA, 20 nt, synthetic construct
  source 1..20: mol_type = other RNA
tccatctggcataacagctg

SEQ ID NO: 145 - RNA, 20 nt, synthetic construct
  source 1..20: mol_type = other RNA
atgtctctgaattgtccatc

SEQ ID NO: 146 - RNA, 20 nt, synthetic construct
  source 1..20: mol_type = other RNA
tcttacctctgtattcactt

SEQ ID NO: 147 - RNA, 20 nt, synthetic construct
  source 1..20: mol_type = other RNA
cttcgggtcttggacagggg

SEQ ID NO: 148 - RNA, 20 nt, synthetic construct
  source 1..20: mol_type = other RNA
taccttcgggtcttggacag

SEQ ID NO: 149 - RNA, 20 nt, synthetic construct
  source 1..20: mol_type = other RNA
ggtgtggagcaagcccacag

SEQ ID NO: 150 - RNA, 20 nt, synthetic construct
  source 1..20: mol_type = other RNA
gcaaatcactgcaaatctca

SEQ ID NO: 151 - RNA, 20 nt, synthetic construct
  source 1..20: mol_type = other RNA
gagaggaggcaatgccaaag

SEQ ID NO: 152 - RNA, 20 nt, synthetic construct
  source 1..20: mol_type = other RNA
tggcattgcctcctctctcc

SEQ ID NO: 153 - RNA, 20 nt, synthetic construct
  source 1..20: mol_type = other RNA
caaggccctttaccagtcgt

SEQ ID NO: 154 - RNA, 20 nt, synthetic construct
  source 1..20: mol_type = other RNA
cagcccacacagcatccagt

SEQ ID NO: 155 - RNA, 20 nt, synthetic construct
  source 1..20: mol_type = other RNA
tactggccagatcttcagtg

SEQ ID NO: 156 - protein, 1016 aa, Cricetulus griseus
MASHQHAVKANFWRLLEKVTTNGIIAMSEPPARESHPGTFPPSFGSVAPFLADLDTTDGLGNVYYREDLSPSIMQMAAEYVQRGFPEVPFQPTSVVVVTWESVAPYEGPSGSSAQEGKRNTFQAVLASSNSSSYAIFLYPEDGLQFFTTFSKKDENQVPAMVGFSQGLVGFLWRSDGAYNIFANDRESIENLAKSSNAGHQGVWVFEIGSPATAKGVVSADVNLGLDDDGSDYEDEEYDLATSHLGLEDMATQPFPSPSPRRGNTHPHDVPRVLSPSYEATERPHGIPTERTRTFQLPAERFHQQHPQVIDVDEVEETGIVFSYNIGSQQTCANNRHQCSVHAECRDYATGFCCRCVANYTGNGRQCVAEGSPQRVNGKVKGRIFVGNSQVPVVFENTDLHSYVVMNHGRSYTAISTIPETVGYSLLPLAPIGGIIGWMFAVEQNGFKNGFSITGGEFTRQAEVTFLGHPGKLVLKQHFSGIDEHGHLTINTELDGRVPQIPYGSSVHIEPYTELYHYSSSVITSSSTREYTVTEPDPDGTAPSHTHVYQWRQTITFQECVHDDSRPALPSTQQLSVDSVFVLYNQEERILRYALSNSIGPVREGSPDALQNPCYIGTHGCDSNAACRPGPGTQFTCECSIGFRGDGQTCYDIDECSEQPSRCGNHAICNNYPGAYRCECVEGYHFSDGGICVADVDQRPINYCETGLHNCDIPQRAQCIYMGGSSYTCSCLPGFSGDGRACQDVDECQLSRCHPDAFCYNTPGSFTCQCKPGYQGDGFQCVPGGLYVTDEAREKICSLVLLLWTGVKQDLKVGSKVKYLTVVGSMKQSQVPDYGGQYGEKPRNSLTTKKHKEELGAMRGLSSLISPECPAESVLLPFAVSHADLDTSLACGHRTAQLWGSESPQGCIPHISYTLVALLLSHAAPPADLSFPKDTICYQSTKFYNTPASWLTVLLDISQWLWSVSHCTKPQVCHSERSATPLMEMDELLPVTINLSTKSHRDPLPHVRFLPATRPN